European Patent Application EP 4 293 118 A1, published December 20, 2023. Title: Kit for producing adeno-associated virus and use thereof. Applicant: FUJIFILM Corporation. The sequence listing filed with the application follows.

SEQUENCE LISTING (43 sequences)

SEQ ID NO: 1 - DNA, 11635 bp, Artificial Sequence
  plasmid
ggtacccaactccatgcttaacagtccccaggtacagcccaccctgcgtcgcaaccaggaacagctctacagcttcctggagcgccactcgccctacttccgcagccacagtgcgcagattaggagcgccacttctttttgtcacttgaaaaacatgtaaaaataatgtactaggagacactttcaataaaggcaaatgtttttatttgtacactctcgggtgattatttaccccccacccttgccgtctgcgccgtttaaaaatcaaaggggttctgccgcgcatcgctatgcgccactggcagggacacgttgcgatactggtgtttagtgctccacttaaactcaggcacaaccatccgcggcagctcggtgaagttttcactccacaggctgcgcaccatcaccaacgcgtttagcaggtcgggcgccgatatcttgaagtcgcagttggggcctccgccctgcgcgcgcgagttgcgatacacagggttgcagcactggaacactatcagcgccgggtggtgcacgctggccagcacgctcttgtcggagatcagatccgcgtccaggtcctccgcgttgctcagggcgaacggagtcaactttggtagctgccttcccaaaaagggtgcatgcccaggctttgagttgcactcgcaccgtagtggcatcagaaggtgaccgtgcccggtctgggcgttaggatacagcgcctgcatgaaagccttgatctgcttaaaagccacctgagcctttgcgccttcagagaagaacatgccgcaagacttgccggaaaactgattggccggacaggccgcgtcatgcacgcagcaccttgcgtcggtgttggagatctgcaccacatttcggccccaccggttcttcacgatcttggccttgctagactgctccttcagcgcgcgctgcccgttttcgctcgtcacatccatttcaatcacgtgctccttatttatcataatgctcccgtgtagacacttaagctcgccttcgatctcagcgcagcggtgcagccacaacgcgcagcccgtgggctcgtggtgcttgtaggttacctctgcaaacgactgcaggtacgcctgcaggaatcgccccatcatcgtcacaaaggtcttgttgctggtgaaggtcagctgcaacccgcggtgctcctcgtttagccaggtcttgcatacggccgccagagcttccacttggtcaggcagtagcttgaagtttgcctttagatcgttatccacgtggtacttgtccatcaacgcgcgcgcagcctccatgcccttctcccacgcagacacgatcggcaggctcagcgggtttatcaccgtgctttcactttccgcttcactggactcttccttttcctcttgcgtccgcataccccgcgccactgggtcgtcttcattcagccgccgcaccgtgcgcttacctcccttgccgtgcttgattagcaccggtgggttgctgaaacccaccatttgtagcgccacatcttctctttcttcctcgctgtccacgatcacctctggggatggcgggcgctcgggcttgggagaggggcgcttctttttctttttggacgcaatggccaaatccgccgtcgaggtcgatggccgcgggctgggtgtgcgcggcaccagcgcatcttgtgacgagtcttcttcgtcctcggactcgagacgccgcctcagccgcttttttgggggcgcgcggggaggcggcggcgacggcgacggggacgacacgtcctccatggttggtggacgtcgcgccgcaccgcgtccgcgctcgggggtggtttcgcgctgctcctcttcccgactggccatttccttctcctataggcagaaaaagatcatggagtcagtcgagaaggaggacagcctaaccgccccctttgagttcgccaccaccgcctccaccgatgccgccaacgcgcctaccaccttccccgtcgaggcacccccgcttgaggaggaggaagtgattatcgagcaggacccaggttttgtaagcgaagacgacgaggatcgctcagtaccaacagaggataaaaagcaagaccaggacgacgcagaggcaaacgaggaacaagtcgggcggggggaccaaaggcatggcgactacctagatgtgggagacgacgtgctgttgaagcatctgcagcgccagtgcgccattatctgcgacgcgttgcaagagcgcagcgatgtgcccctcgccatagcggatgtcagccttgcctacgaacgccacctgttctcaccgcgcgtaccccccaaacgccaagaaaacggcacatgcgagcccaacccgcgcctcaacttctaccccgtatttgccgtgccagaggtgcttgccacctatcacatctttttccaaaactgcaagatacccctatcctgccgtgccaaccgcagccgagcggacaagcagctggccttgcggcagggcgctgtcatacctgatatcgcctcgctcgacgaagtgccaaaaatctttgagggtcttggacgcgacgagaaacgcgcggcaaacgctctgcaacaagaaaacagcgaaaatgaaagtcactgtggagtgctggtggaacttgagggtgacaacgcgcgcctagccgtgctgaaacgcagcatcgaggtcacccactttgcctacccggcacttaacctaccccccaaggttatgagcacagtcatgagcgagctgatcgtgcgccgtgcacgacccctggagagggatgcaaacttgcaagaacaaaccgaggagggcctacccgcagttggcgatgagcagctggcgcgctggcttgagacgcgcgagcctgccgacttggaggagcgacgcaagctaatgatggccgcagtgcttgttaccgtggagcttgagtgcatgcagcggttctttgctgacccggagatgcagcgcaagctagaggaaacgttgcactacacctttcgccagggctacgtgcgccaggcctgcaaaatttccaacgtggagctctgcaacctggtctcctaccttggaattttgcacgaaaaccgcctcgggcaaaacgtgcttcattccacgctcaagggcgaggcgcgccgcgactacgtccgcgactgcgtttacttatttctgtgctacacctggcaaacggccatgggcgtgtggcagcaatgcctggaggagcgcaacctaaaggagctgcagaagctgctaaagcaaaacttgaaggacctatggacggccttcaacgagcgctccgtggccgcgcacctggcggacattatcttccccgaacgcctgcttaaaaccctgcaacagggtctgccagacttcaccagtcaaagcatgttgcaaaactttaggaactttatcctagagcgttcaggaattctgcccgccacctgctgtgcgcttcctagcgactttgtgcccattaagtaccgtgaatgccctccgccgctttggggtcactgctaccttctgcagctagccaactaccttgcctaccactccgacatcatggaagacgtgagcggtgacggcctactggagtgtcactgtcgctgcaacctatgcaccccgcaccgctccctggtctgcaattcgcaactgcttagcgaaagtcaaattatcggtacctttgagctgcagggtccctcgcctgacgaaaagtccgcggctccggggttgaaactcactccggggctgtggacgtcggcttaccttcgcaaatttgtacctgaggactaccacgcccacgagattaggttctacgaagaccaatcccgcccgccaaatgcggagcttaccgcctgcgtcattacccagggccacatccttggccaattgcaagccatcaacaaagcccgccaagagtttctgctacgaaagggacggggggtttacctggacccccagtccggcgaggagctcaacccaatccccccgccgccgcagccctatcagcagccgcgggcccttgcttcccaggatggcacccaaaaagaagctgcagctgccgccgccgccacccacggacgaggaggaatactgggacagtcaggcagaggaggttttggacgaggaggaggagatgatggaagactgggacagcctagacgaagcttccgaggccgaagaggtgtcagacgaaacaccgtcaccctcggtcgcattcccctcgccggcgccccagaaattggcaaccgttcccagcatcgctacaacctccgctcctcaggcgccgccggcactgcctgttcgccgacccaaccgtagatgggacaccactggaaccagggccggtaagtctaagcagccgccgccgttagcccaagagcaacaacagcgccaaggctaccgctcgtggcgcgggcacaagaacgccatagttgcttgcttgcaagactgtgggggcaacatctccttcgcccgccgctttcttctctaccatcacggcgtggccttcccccgtaacatcctgcattactaccgtcatctctacagcccctactgcaccggcggcagcggcagcggcagcaacagcagcggtcacacagaagcaaaggcgaccggatagcaagactctgacaaagcccaagaaatccacagcggcggcagcagcaggaggaggagcgctgcgtctggcgcccaacgaacccgtatcgacccgcgagcttagaaataggatttttcccactctgtatgctatatttcaacaaagcaggggccaagaacaagagctgaaaataaaaaacaggtctctgcgctccctcacccgcagctgcctgtatcacaaaagcgaagatcagcttcggcgcacgctggaagacgcggaggctctcttcagcaaatactgcgcgctgactcttaaggactagtttcgcgccctttctcaaatttaagcgcgaaaactacgtcatctccagcggccacacccggcgccagcacctgtcgtcagcgccattatgagcaaggaaattcccacgccctacatgtggagttaccagccacaaatgggacttgcggctggagctgcccaagactactcaacccgaataaactacatgagcgcgggaccccacatgatatcccgggtcaacggaatccgcgcccaccgaaaccgaattctcctcgaacaggcggctattaccaccacacctcgtaataaccttaatccccgtagttggcccgctgccctggtgtaccaggaaagtcccgctcccaccactgtggtacttcccagagacgcccaggccgaagttcagatgactaactcaggggcgcagcttgcgggcggctttcgtcacagggtgcggtcgcccgggcgttttagggcggagtaacttgcatgtattgggaattgtagtttttttaaaatgggaagtgacgtatcgtgggaaaacggaagtgaagatttgaggaagttgtgggttttttggctttcgtttctgggcgtaggttcgcgtgcggttttctgggtgttttttgtggactttaaccgttacgtcattttttagtcctatatatactcgctctgtacttggccctttttacactgtgactgattgagctggtgccgtgtcgagtggtgttttttaataggtttttttactggtaaggctgactgttatggctgccgctgtggaagcgctgtatgttgttctggagcgggagggtgctattttgcctaggcaggagggtttttcaggtgtttatgtgtttttctctcctattaattttgttatacctcctatgggggctgtaatgttgtctctacgcctgcgggtatgtattcccccgggctatttcggtcgctttttagcactgaccgatgttaaccaacctgatgtgtttaccgagtcttacattatgactccggacatgaccgaggaactgtcggtggtgctttttaatcacggtgaccagtttttttacggtcacgccggcatggccgtagtccgtcttatgcttataagggttgtttttcctgttgtaagacaggcttctaatgtttaaatgtttttttttttgttattttattttgtgtttaatgcaggaacccgcagacatgtttgagagaaaaatggtgtctttttctgtggtggttccggaacttacctgcctttatctgcatgagcatgactacgatgtgcttgcttttttgcgcgaggctttgcctgattttttgagcagcaccttgcattttatatcgccgcccatgcaacaagcttacataggggctacgctggttagcatagctccgagtatgcgtgtcataatcagtgtgggttcttttgtcatggttcctggcggggaagtggccgcgctggtccgtgcagacctgcacgattatgttcagctggccctgcgaagggacctacgggatcgcggtatttttgttaatgttccgcttttgaatcttatacaggtctgtgaggaacctgaatttttgcaatcatgattcgctgcttgaggctgaaggtggagggcgctctggagcagatttttacaatggccggacttaatattcgggatttgcttagagacatattgataaggtggcgagatgaaaattatttgggcatggttgaaggtgctggaatgtttatagaggagattcaccctgaagggtttagcctttacgtccacttggacgtgagggcagtttgccttttggaagccattgtgcaacatcttacaaatgccattatctgttctttggctgtagagtttgaccacgccaccggaggggagcgcgttcacttaatagatcttcattttgaggttttggataatcttttggaataaaaaaaaaaaaacatggttcttccagctcttcccgctcctcccgtgtgtgactcgcagaacgaatgtgtaggttggctgggtgtggcttattctgcggtggtggatgttatcagggcagcggcgcatgaaggagtttacatagaacccgaagccagggggcgcctggatgctttgagagagtggatatactacaactactacacagagcgagctaagcgacgagaccggagacgcagatctgtttgtcacgcccgcacctggttttgcttcaggaaatatgactacgtccggcgttccatttggcatgacactacgaccaacacgatctcggttgtctcggcgcactccgtacagtagggatcgcctacctccttttgagacagagacccgcgctaccatactggaggatcatccgctgctgcccgaatgtaacactttgacaatgcacaacgtgagttacgtgcgaggtcttccctgcagtgtgggatttacgctgattcaggaatgggttgttccctgggatatggttctgacgcgggaggagcttgtaatcctgaggaagtgtatgcacgtgtgcctgtgttgtgccaacattgatatcatgacgagcatgatgatccatggttacgagtcctgggctctccactgtcattgttccagtcccggttccctgcagtgcatagccggcgggcaggttttggccagctggtttaggatggtggtggatggcgccatgtttaatcagaggtttatatggtaccgggaggtggtgaattacaacatgccaaaagaggtaatgtttatgtccagcgtgtttatgaggggtcgccacttaatctacctgcgcttgtggtatgatggccacgtgggttctgtggtccccgccatgagctttggatacagcgccttgcactgtgggattttgaacaatattgtggtgctgtgctgcagttactgtgctgatttaagtgagatcagggtgcgctgctgtgcccggaggacaaggcgtctcatgctgcgggcggtgcgaatcatcgctgaggagaccactgccatgttgtattcctgcaggacggagcggcggcggcagcagtttattcgcgcgctgctgcagcaccaccgccctatcctgatgcacgattatgactctacccccatgtaggcgtggacttccccttcgccgcccgttgagcaaccgcaagttggacagcagcctgtggctcagcagctggacagcgacatgaacttaagcgagctgcccggggagtttattaatatcactgatgagcgtttggctcgacaggaaaccgtgtggaatataacacctaagaatatgtctgttacccatgatatgatgctttttaaggccagccggggagaaaggactgtgtactctgtgtgttgggagggaggtggcaggttgaatactagggttctgtgagtttgattaaggtacggtgatcaatataagctatgtggtggtggggctatactactgaatgaaaaatgacttgaaattttctgcaattgaaaaataaacacgttgaaacataacatgcaacaggttcacgattctttattcctgggcaatgtaggagaaggtgtaagagttggtagcaaaagtttcagtggtgtattttccactttcccaggaccatgtaaaagacatagagtaagtgcttacctcgctagtttctgtggattcactagaatcgatgtaggatgttgcccctcctgacgcggtaggagaaggggagggtgccctgcatgtctgccgctgctcttgctcttgccgctgctgaggaggggggcgcatctgccgcagcaccggatgcatctgggaaaagcaaaaaaggggctcgtccctgtttccggaggaatttgcaagcggggtcttgcatgacggggaggcaaacccccgttcgccgcagtccggccggcccgagactcgaaccgggggtcctgcgactcaacccttggaaaataaccctccggctacagggagcgagccacttaatgctttcgctttccagcctaaccgcttacgccgcgcgcggccagtggccaaaaaagctagcgcagcagccgccgcgcctggaaggaagccaaaaggagcgctcccccgttgtctgacgtcgcacacctgggttcgacacgcgggcggtaaccgcatggatcacggcggacggccggatccggggttcgaaccccggtcgtccgccatgatacccttgcgaatttatccaccagaccacggaagagtgcccgcttacaggctctccttttgcacggtctagagcgtcaacgactgcgcacgcctcaccggccagagcgtcccgaccatggagcactttttgccgctgcgcaacatctggaaccgcgtccgcgactttccgcgcgcctccaccaccgccgccggcatcacctggatgtccaggtacatctacggattacgtcgacgtttaaaccatatgatcagctcactcaaaggcggtaatacggttatccacagaatcaggggataacgcaggaaagaacatgtgagcaaaaggccagcaaaaggccaggaaccgtaaaaaggccgcgttgctggcgtttttccataggctccgcccccctgacgagcatcacaaaaatcgacgctcaagtcagaggtggcgaaacccgacaggactataaagataccaggcgtttccccctggaagctccctcgtgcgctctcctgttccgaccctgccgcttaccggatacctgtccgcctttctcccttcgggaagcgtggcgctttctcatagctcacgctgtaggtatctcagttcggtgtaggtcgttcgctccaagctgggctgtgtgcacgaaccccccgttcagcccgaccgctgcgccttatccggtaactatcgtcttgagtccaacccggtaagacacgacttatcgccactggcagcagccactggtaacaggattagcagagcgaggtatgtaggcggtgctacagagttcttgaagtggtggcctaactacggctacactagaagaacagtatttggtatctgcgctctgctgaagccagttaccttcggaaaaagagttggtagctcttgatccggcaaacaaaccaccgctggtagcggtggtttttttgtttgcaagcagcagattacgcgcagaaaaaaaggatctcaagaagatcctttgatcttttctacggggtctgacgctcagtggaacgaaaactcacgttaagggattttggtcatgagattatcaaaaaggatcttcacctagatccttttaaattaaaaatgaagttttaaatcaatctaaagtatatatgagtaaacttggtctgacagttaccaatgcttaatcagtgaggcacctatctcagcgatctgtctatttcgttcatccatagttgcctgactccccgtcgtgtagataactacgatacgggagggcttaccatctggccccagtgctgcaatgataccgcgagacccacgctcaccggctccagatttatcagcaataaaccagccagccggaagggccgagcgcagaagtggtcctgcaactttatccgcctccatccagtctattaattgttgccgggaagctagagtaagtagttcgccagttaatagtttgcgcaacgttgttgccattgctacaggcatcgtggtgtcacgctcgtcgtttggtatggcttcattcagctccggttcccaacgatcaaggcgagttacatgatcccccatgttgtgcaaaaaagcggttagctccttcggtcctccgatcgttgtcagaagtaagttggccgcagtgttatcactcatggttatggcagcactgcataattctcttactgtcatgccatccgtaagatgcttttctgtgactggtgagtactcaaccaagtcattctgagaatagtgtatgcggcgaccgagttgctcttgcccggcgtcaatacgggataataccgcgccacatagcagaactttaaaagtgctcatcattggaaaacgttcttcggggcgaaaactctcaaggatcttaccgctgttgagatccagttcgatgtaacccactcgtgcacccaactgatcttcagcatcttttactttcaccagcgtttctgggtgagcaaaaacaggaaggcaaaatgccgcaaaaaagggaataagggcgacacggaaatgttgaatactcatactcttcctttttcaatattattgaagcatttatcagggttattgtctcatgagcggatacatatttgaatgtatttagaaaaataaacaaataggggttccgcgcacatttccccgaaaagtgccacctaaattgtaagcgttaatattttgttaaaattcgcgttaaatttttgttaaatcagctcattttttaaccaataggccgaaatcggcaaaatcccttataaatcaaaagaatagaccgagatagggttgagtgttgttccagtttggaacaagagtccactattaaagaacgtggactccaacgtcaaagggcgaaaaaccgtctatcagggcgatggcccactacgtgaaccatcaccctaatcaagttttttggggtcgaggtgccgtaaagcactaaatcggaaccctaaagggagcccccgatttagagcttgacggggaaagccggcgaacgtggcgagaaaggaagggaagaaagcgaaaggagcgggcgctagggcgctggcaagtgtagcggtcacgctgcgcgtaaccaccacacccgccgcgcttaatgcgccgctacagggcgcgatggatcc

SEQ ID NO: 2 - DNA, 7294 bp, Artificial Sequence
  plasmid
gcgcgccgatatcgttaacgccccgcgccggccgctctagaactagtggatcccccggaagatcagaagttcctattccgaagttcctattctctagaaagtataggaacttctgatctgcgcagccgccatgccggggttttacgagattgtgattaaggtccccagcgaccttgacgagcatctgcccggcatttctgacagctttgtgaactgggtggccgagaaggaatgggagttgccgccagattctgacatggatctgaatctgattgagcaggcacccctgaccgtggccgagaagctgcagcgcgactttctgacggaatggcgccgtgtgagtaaggccccggaggcccttttctttgtgcaatttgagaagggagagagctacttccacatgcacgtgctcgtggaaaccaccggggtgaaatccatggttttgggacgtttcctgagtcagattcgcgaaaaactgattcagagaatttaccgcgggatcgagccgactttgccaaactggttcgcggtcacaaagaccagaaatggcgccggaggcgggaacaaggtggtggatgagtgctacatccccaattacttgctccccaaaacccagcctgagctccagtgggcgtggactaatatggaacagtatttaagcgcctgtttgaatctcacggagcgtaaacggttggtggcgcagcatctgacgcacgtgtcgcagacgcaggagcagaacaaagagaatcagaatcccaattctgatgcgccggtgatcagatcaaaaacttcagccaggtacatggagctggtcgggtggctcgtggacaaggggattacctcggagaagcagtggatccaggaggaccaggcctcatacatctccttcaatgcggcctccaactcgcggtcccaaatcaaggctgccttggacaatgcgggaaagattatgagcctgactaaaaccgcccccgactacctggtgggccagcagcccgtggaggacatttccagcaatcggatttataaaattttggaactaaacgggtacgatccccaatatgcggcttccgtctttctgggatgggccacgaaaaagttcggcaagaggaacaccatctggctgtttgggcctgcaactaccgggaagaccaacatcgcggaggccatagcccacactgtgcccttctacgggtgcgtaaactggaccaatgagaactttcccttcaacgactgtgtcgacaagatggtgatctggtgggaggaggggaagatgaccgccaaggtcgtggagtcggccaaagccattctcggaggaagcaaggtgcgcgtggaccagaaatgcaagtcctcggcccagatagacccgactcccgtgatcgtcacctccaacaccaacatgtgcgccgtgattgacgggaactcaacgaccttcgaacaccagcagccgttgcaagaccggatgttcaaatttgaactcacccgccgtctggatcatgactttgggaaggtcaccaagcaggaagtcaaagactttttccggtgggcaaaggatcacgtggttgaggtggagcatgaattctacgtcaaaaagggtggagccaagaaaagacccgcccccagtgacgcagatataagtgagcccaaacgggtgcgcgagtcagttgcgcagccatcgacgtcagacgcggaagcttcgatcaactacgcagacaggtaccaaaacaaatgttctcgtcacgtgggcatgaatctgatgctgtttccctgcagacaatgcgagagaatgaatcagaattcaaatatctgcttcactcacggacagaaagactgtttagagtgctttcccgtgtcagaatctcaacccgtttctgtcgtcaaaaaggcgtatcagaaactgtgctacattcatcatatcatgggaaaggtgccagacgcttgcactgcctgcgatctggtcaatgtggatttggatgactgcatctttgaacaataaatgatttaaatcaggtatgtcttttgttgatcaccctccagattggttggaagaagttggtgaaggtcttcgcgagtttttgggccttgaagcgggcccaccgaaaccaaaacccaatcagcagcatcaagatcaagcccgtggtcttgtgctgcctggttataactatctcggacccggaaacggtctcgatcgaggagagcctgtcaacagggcagacgaggtcgcgcgagagcacgacatctcgtacaacgagcagcttgaggcgggagacaacccctacctcaagtacaaccacgcggacgccgagtttcaggagaagctcgccgacgacacatccttcgggggaaacctcggaaaggcagtctttcaggccaagaaaagggttctcgaaccttttggcctggttgaagagggtgctaagacggcccctaccggaaagcggatagacgaccactttccaaaaagaaagaaggctcggaccgaagaggactccaagccttccacctcgtcagacgccgaagctggacccagcggatcccagcagctgcaaatcccagcccaaccagcctcaagtttgggagctgatacaatgtctgcgggaggtggcggcccattgggcgacaataaccaaggtgccgatggagtgggcaatgcctcgggagattggcattgcgattccacgtggatgggggacagagtcgtcaccaagtccacccgaacctgggtgctgcccagctacaacaaccaccagtaccgagagatcaaaagcggctccgtcgacggaagcaacgccaacgcctactttggatacagcaccccctgggggtactttgactttaaccgcttccacagccactggagcccccgagactggcaaagactcatcaacaactactggggcttcagaccccggtccctcagagtcaaaatcttcaacattcaagtcaaagaggtcacggtgcaggactccaccaccaccatcgccaacaacctcacctccaccgtccaagtgtttacggacgacgactaccagctgccctacgtcgtcggcaacgggaccgagggatgcctgccggccttccctccgcaggtctttacgctgccgcagtacggttacgcgacgctgaaccgcgacaacacagaaaatcccaccgagaggagcagcttcttctgcctagagtactttcccagcaagatgctgagaacgggcaacaactttgagtttacctacaactttgaggaggtgcccttccactccagcttcgctcccagtcagaacctgttcaagctggccaacccgctggtggaccagtacttgtaccgcttcgtgagcacaaataacactggcggagtccagttcaacaagaacctggccgggagatacgccaacacctacaaaaactggttcccggggcccatgggccgaacccagggctggaacctgggctccggggtcaaccgcgccagtgtcagcgccttcgccacgaccaataggatggagctcgagggcgcgagttaccaggtgcccccgcagccgaacggcatgaccaacaacctccagggcagcaacacctatgccctggagaacactatgatcttcaacagccagccggcgaacccgggcaccaccgccacgtacctcgagggcaacatgctcatcaccagcgagagcgagacgcagccggtgaaccgcgtggcgtacaacgtcggcgggcagatggccaccaacaaccagagctccaccactgcccccgcgaccggcacgtacaacctccaggaaatcgtgcccggcagcgtgtggatggagagggacgtgtacctccaaggacccatctgggccaagatcccagagacgggggcgcactttcacccctctccggccatgggcggattcggactcaaacacccaccgcccatgatgctcatcaagaacacgcctgtgcccggaaatatcaccagcttctcggacgtgcccgtcagcagcttcatcacccagtacagcaccgggcaggtcaccgtggagatggagtgggagctcaagaaggaaaactccaagaggtggaacccagagatccagtacacaaacaactacaacgacccccagtttgtggactttgccccggacagcaccggggaatacagaaccaccagacctatcggaacccgataccttacccgacccctttaattgcttgttaatcaataaaccgtttaattcgtttcagttgaactttggtctctgcgtatttctttcttatctagtttccatggctacgtagataagtagcatggcgggttaatcattaactacagcccgggcgtttaaacagcgggcggaggggtggagtcgtgacgtgaattacgtcatagggttagggaggtcctgtattagaggtcacgtgagtgttttgcgacattttgcgacaccatgtggtctcgctgggggggggggcccgagtgagcacgcagggtctccattttgaagcgggaggtttgaacgagcgctggcgcgctcactggccgtcgttttacaacgtcgtgactgggaaaaccctggcgttacccaacttaatcgccttgcagcacatccccctttcgccagctggcgtaatagcgaagaggcccgcaccgatcgcccttcccaacagttgcgcagcctgaatggcgaatggaaattgtaagcgttaatattttgttaaaattcgcgttaaatttttgttaaatcagctcatttttttaaccaataggccgaaatcggcaaaatcccttataaatcaaaagaatagaccgagatagggttgagtgttgttccagtttggaacaagagtccactattaagaacgtggactccaacgtcaaagggcgaaaaaccgtctatcagggcgatggcccactacgtgaaccatcaccctaatcaagttttttggggtcgaggtgccgtaaagcactaaatcggaaccctaaagggagcccccgatttagagcttgacggggaaagccggcgaacgtggcgagaaaggaagggaagaaagcgaaaggagcgggcgctagggcgctggcaagtgtagcggtcacgctgcgcgtaaccaccacacccgccgcgcttaatgcgccgctacagggcgcgtcaggtggcacttttcggggaaatgtgcgcggaacccctatttgtttatttttctaaatacattcaaatatgtatccgctcatgagacaataaccctgataaatgcttcaataatattgaaaaaggaagagtatgagtattcaacatttccgtgtcgcccttattcccttttttgcggcattttgccttcctgtttttgctcacccagaaacgctggtgaaagtaaaagatgctgaagatcagttgggtgcacgagtgggttacatcgaactggatctcaacagcggtaagatccttgagagttttcgccccgaagaacgttttccaatgatgagcacttttaaagttctgctatgtggcgcggtattatcccgtattgacgccgggcaagagcaactcggtcgccgcatacactattctcagaatgacttggttgagtactcaccagtcacagaaaagcatcttacggatggcatgacagtaagagaattatgcagtgctgccataaccatgagtgataacactgcggccaacttacttctgacaacgatcggaggaccgaaggagctaaccgcttttttgcacaacatgggggatcatgtaactcgccttgatcgttgggaaccggagctgaatgaagccataccaaacgacgagcgtgacaccacgatgcctgtagcaatggcaacaacgttgcgcaaactattaactggcgaactacttactctagcttcccggcaacaattaatagactggatggaggcggataaagttgcaggaccacttctgcgctcggcccttccggctggctggtttattgctgataaatctggagccggtgagcgtgggtctcgcggtatcattgcagcactggggccagatggtaagccctcccgtatcgtagttatctacacgacggggagtcaggcaactatggatgaacgaaatagacagatcgctgagataggtgcctcactgattaagcattggtaactgtcagaccaagtttactcatatatactttagattgatttaaaacttcatttttaatttaaaaggatctaggtgaagatcctttttgataatctcatgaccaaaatcccttaacgtgagttttcgttccactgagcgtcagaccccgtagaaaagatcaaaggatcttcttgagatcctttttttctgcgcgtaatctgctgcttgcaaacaaaaaaaccaccgctaccagcggtggtttgtttgccggatcaagagctaccaactctttttccgaaggtaactggcttcagcagagcgcagataccaaatactgttcttctagtgtagccgtagttaggccaccacttcaagaactctgtagcaccgcctacatacctcgctctgctaatcctgttaccagtggctgctgccagtggcgataagtcgtgtcttaccgggttggactcaagacgatagttaccggataaggcgcagcggtcgggctgaacggggggttcgtgcacacagcccagcttggagcgaacgacctacaccgaactgagatacctacagcgtgagctatgagaaagcgccacgcttcccgaagggagaaaggcggacaggtatccggtaagcggcagggtcggaacaggagagcgcacgagggagcttccagggggaaacgcctggtatctttatagtcctgtcgggtttcgccacctctgacttgagcgtcgatttttgtgatgctcgtcaggggggcggagcctatggaaaaacgccagcaacgcggcctttttacggttcctggccttttgctggccttttgctcacatgttctttcctgcgttatcccctgattctgtggataaccgtattaccgcctttgagtgagctgataccgctcgccgcagccgaacgaccgagcgcagcgagtcagtgagcgaggaagcggaagagcgcccaatacgcaaaccgcctctccccgcgcgttggccgattcattaatgcagctggcacgacaggtttcccgactggaaagcgggcagtgagcgcaacgcaattaatgtgagttagctcactcattaggcaccccaggctttacactttatgcttccggctcgtatgttgtgtggaattgtgagcggataacaatttcacacaggaaacagctatgaccatgattacgccaa

SEQ ID NO: 3 - DNA, 5952 bp, Artificial Sequence
  plasmid
gcgcgccgatatcgttaacgccccgcgccggccgctctagaactagtggatcccccggaagatcagaagttcctattccgaagttcctattctctagaaagtataggaacttctgatctgcgcagccgccgcggccgcacccgccgtctggatcatgactttgggaaggtcaccaagcaggaagtcaaagactttttccggtgggcaaaggatcacgtggttgaggtggagcatgaattctacgtcaaaaagggtggagccaagaaaagacccgcccccagtgacgcagatataagtgagcccaaacgggtgcgcgagtcagttgcgcagccatcgacgtcagacgcggaagcttcgatcaactacgcagacaggtaccaaaacaaatgttctcgtcacgtgggcatgaatctgatgctgtttccctgcagacaatgcgagagaatgaatcagaattcaaatatctgcttcactcacggacagaaagactgtttagagtgctttcccgtgtcagaatctcaacccgtttctgtcgtcaaaaaggcgtatcagaaactgtgctacattcatcatatcatgggaaaggtgccagacgcttgcactgcctgcgatctggtcaatgtggatttggatgactgcatctttgaacaataaatgatttaaatcaggtatgtcttttgttgatcaccctccagattggttggaagaagttggtgaaggtcttcgcgagtttttgggccttgaagcgggcccaccgaaaccaaaacccaatcagcagcatcaagatcaagcccgtggtcttgtgctgcctggttataactatctcggacccggaaacggtctcgatcgaggagagcctgtcaacagggcagacgaggtcgcgcgagagcacgacatctcgtacaacgagcagcttgaggcgggagacaacccctacctcaagtacaaccacgcggacgccgagtttcaggagaagctcgccgacgacacatccttcgggggaaacctcggaaaggcagtctttcaggccaagaaaagggttctcgaaccttttggcctggttgaagagggtgctaagacggcccctaccggaaagcggatagacgaccactttccaaaaagaaagaaggctcggaccgaagaggactccaagccttccacctcgtcagacgccgaagctggacccagcggatcccagcagctgcaaatcccagcccaaccagcctcaagtttgggagctgatacaatgtctgcgggaggtggcggcccattgggcgacaataaccaaggtgccgatggagtgggcaatgcctcgggagattggcattgcgattccacgtggatgggggacagagtcgtcaccaagtccacccgaacctgggtgctgcccagctacaacaaccaccagtaccgagagatcaaaagcggctccgtcgacggaagcaacgccaacgcctactttggatacagcaccccctgggggtactttgactttaaccgcttccacagccactggagcccccgagactggcaaagactcatcaacaactactggggcttcagaccccggtccctcagagtcaaaatcttcaacattcaagtcaaagaggtcacggtgcaggactccaccaccaccatcgccaacaacctcacctccaccgtccaagtgtttacggacgacgactaccagctgccctacgtcgtcggcaacgggaccgagggatgcctgccggccttccctccgcaggtctttacgctgccgcagtacggttacgcgacgctgaaccgcgacaacacagaaaatcccaccgagaggagcagcttcttctgcctagagtactttcccagcaagatgctgagaacgggcaacaactttgagtttacctacaactttgaggaggtgcccttccactccagcttcgctcccagtcagaacctgttcaagctggccaacccgctggtggaccagtacttgtaccgcttcgtgagcacaaataacactggcggagtccagttcaacaagaacctggccgggagatacgccaacacctacaaaaactggttcccggggcccatgggccgaacccagggctggaacctgggctccggggtcaaccgcgccagtgtcagcgccttcgccacgaccaataggatggagctcgagggcgcgagttaccaggtgcccccgcagccgaacggcatgaccaacaacctccagggcagcaacacctatgccctggagaacactatgatcttcaacagccagccggcgaacccgggcaccaccgccacgtacctcgagggcaacatgctcatcaccagcgagagcgagacgcagccggtgaaccgcgtggcgtacaacgtcggcgggcagatggccaccaacaaccagagctccaccactgcccccgcgaccggcacgtacaacctccaggaaatcgtgcccggcagcgtgtggatggagagggacgtgtacctccaaggacccatctgggccaagatcccagagacgggggcgcactttcacccctctccggccatgggcggattcggactcaaacacccaccgcccatgatgctcatcaagaacacgcctgtgcccggaaatatcaccagcttctcggacgtgcccgtcagcagcttcatcacccagtacagcaccgggcaggtcaccgtggagatggagtgggagctcaagaaggaaaactccaagaggtggaacccagagatccagtacacaaacaactacaacgacccccagtttgtggactttgccccggacagcaccggggaatacagaaccaccagacctatcggaacccgataccttacccgacccctttaattgcttgttaatcaataaaccgtttaattcgtttcagttgaactttggtctctgcgtatttctttcttatctagtttccatggctacgtagataagtagcatggcgggttaatcattaactacagcccgggcgtttaaacagcgggcggaggggtggagtcgtgacgtgaattacgtcatagggttagggaggtcctgtattagaggtcacgtgagtgttttgcgacattttgcgacaccatgtggtctcgctgggggggggggcccgagtgagcacgcagggtctccattttgaagcgggaggtttgaacgagcgctggcgcgctcactggccgtcgttttacaacgtcgtgactgggaaaaccctggcgttacccaacttaatcgccttgcagcacatccccctttcgccagctggcgtaatagcgaagaggcccgcaccgatcgcccttcccaacagttgcgcagcctgaatggcgaatggaaattgtaagcgttaatattttgttaaaattcgcgttaaatttttgttaaatcagctcatttttttaaccaataggccgaaatcggcaaaatcccttataaatcaaaagaatagaccgagatagggttgagtgttgttccagtttggaacaagagtccactattaagaacgtggactccaacgtcaaagggcgaaaaaccgtctatcagggcgatggcccactacgtgaaccatcaccctaatcaagttttttggggtcgaggtgccgtaaagcactaaatcggaaccctaaagggagcccccgatttagagcttgacggggaaagccggcgaacgtggcgagaaaggaagggaagaaagcgaaaggagcgggcgctagggcgctggcaagtgtagcggtcacgctgcgcgtaaccaccacacccgccgcgcttaatgcgccgctacagggcgcgtcaggtggcacttttcggggaaatgtgcgcggaacccctatttgtttatttttctaaatacattcaaatatgtatccgctcatgagacaataaccctgataaatgcttcaataatattgaaaaaggaagagtatgagtattcaacatttccgtgtcgcccttattcccttttttgcggcattttgccttcctgtttttgctcacccagaaacgctggtgaaagtaaaagatgctgaagatcagttgggtgcacgagtgggttacatcgaactggatctcaacagcggtaagatccttgagagttttcgccccgaagaacgttttccaatgatgagcacttttaaagttctgctatgtggcgcggtattatcccgtattgacgccgggcaagagcaactcggtcgccgcatacactattctcagaatgacttggttgagtactcaccagtcacagaaaagcatcttacggatggcatgacagtaagagaattatgcagtgctgccataaccatgagtgataacactgcggccaacttacttctgacaacgatcggaggaccgaaggagctaaccgcttttttgcacaacatgggggatcatgtaactcgccttgatcgttgggaaccggagctgaatgaagccataccaaacgacgagcgtgacaccacgatgcctgtagcaatggcaacaacgttgcgcaaactattaactggcgaactacttactctagcttcccggcaacaattaatagactggatggaggcggataaagttgcaggaccacttctgcgctcggcccttccggctggctggtttattgctgataaatctggagccggtgagcgtgggtctcgcggtatcattgcagcactggggccagatggtaagccctcccgtatcgtagttatctacacgacggggagtcaggcaactatggatgaacgaaatagacagatcgctgagataggtgcctcactgattaagcattggtaactgtcagaccaagtttactcatatatactttagattgatttaaaacttcatttttaatttaaaaggatctaggtgaagatcctttttgataatctcatgaccaaaatcccttaacgtgagttttcgttccactgagcgtcagaccccgtagaaaagatcaaaggatcttcttgagatcctttttttctgcgcgtaatctgctgcttgcaaacaaaaaaaccaccgctaccagcggtggtttgtttgccggatcaagagctaccaactctttttccgaaggtaactggcttcagcagagcgcagataccaaatactgttcttctagtgtagccgtagttaggccaccacttcaagaactctgtagcaccgcctacatacctcgctctgctaatcctgttaccagtggctgctgccagtggcgataagtcgtgtcttaccgggttggactcaagacgatagttaccggataaggcgcagcggtcgggctgaacggggggttcgtgcacacagcccagcttggagcgaacgacctacaccgaactgagatacctacagcgtgagctatgagaaagcgccacgcttcccgaagggagaaaggcggacaggtatccggtaagcggcagggtcggaacaggagagcgcacgagggagcttccagggggaaacgcctggtatctttatagtcctgtcgggtttcgccacctctgacttgagcgtcgatttttgtgatgctcgtcaggggggcggagcctatggaaaaacgccagcaacgcggcctttttacggttcctggccttttgctggccttttgctcacatgttctttcctgcgttatcccctgattctgtggataaccgtattaccgcctttgagtgagctgataccgctcgccgcagccgaacgaccgagcgcagcgagtcagtgagcgaggaagcggaagagcgcccaatacgcaaaccgcctctccccgcgcgttggccgattcattaatgcagctggcacgacaggtttcccgactggaaagcgggcagtgagcgcaacgcaattaatgtgagttagctcactcattaggcaccccaggctttacactttatgcttccggctcgtatgttgtgtggaattgtgagcggataacaatttcacacaggaaacagctatgaccatgattacgccaa

SEQ ID NO: 4 - DNA, 5127 bp, Artificial Sequence
  plasmid
gcgcgccgatatcgttaacgccccgcgccggccgctctagaactagtggatcccccggaagatcagaagttcctattccgaagttcctattctctagaaagtataggaacttctgatctgcgcagccgccatgccggggttttacgagattgtgattaaggtccccagcgaccttgacgagcatctgcccggcatttctgacagctttgtgaactgggtggccgagaaggaatgggagttgccgccagattctgacatggatctgaatctgattgagcaggcacccctgaccgtggccgagaagctgcagcgcgactttctgacggaatggcgccgtgtgagtaaggccccggaggcccttttctttgtgcaatttgagaagggagagagctacttccacatgcacgtgctcgtggaaaccaccggggtgaaatccatggttttgggacgtttcctgagtcagattcgcgaaaaactgattcagagaatttaccgcgggatcgagccgactttgccaaactggttcgcggtcacaaagaccagaaatggcgccggaggcgggaacaaggtggtggatgagtgctacatccccaattacttgctccccaaaacccagcctgagctccagtgggcgtggactaatatggaacagtatttaagcgcctgtttgaatctcacggagcgtaaacggttggtggcgcagcatctgacgcacgtgtcgcagacgcaggagcagaacaaagagaatcagaatcccaattctgatgcgccggtgatcagatcaaaaacttcagccaggtacatggagctggtcgggtggctcgtggacaaggggattacctcggagaagcagtggatccaggaggaccaggcctcatacatctccttcaatgcggcctccaactcgcggtcccaaatcaaggctgccttggacaatgcgggaaagattatgagcctgactaaaaccgcccccgactacctggtgggccagcagcccgtggaggacatttccagcaatcggatttataaaattttggaactaaacgggtacgatccccaatatgcggcttccgtctttctgggatgggccacgaaaaagttcggcaagaggaacaccatctggctgtttgggcctgcaactaccgggaagaccaacatcgcggaggccatagcccacactgtgcccttctacgggtgcgtaaactggaccaatgagaactttcccttcaacgactgtgtcgacaagatggtgatctggtgggaggaggggaagatgaccgccaaggtcgtggagtcggccaaagccattctcggaggaagcaaggtgcgcgtggaccagaaatgcaagtcctcggcccagatagacccgactcccgtgatcgtcacctccaacaccaacatgtgcgccgtgattgacgggaactcaacgaccttcgaacaccagcagccgttgcaagaccggatgttcaaatttgaactcacccgccgtctggatcatgactttgggaaggtcaccaagcaggaagtcaaagactttttccggtgggcaaaggatcacgtggttgaggtggagcatgaattctacgtcaaaaagggtggagccaagaaaagacccgcccccagtgacgcagatataagtgagcccaaacgggtgcgcgagtcagttgcgcagccatcgacgtcagacgcggaagcttcgatcaactacgcagacaggtaccaaaacaaatgttctcgtcacgtgggcatgaatctgatgctgtttccctgcagacaatgcgagagaatgaatcagaattcaaatatctgcttcactcacggacagaaagactgtttagagtgctttcccgtgtcagaatctcaacccgtttctgtcgtcaaaaaggcgtatcagaaactgtgctacattcatcatatcatgggaaaggtgccagacgcttgcactgcctgcgatctggtcaatgtggatttggatgactgcatctttgaacaataaatgatttaaatcaggtgcggccgcttgcttgttaatcaataaaccgtttaattcgtttcagttgaactttggtctctgcgtatttctttcttatctagtttccatggctacgtagataagtagcatggcgggttaatcattaactacagcccgggcgtttaaacagcgggcggaggggtggagtcgtgacgtgaattacgtcatagggttagggaggtcctgtattagaggtcacgtgagtgttttgcgacattttgcgacaccatgtggtctcgctgggggggggggcccgagtgagcacgcagggtctccattttgaagcgggaggtttgaacgagcgctggcgcgctcactggccgtcgttttacaacgtcgtgactgggaaaaccctggcgttacccaacttaatcgccttgcagcacatccccctttcgccagctggcgtaatagcgaagaggcccgcaccgatcgcccttcccaacagttgcgcagcctgaatggcgaatggaaattgtaagcgttaatattttgttaaaattcgcgttaaatttttgttaaatcagctcatttttttaaccaataggccgaaatcggcaaaatcccttataaatcaaaagaatagaccgagatagggttgagtgttgttccagtttggaacaagagtccactattaagaacgtggactccaacgtcaaagggcgaaaaaccgtctatcagggcgatggcccactacgtgaaccatcaccctaatcaagttttttggggtcgaggtgccgtaaagcactaaatcggaaccctaaagggagcccccgatttagagcttgacggggaaagccggcgaacgtggcgagaaaggaagggaagaaagcgaaaggagcgggcgctagggcgctggcaagtgtagcggtcacgctgcgcgtaaccaccacacccgccgcgcttaatgcgccgctacagggcgcgtcaggtggcacttttcggggaaatgtgcgcggaacccctatttgtttatttttctaaatacattcaaatatgtatccgctcatgagacaataaccctgataaatgcttcaataatattgaaaaaggaagagtatgagtattcaacatttccgtgtcgcccttattcccttttttgcggcattttgccttcctgtttttgctcacccagaaacgctggtgaaagtaaaagatgctgaagatcagttgggtgcacgagtgggttacatcgaactggatctcaacagcggtaagatccttgagagttttcgccccgaagaacgttttccaatgatgagcacttttaaagttctgctatgtggcgcggtattatcccgtattgacgccgggcaagagcaactcggtcgccgcatacactattctcagaatgacttggttgagtactcaccagtcacagaaaagcatcttacggatggcatgacagtaagagaattatgcagtgctgccataaccatgagtgataacactgcggccaacttacttctgacaacgatcggaggaccgaaggagctaaccgcttttttgcacaacatgggggatcatgtaactcgccttgatcgttgggaaccggagctgaatgaagccataccaaacgacgagcgtgacaccacgatgcctgtagcaatggcaacaacgttgcgcaaactattaactggcgaactacttactctagcttcccggcaacaattaatagactggatggaggcggataaagttgcaggaccacttctgcgctcggcccttccggctggctggtttattgctgataaatctggagccggtgagcgtgggtctcgcggtatcattgcagcactggggccagatggtaagccctcccgtatcgtagttatctacacgacggggagtcaggcaactatggatgaacgaaatagacagatcgctgagataggtgcctcactgattaagcattggtaactgtcagaccaagtttactcatatatactttagattgatttaaaacttcatttttaatttaaaaggatctaggtgaagatcctttttgataatctcatgaccaaaatcccttaacgtgagttttcgttccactgagcgtcagaccccgtagaaaagatcaaaggatcttcttgagatcctttttttctgcgcgtaatctgctgcttgcaaacaaaaaaaccaccgctaccagcggtggtttgtttgccggatcaagagctaccaactctttttccgaaggtaactggcttcagcagagcgcagataccaaatactgttcttctagtgtagccgtagttaggccaccacttcaagaactctgtagcaccgcctacatacctcgctctgctaatcctgttaccagtggctgctgccagtggcgataagtcgtgtcttaccgggttggactcaagacgatagttaccggataaggcgcagcggtcgggctgaacggggggttcgtgcacacagcccagcttggagcgaacgacctacaccgaactgagatacctacagcgtgagctatgagaaagcgccacgcttcccgaagggagaaaggcggacaggtatccggtaagcggcagggtcggaacaggagagcgcacgagggagcttccagggggaaacgcctggtatctttatagtcctgtcgggtttcgccacctctgacttgagcgtcgatttttgtgatgctcgtcaggggggcggagcctatggaaaaacgccagcaacgcggcctttttacggttcctggccttttgctggccttttgctcacatgttctttcctgcgttatcccctgattctgtggataaccgtattaccgcctttgagtgagctgataccgctcgccgcagccgaacgaccgagcgcagcgagtcagtgagcgaggaagcggaagagcgcccaatacgcaaaccgcctctccccgcgcgttggccgattcattaatgcagctggcacgacaggtttcccgactggaaagcgggcagtgagcgcaacgcaattaatgtgagttagctcactcattaggcaccccaggctttacactttatgcttccggctcgtatgttgtgtggaattgtgagcggataacaatttcacacaggaaacagctatgaccatgattacgccaa

SEQ ID NO: 5 - DNA, 6300 bp, Artificial Sequence
  plasmid
gcggccgcgttttagggcggagtaacttgcatgtattgggaattgtagtttttttaaaatgggaagtgacgtatcgtgggaaaacggaagtgaagatttgaggaagttgtgggttttttggctttcgtttctgggcgtaggttcgcgtgcggttttctgggtgttttttgtggactttaaccgttacgtcattttttagtcctatatatactcgctctgtacttggccctttttacactgtgactgattgagctggtgccgtgtcgagtggtgttttttaataggtttttttactggtaaggctgactgttatggctgccgctgtggaagcgctgtatgttgttctggagcgggagggtgctattttgcctaggcaggagggtttttcaggtgtttatgtgtttttctctcctattaattttgttatacctcctatgggggctgtaatgttgtctctacgcctgcgggtatgtattcccccgggctatttcggtcgctttttagcactgaccgatgttaaccaacctgatgtgtttaccgagtcttacattatgactccggacatgaccgaggaactgtcggtggtgctttttaatcacggtgaccagtttttttacggtcacgccggcatggccgtagtccgtcttatgcttataagggttgtttttcctgttgtaagacaggcttctaatgtttaaatgtttttttttttgttattttattttgtgtttaatgcaggaacccgcagacatgtttgagagaaaaatggtgtctttttctgtggtggttccggaacttacctgcctttatctgcatgagcatgactacgatgtgcttgcttttttgcgcgaggctttgcctgattttttgagcagcaccttgcattttatatcgccgcccatgcaacaagcttacataggggctacgctggttagcatagctccgagtatgcgtgtcataatcagtgtgggttcttttgtcatggttcctggcggggaagtggccgcgctggtccgtgcagacctgcacgattatgttcagctggccctgcgaagggacctacgggatcgcggtatttttgttaatgttccgcttttgaatcttatacaggtctgtgaggaacctgaatttttgcaatcatgattcgctgcttgaggctgaaggtggagggcgctctggagcagatttttacaatggccggacttaatattcgggatttgcttagagacatattgataaggtggcgagatgaaaattatttgggcatggttgaaggtgctggaatgtttatagaggagattcaccctgaagggtttagcctttacgtccacttggacgtgagggcagtttgccttttggaagccattgtgcaacatcttacaaatgccattatctgttctttggctgtagagtttgaccacgccaccggaggggagcgcgttcacttaatagatcttcattttgaggttttggataatcttttggaataaaaaaaaaaaaacatggttcttccagctcttcccgctcctcccgtgtgtgactcgcagaacgaatgtgtaggttggctgggtgtggcttattctgcggtggtggatgttatcagggcagcggcgcatgaaggagtttacatagaacccgaagccagggggcgcctggatgctttgagagagtggatatactacaactactacacagagcgagctaagcgacgagaccggagacgcagatctgtttgtcacgcccgcacctggttttgcttcaggaaatatgactacgtccggcgttccatttggcatgacactacgaccaacacgatctcggttgtctcggcgcactccgtacagtagggatcgcctacctccttttgagacagagacccgcgctaccatactggaggatcatccgctgctgcccgaatgtaacactttgacaatgcacaacgtgagttacgtgcgaggtcttccctgcagtgtgggatttacgctgattcaggaatgggttgttccctgggatatggttctgacgcgggaggagcttgtaatcctgaggaagtgtatgcacgtgtgcctgtgttgtgccaacattgatatcatgacgagcatgatgatccatggttacgagtcctgggctctccactgtcattgttccagtcccggttccctgcagtgcatagccggcgggcaggttttggccagctggtttaggatggtggtggatggcgccatgtttaatcagaggtttatatggtaccgggaggtggtgaattacaacatgccaaaagaggtaatgtttatgtccagcgtgtttatgaggggtcgccacttaatctacctgcgcttgtggtatgatggccacgtgggttctgtggtccccgccatgagctttggatacagcgccttgcactgtgggattttgaacaatattgtggtgctgtgctgcagttactgtgctgatttaagtgagatcagggtgcgctgctgtgcccggaggacaaggcgtctcatgctgcgggcggtgcgaatcatcgctgaggagaccactgccatgttgtattcctgcaggacggagcggcggcggcagcagtttattcgcgcgctgctgcagcaccaccgccctatcctgatgcacgattatgactctacccccatgtaggcgtggacttccccttcgccgcccgttgagcaaccgcaagttggacagcagcctgtggctcagcagctggacagcgacatgaacttaagcgagctgcccggggagtttattaatatcactgatgagcgtttggctcgacaggaaaccgtgtggaatataacacctaagaatatgtctgttacccatgatatgatgctttttaaggccagccggggagaaaggactgtgtactctgtgtgttgggagggaggtggcaggttgaatactagggttctgtgagtttgattaaggtacggtgatcaatataagctatgtggtggtggggctatactactgaatgaaaaatgacttgaaattttctgcaattgaaaaataaacacgttgaaacataacatgcaacaggttcacgattctttattcctgggcaatgtaggagaaggtgtaagagttggtagcaaaagtttcagtggtgtattttccactttcccaggaccatgtaaaagacatagagtaagtgcttacctcgctagtttctgtggattcactagaatcgatgtaggatgttgcccctcctgacgcggtaggagaaggggagggtgccctgcatgtctgccgctgctcttgctcttgccgctgctgaggaggggggcgcatctgccgcagcaccggatgcatctgggaaaagcaaaaaaggggctcgtccctgtttccggaggaatttgcaagcggggtcttgcatgacggggaggcaaacccccgttcgccgcagtccggccggcccgagactcgaaccgggggtcctgcgactcaacccttggaaaataaccctccggctacagggagcgagccacttaatgctttcgctttccagcctaaccgcttacgccgcgcgcggccagtggccaaaaaagctagcgcagcagccgccgcgcctggaaggaagccaaaaggagcgctcccccgttgtctgacgtcgcacacctgggttcgacacgcgggcggtaaccgcatggatcacggcggacggccggatccggggttcgaaccccggtcgtccgccatgatacccttgcgaatttatccaccagaccacggaagagtgcccgcttacaggctctccttttgcacggtctagagcgtcaacgactgcgcacgcctcaccggccagagcgtcccgaccatggagcactttttgccgctgcgcaacatctggaaccgcgtccgcgactttccgcgcgcctccaccaccgccgccggcatcacctggatgtccaggtacatctacggattacgtcgacgtttaaaccatatgatcagctcactcaaaggcggtaatacggttatccacagaatcaggggataacgcaggaaagaacatgtgagcaaaaggccagcaaaaggccaggaaccgtaaaaaggccgcgttgctggcgtttttccataggctccgcccccctgacgagcatcacaaaaatcgacgctcaagtcagaggtggcgaaacccgacaggactataaagataccaggcgtttccccctggaagctccctcgtgcgctctcctgttccgaccctgccgcttaccggatacctgtccgcctttctcccttcgggaagcgtggcgctttctcatagctcacgctgtaggtatctcagttcggtgtaggtcgttcgctccaagctgggctgtgtgcacgaaccccccgttcagcccgaccgctgcgccttatccggtaactatcgtcttgagtccaacccggtaagacacgacttatcgccactggcagcagccactggtaacaggattagcagagcgaggtatgtaggcggtgctacagagttcttgaagtggtggcctaactacggctacactagaagaacagtatttggtatctgcgctctgctgaagccagttaccttcggaaaaagagttggtagctcttgatccggcaaacaaaccaccgctggtagcggtggtttttttgtttgcaagcagcagattacgcgcagaaaaaaaggatctcaagaagatcctttgatcttttctacggggtctgacgctcagtggaacgaaaactcacgttaagggattttggtcatgagattatcaaaaaggatcttcacctagatccttttaaattaaaaatgaagttttaaatcaatctaaagtatatatgagtaaacttggtctgacagttaccaatgcttaatcagtgaggcacctatctcagcgatctgtctatttcgttcatccatagttgcctgactccccgtcgtgtagataactacgatacgggagggcttaccatctggccccagtgctgcaatgataccgcgagacccacgctcaccggctccagatttatcagcaataaaccagccagccggaagggccgagcgcagaagtggtcctgcaactttatccgcctccatccagtctattaattgttgccgggaagctagagtaagtagttcgccagttaatagtttgcgcaacgttgttgccattgctacaggcatcgtggtgtcacgctcgtcgtttggtatggcttcattcagctccggttcccaacgatcaaggcgagttacatgatcccccatgttgtgcaaaaaagcggttagctccttcggtcctccgatcgttgtcagaagtaagttggccgcagtgttatcactcatggttatggcagcactgcataattctcttactgtcatgccatccgtaagatgcttttctgtgactggtgagtactcaaccaagtcattctgagaatagtgtatgcggcgaccgagttgctcttgcccggcgtcaatacgggataataccgcgccacatagcagaactttaaaagtgctcatcattggaaaacgttcttcggggcgaaaactctcaaggatcttaccgctgttgagatccagttcgatgtaacccactcgtgcacccaactgatcttcagcatcttttactttcaccagcgtttctgggtgagcaaaaacaggaaggcaaaatgccgcaaaaaagggaataagggcgacacggaaatgttgaatactcatactcttcctttttcaatattattgaagcatttatcagggttattgtctcatgagcggatacatatttgaatgtatttagaaaaataaacaaataggggttccgcgcacatttccccgaaaagtgccacctaaattgtaagcgttaatattttgttaaaattcgcgttaaatttttgttaaatcagctcattttttaaccaataggccgaaatcggcaaaatcccttataaatcaaaagaatagaccgagatagggttgagtgttgttccagtttggaacaagagtccactattaaagaacgtggactccaacgtcaaagggcgaaaaaccgtctatcagggcgatggcccactacgtgaaccatcaccctaatcaagttttttggggtcgaggtgccgtaaagcactaaatcggaaccctaaagggagcccccgatttagagcttgacggggaaagccggcgaacgtggcgagaaaggaagggaagaaagcgaaaggagcgggcgctagggcgctggcaagtgtagcggtcacgctgcgcgtaaccaccacacccgccgcgcttaatgcgccgctacagggcgcgatggatcc

SEQ ID NO: 6 - DNA, 8451 bp, Artificial Sequence
  plasmid
ggtacccaactccatgcttaacagtccccaggtacagcccaccctgcgtcgcaaccaggaacagctctacagcttcctggagcgccactcgccctacttccgcagccacagtgcgcagattaggagcgccacttctttttgtcacttgaaaaacatgtaaaaataatgtactaggagacactttcaataaaggcaaatgtttttatttgtacactctcgggtgattatttaccccccacccttgccgtctgcgccgtttaaaaatcaaaggggttctgccgcgcatcgctatgcgccactggcagggacacgttgcgatactggtgtttagtgctccacttaaactcaggcacaaccatccgcggcagctcggtgaagttttcactccacaggctgcgcaccatcaccaacgcgtttagcaggtcgggcgccgatatcttgaagtcgcagttggggcctccgccctgcgcgcgcgagttgcgatacacagggttgcagcactggaacactatcagcgccgggtggtgcacgctggccagcacgctcttgtcggagatcagatccgcgtccaggtcctccgcgttgctcagggcgaacggagtcaactttggtagctgccttcccaaaaagggtgcatgcccaggctttgagttgcactcgcaccgtagtggcatcagaaggtgaccgtgcccggtctgggcgttaggatacagcgcctgcatgaaagccttgatctgcttaaaagccacctgagcctttgcgccttcagagaagaacatgccgcaagacttgccggaaaactgattggccggacaggccgcgtcatgcacgcagcaccttgcgtcggtgttggagatctgcaccacatttcggccccaccggttcttcacgatcttggccttgctagactgctccttcagcgcgcgctgcccgttttcgctcgtcacatccatttcaatcacgtgctccttatttatcataatgctcccgtgtagacacttaagctcgccttcgatctcagcgcagcggtgcagccacaacgcgcagcccgtgggctcgtggtgcttgtaggttacctctgcaaacgactgcaggtacgcctgcaggaatcgccccatcatcgtcacaaaggtcttgttgctggtgaaggtcagctgcaacccgcggtgctcctcgtttagccaggtcttgcatacggccgccagagcttccacttggtcaggcagtagcttgaagtttgcctttagatcgttatccacgtggtacttgtccatcaacgcgcgcgcagcctccatgcccttctcccacgcagacacgatcggcaggctcagcgggtttatcaccgtgctttcactttccgcttcactggactcttccttttcctcttgcgtccgcataccccgcgccactgggtcgtcttcattcagccgccgcaccgtgcgcttacctcccttgccgtgcttgattagcaccggtgggttgctgaaacccaccatttgtagcgccacatcttctctttcttcctcgctgtccacgatcacctctggggatggcgggcgctcgggcttgggagaggggcgcttctttttctttttggacgcaatggccaaatccgccgtcgaggtcgatggccgcgggctgggtgtgcgcggcaccagcgcatcttgtgacgagtcttcttcgtcctcggactcgagacgccgcctcagccgcttttttgggggcgcgcggggaggcggcggcgacggcgacggggacgacacgtcctccatggttggtggacgtcgcgccgcaccgcgtccgcgctcgggggtggtttcgcgctgctcctcttcccgactggccatttccttctcctataggcagaaaaagatcatggagtcagtcgagaaggaggacagcctaaccgccccctttgagttcgccaccaccgcctccaccgatgccgccaacgcgcctaccaccttccccgtcgaggcacccccgcttgaggaggaggaagtgattatcgagcaggacccaggttttgtaagcgaagacgacgaggatcgctcagtaccaacagaggataaaaagcaagaccaggacgacgcagaggcaaacgaggaacaagtcgggcggggggaccaaaggcatggcgactacctagatgtgggagacgacgtgctgttgaagcatctgcagcgccagtgcgccattatctgcgacgcgttgcaagagcgcagcgatgtgcccctcgccatagcggatgtcagccttgcctacgaacgccacctgttctcaccgcgcgtaccccccaaacgccaagaaaacggcacatgcgagcccaacccgcgcctcaacttctaccccgtatttgccgtgccagaggtgcttgccacctatcacatctttttccaaaactgcaagatacccctatcctgccgtgccaaccgcagccgagcggacaagcagctggccttgcggcagggcgctgtcatacctgatatcgcctcgctcgacgaagtgccaaaaatctttgagggtcttggacgcgacgagaaacgcgcggcaaacgctctgcaacaagaaaacagcgaaaatgaaagtcactgtggagtgctggtggaacttgagggtgacaacgcgcgcctagccgtgctgaaacgcagcatcgaggtcacccactttgcctacccggcacttaacctaccccccaaggttatgagcacagtcatgagcgagctgatcgtgcgccgtgcacgacccctggagagggatgcaaacttgcaagaacaaaccgaggagggcctacccgcagttggcgatgagcagctggcgcgctggcttgagacgcgcgagcctgccgacttggaggagcgacgcaagctaatgatggccgcagtgcttgttaccgtggagcttgagtgcatgcagcggttctttgctgacccggagatgcagcgcaagctagaggaaacgttgcactacacctttcgccagggctacgtgcgccaggcctgcaaaatttccaacgtggagctctgcaacctggtctcctaccttggaattttgcacgaaaaccgcctcgggcaaaacgtgcttcattccacgctcaagggcgaggcgcgccgcgactacgtccgcgactgcgtttacttatttctgtgctacacctggcaaacggccatgggcgtgtggcagcaatgcctggaggagcgcaacctaaaggagctgcagaagctgctaaagcaaaacttgaaggacctatggacggccttcaacgagcgctccgtggccgcgcacctggcggacattatcttccccgaacgcctgcttaaaaccctgcaacagggtctgccagacttcaccagtcaaagcatgttgcaaaactttaggaactttatcctagagcgttcaggaattctgcccgccacctgctgtgcgcttcctagcgactttgtgcccattaagtaccgtgaatgccctccgccgctttggggtcactgctaccttctgcagctagccaactaccttgcctaccactccgacatcatggaagacgtgagcggtgacggcctactggagtgtcactgtcgctgcaacctatgcaccccgcaccgctccctggtctgcaattcgcaactgcttagcgaaagtcaaattatcggtacctttgagctgcagggtccctcgcctgacgaaaagtccgcggctccggggttgaaactcactccggggctgtggacgtcggcttaccttcgcaaatttgtacctgaggactaccacgcccacgagattaggttctacgaagaccaatcccgcccgccaaatgcggagcttaccgcctgcgtcattacccagggccacatccttggccaattgcaagccatcaacaaagcccgccaagagtttctgctacgaaagggacggggggtttacctggacccccagtccggcgaggagctcaacccaatccccccgccgccgcagccctatcagcagccgcgggcccttgcttcccaggatggcacccaaaaagaagctgcagctgccgccgccgccacccacggacgaggaggaatactgggacagtcaggcagaggaggttttggacgaggaggaggagatgatggaagactgggacagcctagacgaagcttccgaggccgaagaggtgtcagacgaaacaccgtcaccctcggtcgcattcccctcgccggcgccccagaaattggcaaccgttcccagcatcgctacaacctccgctcctcaggcgccgccggcactgcctgttcgccgacccaaccgtagatgggacaccactggaaccagggccggtaagtctaagcagccgccgccgttagcccaagagcaacaacagcgccaaggctaccgctcgtggcgcgggcacaagaacgccatagttgcttgcttgcaagactgtgggggcaacatctccttcgcccgccgctttcttctctaccatcacggcgtggccttcccccgtaacatcctgcattactaccgtcatctctacagcccctactgcaccggcggcagcggcagcggcagcaacagcagcggtcacacagaagcaaaggcgaccggatagcaagactctgacaaagcccaagaaatccacagcggcggcagcagcaggaggaggagcgctgcgtctggcgcccaacgaacccgtatcgacccgcgagcttagaaataggatttttcccactctgtatgctatatttcaacaaagcaggggccaagaacaagagctgaaaataaaaaacaggtctctgcgctccctcacccgcagctgcctgtatcacaaaagcgaagatcagcttcggcgcacgctggaagacgcggaggctctcttcagcaaatactgcgcgctgactcttaaggactagtttcgcgccctttctcaaatttaagcgcgaaaactacgtcatctccagcggccacacccggcgccagcacctgtcgtcagcgccattatgagcaaggaaattcccacgccctacatgtggagttaccagccacaaatgggacttgcggctggagctgcccaagactactcaacccgaataaactacatgagcgcgggaccccacatgatatcccgggtcaacggaatccgcgcccaccgaaaccgaattctcctcgaacaggcggctattaccaccacacctcgtaataaccttaatccccgtagttggcccgctgccctggtgtaccaggaaagtcccgctcccaccactgtggtacttcccagagacgcccaggccgaagttcagatgactaactcaggggcgcagcttgcgggcggctttcgtcacagggtgcggtcgcccgggcgcggccgcaatcgatgtaggatgttgcccctcctgacgcggtaggagaaggggagggtgccctgcatgtctgccgctgctcttgctcttgccgctgctgaggaggggggcgcatctgccgcagcaccggatgcatctgggaaaagcaaaaaaggggctcgtccctgtttccggaggaatttgcaagcggggtcttgcatgacggggaggcaaacccccgttcgccgcagtccggccggcccgagactcgaaccgggggtcctgcgactcaacccttggaaaataaccctccggctacagggagcgagccacttaatgctttcgctttccagcctaaccgcttacgccgcgcgcggccagtggccaaaaaagctagcgcagcagccgccgcgcctggaaggaagccaaaaggagcgctcccccgttgtctgacgtcgcacacctgggttcgacacgcgggcggtaaccgcatggatcacggcggacggccggatccggggttcgaaccccggtcgtccgccatgatacccttgcgaatttatccaccagaccacggaagagtgcccgcttacaggctctccttttgcacggtctagagcgtcaacgactgcgcacgcctcaccggccagagcgtcccgaccatggagcactttttgccgctgcgcaacatctggaaccgcgtccgcgactttccgcgcgcctccaccaccgccgccggcatcacctggatgtccaggtacatctacggattacgtcgacgtttaaaccatatgatcagctcactcaaaggcggtaatacggttatccacagaatcaggggataacgcaggaaagaacatgtgagcaaaaggccagcaaaaggccaggaaccgtaaaaaggccgcgttgctggcgtttttccataggctccgcccccctgacgagcatcacaaaaatcgacgctcaagtcagaggtggcgaaacccgacaggactataaagataccaggcgtttccccctggaagctccctcgtgcgctctcctgttccgaccctgccgcttaccggatacctgtccgcctttctcccttcgggaagcgtggcgctttctcatagctcacgctgtaggtatctcagttcggtgtaggtcgttcgctccaagctgggctgtgtgcacgaaccccccgttcagcccgaccgctgcgccttatccggtaactatcgtcttgagtccaacccggtaagacacgacttatcgccactggcagcagccactggtaacaggattagcagagcgaggtatgtaggcggtgctacagagttcttgaagtggtggcctaactacggctacactagaagaacagtatttggtatctgcgctctgctgaagccagttaccttcggaaaaagagttggtagctcttgatccggcaaacaaaccaccgctggtagcggtggtttttttgtttgcaagcagcagattacgcgcagaaaaaaaggatctcaagaagatcctttgatcttttctacggggtctgacgctcagtggaacgaaaactcacgttaagggattttggtcatgagattatcaaaaaggatcttcacctagatccttttaaattaaaaatgaagttttaaatcaatctaaagtatatatgagtaaacttggtctgacagttaccaatgcttaatcagtgaggcacctatctcagcgatctgtctatttcgttcatccatagttgcctgactccccgtcgtgtagataactacgatacgggagggcttaccatctggccccagtgctgcaatgataccgcgagacccacgctcaccggctccagatttatcagcaataaaccagccagccggaagggccgagcgcagaagtggtcctgcaactttatccgcctccatccagtctattaattgttgccgggaagctagagtaagtagttcgccagttaatagtttgcgcaacgttgttgccattgctacaggcatcgtggtgtcacgctcgtcgtttggtatggcttcattcagctccggttcccaacgatcaaggcgagttacatgatcccccatgttgtgcaaaaaagcggttagctccttcggtcctccgatcgttgtcagaagtaagttggccgcagtgttatcactcatggttatggcagcactgcataattctcttactgtcatgccatccgtaagatgcttttctgtgactggtgagtactcaaccaagtcattctgagaatagtgtatgcggcgaccgagttgctcttgcccggcgtcaatacgggataataccgcgccacatagcagaactttaaaagtgctcatcattggaaaacgttcttcggggcgaaaactctcaaggatcttaccgctgttgagatccagttcgatgtaacccactcgtgcacccaactgatcttcagcatcttttactttcaccagcgtttctgggtgagcaaaaacaggaaggcaaaatgccgcaaaaaagggaataagggcgacacggaaatgttgaatactcatactcttcctttttcaatattattgaagcatttatcagggttattgtctcatgagcggatacatatttgaatgtatttagaaaaataaacaaataggggttccgcgcacatttccccgaaaagtgccacctaaattgtaagcgttaatattttgttaaaattcgcgttaaatttttgttaaatcagctcattttttaaccaataggccgaaatcggcaaaatcccttataaatcaaaagaatagaccgagatagggttgagtgttgttccagtttggaacaagagtccactattaaagaacgtggactccaacgtcaaagggcgaaaaaccgtctatcagggcgatggcccactacgtgaaccatcaccctaatcaagttttttggggtcgaggtgccgtaaagcactaaatcggaaccctaaagggagcccccgatttagagcttgacggggaaagccggcgaacgtggcgagaaaggaagggaagaaagcgaaaggagcgggcgctagggcgctggcaagtgtagcggtcacgctgcgcgtaaccaccacacccgccgcgcttaatgcgccgctacagggcgcgatggatcc

SEQ ID NO: 7 - DNA, 10912 bp, Artificial Sequence
  plasmid
ggtacccaactccatgcttaacagtccccaggtacagcccaccctgcgtcgcaaccaggaacagctctacagcttcctggagcgccactcgccctacttccgcagccacagtgcgcagattaggagcgccacttctttttgtcacttgaaaaacatgtaaaaataatgtactaggagacactttcaataaaggcaaatgtttttatttgtacactctcgggtgattatttaccccccacccttgccgtctgcgccgtttaaaaatcaaaggggttctgccgcgcatcgctatgcgccactggcagggacacgttgcgatactggtgtttagtgctccacttaaactcaggcacaaccatccgcggcagctcggtgaagttttcactccacaggctgcgcaccatcaccaacgcgtttagcaggtcgggcgccgatatcttgaagtcgcagttggggcctccgccctgcgcgcgcgagttgcgatacacagggttgcagcactggaacactatcagcgccgggtggtgcacgctggccagcacgctcttgtcggagatcagatccgcgtccaggtcctccgcgttgctcagggcgaacggagtcaactttggtagctgccttcccaaaaagggtgcatgcccaggctttgagttgcactcgcaccgtagtggcatcagaaggtgaccgtgcccggtctgggcgttaggatacagcgcctgcatgaaagccttgatctgcttaaaagccacctgagcctttgcgccttcagagaagaacatgccgcaagacttgccggaaaactgattggccggacaggccgcgtcatgcacgcagcaccttgcgtcggtgttggagatctgcaccacatttcggccccaccggttcttcacgatcttggccttgctagactgctccttcagcgcgcgctgcccgttttcgctcgtcacatccatttcaatcacgtgctccttatttatcataatgctcccgtgtagacacttaagctcgccttcgatctcagcgcagcggtgcagccacaacgcgcagcccgtgggctcgtggtgcttgtaggttacctctgcaaacgactgcaggtacgcctgcaggaatcgccccatcatcgtcacaaaggtcttgttgctggtgaaggtcagctgcaacccgcggtgctcctcgtttagccaggtcttgcatacggccgccagagcttccacttggtcaggcagtagcttgaagtttgcctttagatcgttatccacgtggtacttgtccatcaacgcgcgcgcagcctccatgcccttctcccacgcagacacgatcggcaggctcagcgggtttatcaccgtgctttcactttccgcttcactggactcttccttttcctcttgcgtccgcataccccgcgccactgggtcgtcttcattcagccgccgcaccgtgcgcttacctcccttgccgtgcttgattagcaccggtgggttgctgaaacccaccatttgtagcgccacatcttctctttcttcctcgctgtccacgatcacctctggggatggcgggcgctcgggcttgggagaggggcgcttctttttctttttggacgcaatggccaaatccgccgtcgaggtcgatggccgcgggctgggtgtgcgcggcaccagcgcatcttgtgacgagtcttcttcgtcctcggactcgagacgccgcctcagccgcttttttgggggcgcgcggggaggcggcggcgacggcgacggggacgacacgtcctccatggttggtggacgtcgcgccgcaccgcgtccgcgctcgggggtggtttcgcgctgctcctcttcccgactggccatttccttctcctataggcagaaaaagatcatggagtcagtcgagaaggaggacagcctaaccgccccctttgagttcgccaccaccgcctccaccgatgccgccaacgcgcctaccaccttccccgtcgaggcacccccgcttgaggaggaggaagtgattatcgagcaggacccaggttttgtaagcgaagacgacgaggatcgctcagtaccaacagaggataaaaagcaagaccaggacgacgcagaggcaaacgaggaacaagtcgggcggggggaccaaaggcatggcgactacctagatgtgggagacgacgtgctgttgaagcatctgcagcgccagtgcgccattatctgcgacgcgttgcaagagcgcagcgatgtgcccctcgccatagcggatgtcagccttgcctacgaacgccacctgttctcaccgcgcgtaccccccaaacgccaagaaaacggcacatgcgagcccaacccgcgcctcaacttctaccccgtatttgccgtgccagaggtgcttgccacctatcacatctttttccaaaactgcaagatacccctatcctgccgtgccaaccgcagccgagcggacaagcagctggccttgcggcagggcgctgtcatacctgatatcgcctcgctcgacgaagtgccaaaaatctttgagggtcttggacgcgacgagaaacgcgcggcaaacgctctgcaacaagaaaacagcgaaaatgaaagtcactgtggagtgctggtggaacttgagggtgacaacgcgcgcctagccgtgctgaaacgcagcatcgaggtcacccactttgcctacccggcacttaacctaccccccaaggttatgagcacagtcatgagcgagctgatcgtgcgccgtgcacgacccctggagagggatgcaaacttgcaagaacaaaccgaggagggcctacccgcagttggcgatgagcagctggcgcgctggcttgagacgcgcgagcctgccgacttggaggagcgacgcaagctaatgatggccgcagtgcttgttaccgtggagcttgagtgcatgcagcggttctttgctgacccggagatgcagcgcaagctagaggaaacgttgcactacacctttcgccagggctacgtgcgccaggcctgcaaaatttccaacgtggagctctgcaacctggtctcctaccttggaattttgcacgaaaaccgcctcgggcaaaacgtgcttcattccacgctcaagggcgaggcgcgccgcgactacgtccgcgactgcgtttacttatttctgtgctacacctggcaaacggccatgggcgtgtggcagcaatgcctggaggagcgcaacctaaaggagctgcagaagctgctaaagcaaaacttgaaggacctatggacggccttcaacgagcgctccgtggccgcgcacctggcggacattatcttccccgaacgcctgcttaaaaccctgcaacagggtctgccagacttcaccagtcaaagcatgttgcaaaactttaggaactttatcctagagcgttcaggaattctgcccgccacctgctgtgcgcttcctagcgactttgtgcccattaagtaccgtgaatgccctccgccgctttggggtcactgctaccttctgcagctagccaactaccttgcctaccactccgacatcatggaagacgtgagcggtgacggcctactggagtgtcactgtcgctgcaacctatgcaccccgcaccgctccctggtctgcaattcgcaactgcttagcgaaagtcaaattatcggtacctttgagctgcagggtccctcgcctgacgaaaagtccgcggctccggggttgaaactcactccggggctgtggacgtcggcttaccttcgcaaatttgtacctgaggactaccacgcccacgagattaggttctacgaagaccaatcccgcccgccaaatgcggagcttaccgcctgcgtcattacccagggccacatccttggccaattgcaagccatcaacaaagcccgccaagagtttctgctacgaaagggacggggggtttacctggacccccagtccggcgaggagctcaacccaatccccccgccgccgcagccctatcagcagccgcgggcccttgcttcccaggatggcacccaaaaagaagctgcagctgccgccgccgccacccacggacgaggaggaatactgggacagtcaggcagaggaggttttggacgaggaggaggagatgatggaagactgggacagcctagacgaagcttccgaggccgaagaggtgtcagacgaaacaccgtcaccctcggtcgcattcccctcgccggcgccccagaaattggcaaccgttcccagcatcgctacaacctccgctcctcaggcgccgccggcactgcctgttcgccgacccaaccgtagatgggacaccactggaaccagggccggtaagtctaagcagccgccgccgttagcccaagagcaacaacagcgccaaggctaccgctcgtggcgcgggcacaagaacgccatagttgcttgcttgcaagactgtgggggcaacatctccttcgcccgccgctttcttctctaccatcacggcgtggccttcccccgtaacatcctgcattactaccgtcatctctacagcccctactgcaccggcggcagcggcagcggcagcaacagcagcggtcacacagaagcaaaggcgaccggatagcaagactctgacaaagcccaagaaatccacagcggcggcagcagcaggaggaggagcgctgcgtctggcgcccaacgaacccgtatcgacccgcgagcttagaaataggatttttcccactctgtatgctatatttcaacaaagcaggggccaagaacaagagctgaaaataaaaaacaggtctctgcgctccctcacccgcagctgcctgtatcacaaaagcgaagatcagcttcggcgcacgctggaagacgcggaggctctcttcagcaaatactgcgcgctgactcttaaggactagtttcgcgccctttctcaaatttaagcgcgaaaactacgtcatctccagcggccacacccggcgccagcacctgtcgtcagcgccattatgagcaaggaaattcccacgccctacatgtggagttaccagccacaaatgggacttgcggctggagctgcccaagactactcaacccgaataaactacatgagcgcgggaccccacatgatatcccgggtcaacggaatccgcgcccaccgaaaccgaattctcctcgaacaggcggctattaccaccacacctcgtaataaccttaatccccgtagttggcccgctgccctggtgtaccaggaaagtcccgctcccaccactgtggtacttcccagagacgcccaggccgaagttcagatgactaactcaggggcgcagcttgcgggcggctttcgtcacagggtgcggtcgcccgggcgttttagggcggagtaacttgcatgtattgggaattgtagtttttttaaaatgggaagtgacgtatcgtgggaaaacggaagtgaagatttgaggaagttgtgggttttttggctttcgtttctgggcgtaggttcgcgtgcggttttctgggtgttttttgtggactttaaccgttacgtcattttttagtcctatatatactcgctctgtacttggccctttttacactgtgactgattgagctggtgccgtgtcgagtggtgttttttaataggtttttttactggtaaggctgactgttatggctgccgctgtggaagcgctgtatgttgttctggagcgggagggtgctattttgcctaggcaggagggtttttcaggtgtttatgtgtttttctctcctattaattttgttatacctcctatgggggctgtaatgttgtctctacgcctgcgggtatgtattcccccgggctatttcggtcgctttttagcactgaccgatgttaaccaacctgatgtgtttaccgagtcttacattatgactccggacatgaccgaggaactgtcggtggtgctttttaatcacggtgaccagtttttttacggtcacgccggcatggccgtagtccgtcttatgcttataagggttgtttttcctgttgtaagacaggcttctaatgtttaaatgtttttttttttgttattttattttgtgtttaatgcaggaacccgcagacatgtttgagagaaaaatggtgtctttttctgtggtggttccggaacttacctgcctttatctgcatgagcatgactacgatgtgcttgcttttttgcgcgaggctttgcctgattttttgagcagcaccttgcattttatatcgccgcccatgcaacaagcttacataggggctacgctggttagcatagctccgagtatgcgtgtcataatcagtgtgggttcttttgtcatggttcctggcggggaagtggccgcgctggtccgtgcagacctgcacgattatgttcagctggccctgcgaagggacctacgggatcgcggtatttttgttaatgttccgcttttgaatcttatacaggtctgtgaggaacctgaatttttgcaatcatgattcgctgcttgaggctgaaggtggagggcgctctggagcagatttttacaatggccggacttaatattcgggatttgcttagagacatattgataaggtggcgagatgaaaattatttgggcatggttgaaggtgctggaatgtttatagaggagattcaccctgaagggtttagcctttacgtccacttggacgtgagggcagtttgccttttggaagccattgtgcaacatcttacaaatgccattatctgttctttggctgtagagtttgaccacgccaccggaggggagcgcgttcacttaatagatcttcattttgaggttttggataatcttttggaataaaaaaaaaaaaacatggttcttccagctcttcccgctcctcccgtgtgtgactcgcagaacgaatgtgtaggttggctgggtgtggcttattctgcggtggtggatgttatcagggcagcggcgcatgaaggagtttacatagaacccgaagccagggggcgcctggatgctttgagagagtggatatactacaactactacacagagcgagctaagcgacgagaccggagacgcagatctgtttgtcacgcccgcacctggttttgcttcaggaaatatgactacgtccggcgttccatttggcatgacactacgaccaacacgatctcggttgtctcggcgcactccgtacagtagggatcgcctacctccttttgagacagagacccgcgctaccatactggaggatcatccgctgctgcccgaatgtaacactttgacaatgcacaacgtgagttacgtgcgaggtcttccctgcagtgtgggatttacgctgattcaggaatgggttgttccctgggatatggttctgacgcgggaggagcttgtaatcctgaggaagtgtatgcacgtgtgcctgtgttgtgccaacattgatatcatgacgagcatgatgatccatggttacgagtcctgggctctccactgtcattgttccagtcccggttccctgcagtgcatagccggcgggcaggttttggccagctggtttaggatggtggtggatggcgccatgtttaatcagaggtttatatggtaccgggaggtggtgaattacaacatgccaaaagaggtaatgtttatgtccagcgtgtttatgaggggtcgccacttaatctacctgcgcttgtggtatgatggccacgtgggttctgtggtccccgccatgagctttggatacagcgccttgcactgtgggattttgaacaatattgtggtgctgtgctgcagttactgtgctgatttaagtgagatcagggtgcgctgctgtgcccggaggacaaggcgtctcatgctgcgggcggtgcgaatcatcgctgaggagaccactgccatgttgtattcctgcaggacggagcggcggcggcagcagtttattcgcgcgctgctgcagcaccaccgccctatcctgatgcacgattatgactctacccccatgtaggcgtggacttccccttcgccgcccgttgagcaaccgcaagttggacagcagcctgtggctcagcagctggacagcgacatgaacttaagcgagctgcccggggagtttattaatatcactgatgagcgtttggctcgacaggaaaccgtgtggaatataacacctaagaatatgtctgttacccatgatatgatgctttttaaggccagccggggagaaaggactgtgtactctgtgtgttgggagggaggtggcaggttgaatactagggttctgtgagtttgattaaggtacggtgatcaatataagctatgtggtggtggggctatactactgaatgaaaaatgacttgaaattttctgcaattgaaaaataaacacgttgaaacataacatgcaacaggttcacgattctttattcctgggcaatgtaggagaaggtgtaagagttggtagcaaaagtttcagtggtgtattttccactttcccaggaccatgtaaaagacatagagtaagtgcttacctcgctagtttctgtggattcactagaatcgatgtagcggccgctacgtcgacgtttaaaccatatgatcagctcactcaaaggcggtaatacggttatccacagaatcaggggataacgcaggaaagaacatgtgagcaaaaggccagcaaaaggccaggaaccgtaaaaaggccgcgttgctggcgtttttccataggctccgcccccctgacgagcatcacaaaaatcgacgctcaagtcagaggtggcgaaacccgacaggactataaagataccaggcgtttccccctggaagctccctcgtgcgctctcctgttccgaccctgccgcttaccggatacctgtccgcctttctcccttcgggaagcgtggcgctttctcatagctcacgctgtaggtatctcagttcggtgtaggtcgttcgctccaagctgggctgtgtgcacgaaccccccgttcagcccgaccgctgcgccttatccggtaactatcgtcttgagtccaacccggtaagacacgacttatcgccactggcagcagccactggtaacaggattagcagagcgaggtatgtaggcggtgctacagagttcttgaagtggtggcctaactacggctacactagaagaacagtatttggtatctgcgctctgctgaagccagttaccttcggaaaaagagttggtagctcttgatccggcaaacaaaccaccgctggtagcggtggtttttttgtttgcaagcagcagattacgcgcagaaaaaaaggatctcaagaagatcctttgatcttttctacggggtctgacgctcagtggaacgaaaactcacgttaagggattttggtcatgagattatcaaaaaggatcttcacctagatccttttaaattaaaaatgaagttttaaatcaatctaaagtatatatgagtaaacttggtctgacagttaccaatgcttaatcagtgaggcacctatctcagcgatctgtctatttcgttcatccatagttgcctgactccccgtcgtgtagataactacgatacgggagggcttaccatctggccccagtgctgcaatgataccgcgagacccacgctcaccggctccagatttatcagcaataaaccagccagccggaagggccgagcgcagaagtggtcctgcaactttatccgcctccatccagtctattaattgttgccgggaagctagagtaagtagttcgccagttaatagtttgcgcaacgttgttgccattgctacaggcatcgtggtgtcacgctcgtcgtttggtatggcttcattcagctccggttcccaacgatcaaggcgagttacatgatcccccatgttgtgcaaaaaagcggttagctccttcggtcctccgatcgttgtcagaagtaagttggccgcagtgttatcactcatggttatggcagcactgcataattctcttactgtcatgccatccgtaagatgcttttctgtgactggtgagtactcaaccaagtcattctgagaatagtgtatgcggcgaccgagttgctcttgcccggcgtcaatacgggataataccgcgccacatagcagaactttaaaagtgctcatcattggaaaacgttcttcggggcgaaaactctcaaggatcttaccgctgttgagatccagttcgatgtaacccactcgtgcacccaactgatcttcagcatcttttactttcaccagcgtttctgggtgagcaaaaacaggaaggcaaaatgccgcaaaaaagggaataagggcgacacggaaatgttgaatactcatactcttcctttttcaatattattgaagcatttatcagggttattgtctcatgagcggatacatatttgaatgtatttagaaaaataaacaaataggggttccgcgcacatttccccgaaaagtgccacctaaattgtaagcgttaatattttgttaaaattcgcgttaaatttttgttaaatcagctcattttttaaccaataggccgaaatcggcaaaatcccttataaatcaaaagaatagaccgagatagggttgagtgttgttccagtttggaacaagagtccactattaaagaacgtggactccaacgtcaaagggcgaaaaaccgtctatcagggcgatggcccactacgtgaaccatcaccctaatcaagttttttggggtcgaggtgccgtaaagcactaaatcggaaccctaaagggagcccccgatttagagcttgacggggaaagccggcgaacgtggcgagaaaggaagggaagaaagcgaaaggagcgggcgctagggcgctggcaagtgtagcggtcacgctgcgcgtaaccaccacacccgccgcgcttaatgcgccgctacagggcgcgatggatcc

SEQ ID NO: 8 - DNA, 5127 bp, Artificial Sequence; identical to SEQ ID NO: 4
  plasmid

SEQ ID NO: 9 - DNA, 5952 bp, Artificial Sequence; identical to SEQ ID NO: 3
  plasmid

SEQ ID NO: 10 - DNA, 8012 bp, Artificial Sequence
  plasmid
tcgcgcgtttcggtgatgacggtgaaaacctctgacacatgcagctcccggagactgtcacagcttgtctgtaagcggatgccgggagcagacaagcccgtcagggcgcgtcagcgggtgttggcgggtgtcggggctggcttaactatgcggcatcagagcagattgtactgagagtgcaccatatgcggtgtgaaataccgcacagatgcgtaaggagaaaataccgcatcaggcgccattcgccattcaggctgcgcaactgttgggaagggcgatcggtgcgggcctcttcgctattacgccagctggcgaaagggggatgtgctgcaaggcgattaagttgggtaacgccagggttttcccagtcacgacgttgtaaaacgacggccagtgaattgacgcgtattgggatggtacccaactccatgctcaacagtccccaggtacagcccaccctgcgtcgcaaccaggaacagctctacagcttcctggagcgccactcgccctacttccgcagccacagtgcgcagattaggagcgccacttctttttgtcacttgaaaaacatgtaaaaataatgtactagagacactttcaataaaggcaaatgcttttatttgtacactctcgggtgattatttacccccacccttgccgtctgcgccgtttaaaaatcaaaggggttctgccgcgcatcgctatgcgccactggcagggacacgttgcgatactggtgtttagtgctccacttaaactcaggcacaaccatccgcggcagctcggtgaagttttcactccacaggctgcgcaccatcaccaacgcgtttagcaggtcgggcgccgatatcttgaagtcgcagttggggcctccgccctgcgcgcgcgagttgcgatacacagggttgcagcactggaacactatcagcgccgggtggtgcacgctggccagcacgctcttgtcggagatcagatccgcgtccaggtcctccgcgttgctcagggcgaacggagtcaactttggtagctgccttcccaaaaagggcgcgtgcccaggctttgagttgcactcgcaccgtagtggcatcaaaaggtgaccgtgcccggtctgggcgttaggatacagcgcctgcataaaagccttgatctgcttaaaagccacctgagcctttgcgccttcagagaagaacatgccgcaagacttgccggaaaactgattggccggacaggccgcgtcgtgcacgcagcaccttgcgtcggtgttggagatctgcaccacatttcggccccaccggttcttcacgatcttggccttgctagactgctccttcagcgcgcgctgcccgttttcgctcgtcacatccatttcaatcacgtgctccttatttatcataatgcttccgtgtagacacttaagctcgccttcgatctcagcgcagcggtgcagccacaacgcgcagcccgtgggctcgtgatgcttgtaggtcacctctgcaaacgactgcaggtacgcctgcaggaatcgccccatcatcgtcacaaaggtcttgttgctggtgaaggtcagctgcaacccgcggtgctcctcgttcagccaggtcttgcatacggccgccagagcttccacttggtcaggcagtagtttgaagttcgcctttagatcgttatccacgtggtacttgtccatcagcgcgcgcgcagcctccatgcccttctcccacgcagacacgatcggcacactcagcgggttcatcaccgtaatttcactttccgcttcgctgggctcttcctcttcctcttgcgtccgcataccacgcgccactgggtcgtcttcattcagccgccgcactgtgcgcttacctcctttgccatgcttgattagcaccggtgggttgctgaaacccaccatttgtagcgccacatcttctctttcttcctcgctgtccacgattacctctggtgatggcgggcgctcgggcttgggagaagggcgcttctttttcttcttgggcgcaatggccaaatccgccgccgaggtcgatggccgcgggctgggtgtgcgcggcaccagcgcgtcttgtgatgagtcttcctcgtcctcggactcgatacgccgcctcatccgcttttttgggggcgcccggggaggcggcggcgacggggacggggacgacacgtcctccatggttgggggacgtcgcgccgcaccgcgtccgcgctcgggggtggtttcgcgctgctcctcttcccgactggccatttccttctcctataggcagaaaaagatcatggagtcagtcgagaagaaggacagcctaaccgccccctctgagttcgccaccaccgcctccaccgatgccgccaacgcgcctaccaccttccccgtcgaggcacccccgcttgaggaggaggaagtgattatcgagcaggacccaggttttgtaagcgaagacgacgaggaccgctcagtaccaacagaggataaaaagcaagaccaggacaacgcagaggcaaacgaggaacaagtcgggcggggggacgaaaggcatggcgactacctagatgtgggagacgacgtgctgttgaagcatctgcagcgccagtgcgccattatctgcgacgcgttgcaagagcgcagcgatgtgcccctcgccatagcggatgtcagccttgcctacgaacgccacctattctcaccgcgcgtaccccccaaacgccaagaaaacggcacatgcgagcccaacccgcgcctcaacttctaccccgtatttgccgtgccagaggtgcttgccacctatcacatctttttccaaaactgcaagatacccctatcctgccgtgccaaccgcagccgagcggacaagcagctggccttgcggcagggcgctgtcatacctgatatcgcctcgctcaacgaagtgccaaaaatctttgagggtcttggacgcgacgagaagcgcgcggcaaacgctctgcaacaggaaaacagcgaaaatgaaagtcactctggagtgttggtggaactcgagggtgacaacgcgcgcctagccgtactaaaacgcagcatcgaggtcacccactttgcctacccggcacttaacctaccccccaaggtcatgagcacagtcatgagtgagctgatcgtgcgccgtgcgcagcccctggagagggatgcaaatttgcaagaacaaacagaggagggcctacccgcagttggcgacgagcagctagcgcgctggcttcaaacgcgcgagcctgccgacttggaggagcgacgcaaactaatgatggccgcagtgctcgttaccgtggagcttgagtgcatgcagcggttctttgctgacccggagatgcagcgcaagctagaggaaacattgcactacacctttcgacagggctacgtacgccaggcctgcaagatctccaacgtggagctctgcaacctggtctcctaccttggaattttgcacgaaaaccgccttgggcaaaacgtgcttcattccacgctcaagggcgaggcgcgccgcgactacgtccgcgactgcgtttacttatttctatgctacacctggcagacggccatgggcgtttggcagcagtgcttggaggagtgcaacctcaaggagctgcagaaactgctaaagcaaaacttgaaggacctatggacggccttcaacgagcgctccgtggccgcgcacctggcggacatcattttccccgaacgcctgcttaaaaccctgcaacagggtctgccagacttcaccagtcaaagcatgttgcagaactttaggaactttatcctagagcgctcaggaatcttgcccgccacctgctgtgcacttcctagcgactttgtgcccattaagtaccgcgaatgccctccgccgctttggggccactgctaccttctgcagctagccaactaccttgcctaccactctgacataatggaagacgtgagcggtgacggtctactggagtgtcactgtcgctgcaacctatgcaccccgcaccgctccctggtttgcaattcgcagctgcttaacgaaagtcaaattatcggtacctttgagctgcagggtccctcgcctgacgaaaagtccgcggctccggggttgaaactcactccggggctgtggacgtcggcttaccttcgcaaatttgtacctgaggactaccacgcccacgagattaggttctacgaagaccaatcccgcccgcctaatgcggagcttaccgcctgcgtcattacccagggccacattcttggccaattgcaagccatcaacaaagcccgccaagagtttctgctacgaaagggacggggggtttacttggacccccagtccggcgaggagctcaacccaatccccccgccgccgcagccctatcagcagcagccgcgggcccttgcttcccaggatggcacccaaaaagaagctgcagctgccgccgccacccacggacgaggaggaatactgggacagtcaggcagaggaggttttggacgaggaggaggaggacatgatggaagactgggagagcctagacgaggaagcttccgaggtcgaagaggtgtcagacgaaacaccgtcaccctcggtcgcattcccctcgccggcgccccagaaatcggcaaccggttccagcatggctacaacctccgctcctcaggcgccgccggcactgcccgttcgccgacccaaccgtagatgggacaccactggaaccagggccggtaagtccaagcagccgccgccgttagcccaagagcaacaacagcgccaaggctaccgctcatggcgcgggcacaagaacgccatagttgcttgcttgcaagactgtgggggcaacatctccttcgcccgccgctttcttctctaccatcacggcgtggccttcccccgtaacatcctgcattactaccgtcatctctacagcccatactgcaccggcggcagcggcagcaacagcagcggccacacagaagcaaaggcgaccggatagcaagactctgacaaagcccaagaaatccacagcggcggcagcagcaggaggaggagcgctgcgtctggcgcccaacgaacccgtatcgacccgcgagcttagaaacaggatttttcccactctgtatgctatatttcaacagagcaggggccaagaacaagagctgaaaataaaaaacaggtctctgcgatccctcacccgcagctgcctgtatcacaaaagcgaagatcagcttcggcgcacgctggaagacgcggaggctctcttcagtaaatactgcgcgctgactcttaaggactagtttcgcgccctttctcaaatttaagcgcgaaaactacgtcatctccagcggccacacccggcgccagcacctgttgtcagcgccattatgagcaaggaaattcccacgccctacatgtggagttaccagccacaaatgggacttgcggctggagctgcccaagactactcaacccgaataaactacatgagcgcgggaccccacatgatatcccgggtcaacggaatacgcgcccaccgaaaccgaattctcctggaacaggcggctattaccaccacacctcgtaataaccttaatccccgtagttggcccgctgccctggtgtaccaggaaagtcccgctcccaccactgtggtacttcccagagacgcccaggccgaagttcagatgactaactcaggggcgcagcttgcgggcggctttcgtcacagggtgcggtcgcccgggcatcccaatggcgcgccgagcttggcgtaatcatggtcatagctgtttcctgtgtgaaattgttatccgctcacaattccacacaacatacgagccggaagcataaagtgtaaagcctggggtgcctaatgagtgagctaactcacattaattgcgttgcgctcactgcccgctttccagtcgggaaacctgtcgtgccagctgcattaatgaatcggccaacgcgcggggagaggcggtttgcgtattgggcgctgttccgcttcctcgctcactgactcgctgcgctcggtcgttcggctgcggcgagcggtatcagctcactcaaaggcggtaatacggttatccacagaatcaggggataacgcaggaaagaacatgtgagcaaaaggccagcaaaaggccaggaaccgtaaaaaggccgcgttgctggcgtttttccataggctccgcccccctgacgagcatcacaaaaatcgacgctcaagtcagaggtggcgaaacccgacaggactataaagataccaggcgtttccccctggaagctccctcgtgcgctctcctgttccgaccctgccgcttaccggatacctgtccgcctttctcccttcgggaagcgtggcgctttctcatagctcacgctgtaggtatctcagttcggtgtaggtcgttcgctccaagctgggctgtgtgcacgaaccccccgttcagcccgaccgctgcgccttatccggtaactatcgtcttgagtccaacccggtaagacacgacttatcgccactggcagcagccactggtaacaggattagcagagcgaggtatgtaggcggtgctacagagttcttgaagtggtggcctaactacggctacactagaagaacagtatttggtatctgcgctctgctgaagccagttaccttcggaaaaagagttggtagctcttgatccggcaaacaaaccaccgctggtagcggtggtttttttgtttgcaagcagcagattacgcgcagaaaaaaaggatctcaagaagatcctttgatcttttctacggggtctgacgctcagtggaacgaaaactcacgttaagggattttggtcatgagattatcaaaaaggatcttcacctagatccttttaaattaaaaatgaagttttaaatcaatctaaagtatatatgagtaaacttggtctgacagttaccaatgcttaatcagtgaggcacctatctcagcgatctgtctatttcgttcatccatagttgcctgactccccgtcgtgtagataactacgatacgggagggcttaccatctggccccagtgctgcaatgataccgcgagaaccacgctcaccggctccagatttatcagcaataaaccagccagccggaagggccgagcgcagaagtggtcctgcaactttatccgcctccatccagtctattaattgttgccgggaagctagagtaagtagttcgccagttaatagtttgcgcaacgttgttgccattgctacaggcatcgtggtgtcacgctcgtcgtttggtatggcttcattcagctccggttcccaacgatcaaggcgagttacatgatcccccatgttgtgcaaaaaagcggttagctccttcggtcctccgatcgttgtcagaagtaagttggccgcagtgttatcactcatggttatggcagcactgcataattctcttactgtcatgccatccgtaagatgcttttctgtgactggtgagtactcaaccaagtcattctgagaatagtgtatgcggcgaccgagttgctcttgcccggcgtcaatacgggataataccgcgccacatagcagaactttaaaagtgctcatcattggaaaacgttcttcggggcgaaaactctcaaggatcttaccgctgttgagatccagttcgatgtaacccactcgtgcacccaactgatcttcagcatcttttactttcaccagcgtttctgggtgagcaaaaacaggaaggcaaaatgccgcaaaaaagggaataagggcgacacggaaatgttgaatactcatactcttcctttttcaatattattgaagcatttatcagggttattgtctcatgagcggatacatatttgaatgtatttagaaaaataaacaaataggggttccgcgcacatttccccgaaaagtgccacctgacgtctaagaaaccattattatcatgacattaacctataaaaataggcgtatcacgaggcccttttgtc

SEQ ID NO: 11 - DNA, 5872 bp, Artificial Sequence
  plasmid
tcgcgcgtttcggtgatgacggtgaaaacctctgacacatgcagctcccggagactgtcacagcttgtctgtaagcggatgccgggagcagacaagcccgtcagggcgcgtcagcgggtgttggcgggtgtcggggctggcttaactatgcggcatcagagcagattgtactgagagtgcaccatatgcggtgtgaaataccgcacagatgcgtaaggagaaaataccgcatcaggcgccattcgccattcaggctgcgcaactgttgggaagggcgatcggtgcgggcctcttcgctattacgccagctggcgaaagggggatgtgctgcaaggcgattaagttgggtaacgccagggttttcccagtcacgacgttgtaaaacgacggccagtgaattgacgcgtattgggatggttttagggcggagtaacttgtatgtgttgggaattgtagttttcttaaaatgggaagtgacgtaacgtgggaaaacggaagtgacgatttgaggaagttgtgggttttttggctttcgtttctgggcgtaggttcgcgtgcggttttctgggtgttttttgtggactttaaccgttacgtcattttttagtcctatatatactcgctctgcacttggcccttttttacactgtgactgattgagctggtgccgtgtcgagtggtgtttttttaataggttttcttttttactggtaaggctgactgttatggctgccgctgtggaagcgctgtatgttgttctggagcgggagggtgctattttgcctaggcaggagggtttttcaggtgtttatgtgtttttctctcctattaattttgttatacctcctatgggggctgtaatgttgtctctacgcctgcgggtatgtattcccccgggctatttcggtcgctttttagcactgaccgatgtgaatcaacctgatgtgtttaccgagtcttacattatgactccggacatgaccgaggagctgtcggtggtgctttttaatcacggtgaccagtttttttacggtcacgccggcatggccgtagtccgtcttatgcttataagggttgtttttcctgttgtaagacaggcttctaatgtttaaatgtttttttgttattttattttgtgtttatgcagaaacccgcagacatgtttgagagaaaaatggtgtctttttctgtggtggttccggagcttacctgcctttatctgcatgagcatgactacgatgtgctttcttttttgcgcgaggctttgcctgattttttgagcagcaccttgcattttatatcgccgcccatgcaacaagcttacatcggggctacgctggttagcatagctccgagtatgcgtgtcataatcagtgtgggttcttttgtcatggttcctggcggggaagtggccgcgctggtccgtgcagacctgcacgattatgttcagctggccctgcgaagggacctacgggatcgcggtatttttgttaatgttccgcttttgaatcttatacaggtctgtgaggaacctgaatttttgcaatcatgattcgctgcttgaggctgaaggtggagggcgctctggagcagatttttacaatggccggacttaatattcgggatttgcttagagatatattgagaaggtggcgagatgagaattatttgggcatggttgaaggtgctggaatgtttatagaggagattcaccctgaagggtttagcctttacgtccacttggacgtgagggccgtttgccttttggaagccattgtgcaacatcttacaaatgccattatctgttctttggctgtagagtttgaccacgccaccggaggggagcgcgttcacttaatagatcttcattttgaggttttggataatcttttggaataaaaaaaaaaaacatggttcttccagctcttcccgctcctcccgtgtgtgactcgcagaacgaatgtgtaggttggctgggtgtggcttattctgcggtggtggatgttatcagggcagcggcgcatgaaggagtttacatagaacccgaagccagggggcgcctggatgctttgagagagtggatatactacaactactacacagagcgatctaagcggcgagaccggagacgcagatctgtttgtcacgcccgcacctggttttgcttcaggaaatatgactacgtccggcgttccatttggcatgacactacgaccaacacgatctcggttgtctcggcgcactccgtacagtagggatcgtctacctccttttgagacagaaacccgcgctaccatactggaggatcatccgctgctgcccgaatgtaacactttgacaatgcacaacgtgagttacgtgcgaggtcttccctgcagtgtgggatttacgctgattcaggaatgggttgttccctgggatatggttctaacgcgggaggagcttgtaatcctgaggaagtgtatgcacgtgtgcctgtgttgtgccaacattgatatcatgacgagcatgatgatccatggttacgagtcctgggctctccactgtcattgttccagtcccggttccctgcagtgtatagccggcgggcaggttttggccagctggtttaggatggtggtggatggcgccatgtttaatcagaggtttatatggtaccgggaggtggtgaattacaacatgccaaaagaggtaatgtttatgtccagcgtgtttatgaggggtcgccacttaatctacctgcgcttgtggtatgatggccacgtgggttctgtggtccccgccatgagctttggatacagcgccttgcactgtgggattttgaacaatattgtggtgctgtgctgcagttactgtgctgatttaagtgagatcagggtgcgctgctgtgcccggaggacaaggcgccttatgctgcgggcggtgcgaatcatcgctgaggagaccactgccatgttgtattcctgcaggacggagcggcggcggcagcagtttattcgcgcgctgctgcagcaccaccgccctatcctgatgcacgattatgactctacccccatgtaggcgtggacttctccttcgccgcccgttaagcaaccgcaagttggacagcagcctgtggctcagcagctggacagcgacatgaacttaagtgagctgcccggggagtttattaatatcactgatgagcgtttggctcgacaggaaaccgtgtggaatataacacctaagaatatgtctgttacccatgatatgatgctttttaaggccagccggggagaaaggactgtgtactctgtgtgttgggagggaggtggcaggttgaatactagggttctgtgagtttgattaaggtacggtgatctgtataagctatgtggtggtggggctatactactgaatgaaaaatgacttgaaattttctgcaattgaaaaataaacacgttgaaacataacacaaacgattctttattcttgggcaatgtatgaaaaagtgtaagaggatgtggcaaatatttcattaatgtagttgtggccagaccagtcccatgaaaatgacatagagtatgcacttggagttgtgtctcctgtttcctgtgtaccgtttagtgtaatggttatcccaatggcgcgccgagcttggcgtaatcatggtcatagctgtttcctgtgtgaaattgttatccgctcacaattccacacaacatacgagccggaagcataaagtgtaaagcctggggtgcctaatgagtgagctaactcacattaattgcgttgcgctcactgcccgctttccagtcgggaaacctgtcgtgccagctgcattaatgaatcggccaacgcgcggggagaggcggtttgcgtattgggcgctgttccgcttcctcgctcactgactcgctgcgctcggtcgttcggctgcggcgagcggtatcagctcactcaaaggcggtaatacggttatccacagaatcaggggataacgcaggaaagaacatgtgagcaaaaggccagcaaaaggccaggaaccgtaaaaaggccgcgttgctggcgtttttccataggctccgcccccctgacgagcatcacaaaaatcgacgctcaagtcagaggtggcgaaacccgacaggactataaagataccaggcgtttccccctggaagctccctcgtgcgctctcctgttccgaccctgccgcttaccggatacctgtccgcctttctcccttcgggaagcgtggcgctttctcatagctcacgctgtaggtatctcagttcggtgtaggtcgttcgctccaagctgggctgtgtgcacgaaccccccgttcagcccgaccgctgcgccttatccggtaactatcgtcttgagtccaacccggtaagacacgacttatcgccactggcagcagccactggtaacaggattagcagagcgaggtatgtaggcggtgctacagagttcttgaagtggtggcctaactacggctacactagaagaacagtatttggtatctgcgctctgctgaagccagttaccttcggaaaaagagttggtagctcttgatccggcaaacaaaccaccgctggtagcggtggtttttttgtttgcaagcagcagattacgcgcagaaaaaaaggatctcaagaagatcctttgatcttttctacggggtctgacgctcagtggaacgaaaactcacgttaagggattttggtcatgagattatcaaaaaggatcttcacctagatccttttaaattaaaaatgaagttttaaatcaatctaaagtatatatgagtaaacttggtctgacagttaccaatgcttaatcagtgaggcacctatctcagcgatctgtctatttcgttcatccatagttgcctgactccccgtcgtgtagataactacgatacgggagggcttaccatctggccccagtgctgcaatgataccgcgagaaccacgctcaccggctccagatttatcagcaataaaccagccagccggaagggccgagcgcagaagtggtcctgcaactttatccgcctccatccagtctattaattgttgccgggaagctagagtaagtagttcgccagttaatagtttgcgcaacgttgttgccattgctacaggcatcgtggtgtcacgctcgtcgtttggtatggcttcattcagctccggttcccaacgatcaaggcgagttacatgatcccccatgttgtgcaaaaaagcggttagctccttcggtcctccgatcgttgtcagaagtaagttggccgcagtgttatcactcatggttatggcagcactgcataattctcttactgtcatgccatccgtaagatgcttttctgtgactggtgagtactcaaccaagtcattctgagaatagtgtatgcggcgaccgagttgctcttgcccggcgtcaatacgggataataccgcgccacatagcagaactttaaaagtgctcatcattggaaaacgttcttcggggcgaaaactctcaaggatcttaccgctgttgagatccagttcgatgtaacccactcgtgcacccaactgatcttcagcatcttttactttcaccagcgtttctgggtgagcaaaaacaggaaggcaaaatgccgcaaaaaagggaataagggcgacacggaaatgttgaatactcatactcttcctttttcaatattattgaagcatttatcagggttattgtctcatgagcggatacatatttgaatgtatttagaaaaataaacaaataggggttccgcgcacatttccccgaaaagtgccacctgacgtctaagaaaccattattatcatgacattaacctataaaaataggcgtatcacgaggcccttttgtc

SEQ ID NO: 12 - DNA, 3398 bp, Artificial Sequence
  plasmid
tcgcgcgtttcggtgatgacggtgaaaacctctgacacatgcagctcccggagactgtcacagcttgtctgtaagcggatgccgggagcagacaagcccgtcagggcgcgtcagcgggtgttggcgggtgtcggggctggcttaactatgcggcatcagagcagattgtactgagagtgcaccatatgcggtgtgaaataccgcacagatgcgtaaggagaaaataccgcatcaggcgccattcgccattcaggctgcgcaactgttgggaagggcgatcggtgcgggcctcttcgctattacgccagctggcgaaagggggatgtgctgcaaggcgattaagttgggtaacgccagggttttcccagtcacgacgttgtaaaacgacggccagtgaattgacgcgtattgggatcgcccctcctgacgcggtaggaggaggggagggtgccctgcatgtctgccgctgctcttgctcttgccgctgctgaggaggggggcgcatctgccgcagcaccggatgcatctgggaaaagcaaaaaaggggctcgtccctgtttccggaggaatttgcaagcggggtcttgcatgacggggaggcaaacccccgttcgccgcagtccggccggtccgagactcgaaccgggggtcccgcgactcaacccttggaaaataaccctccggctacagggagcgagccacttaatgctttcgctttccagcctaaccgcttacgctgcgcgcggccagtggccaaaaaagctagcgcagcagccgccgcgcctggaaggaagccaaaaggagcactcccccgttgtctgacgtcgcacacctgggttcgacacgcgggcggtaaccgcatggatcacggcggacggccggatacggggctcgaaccccggtcgtccgccatgatacccttgcgaatttatccaccagaccacggaagagtgcccgcttacaggctctccttttgcacggtctagagcgtcaacgattgcgcgcgcctgaccggccagagcgtcccgaccatggagcactttttgccgctgcgcaacatctggaaccgcgtccgcgactttccgcgcgcctccaccaccgccgccggcatcacctggatgtccaggtacatctacggatatatcccaatggcgcgccgagcttggcgtaatcatggtcatagctgtttcctgtgtgaaattgttatccgctcacaattccacacaacatacgagccggaagcataaagtgtaaagcctggggtgcctaatgagtgagctaactcacattaattgcgttgcgctcactgcccgctttccagtcgggaaacctgtcgtgccagctgcattaatgaatcggccaacgcgcggggagaggcggtttgcgtattgggcgctgttccgcttcctcgctcactgactcgctgcgctcggtcgttcggctgcggcgagcggtatcagctcactcaaaggcggtaatacggttatccacagaatcaggggataacgcaggaaagaacatgtgagcaaaaggccagcaaaaggccaggaaccgtaaaaaggccgcgttgctggcgtttttccataggctccgcccccctgacgagcatcacaaaaatcgacgctcaagtcagaggtggcgaaacccgacaggactataaagataccaggcgtttccccctggaagctccctcgtgcgctctcctgttccgaccctgccgcttaccggatacctgtccgcctttctcccttcgggaagcgtggcgctttctcatagctcacgctgtaggtatctcagttcggtgtaggtcgttcgctccaagctgggctgtgtgcacgaaccccccgttcagcccgaccgctgcgccttatccggtaactatcgtcttgagtccaacccggtaagacacgacttatcgccactggcagcagccactggtaacaggattagcagagcgaggtatgtaggcggtgctacagagttcttgaagtggtggcctaactacggctacactagaagaacagtatttggtatctgcgctctgctgaagccagttaccttcggaaaaagagttggtagctcttgatccggcaaacaaaccaccgctggtagcggtggtttttttgtttgcaagcagcagattacgcgcagaaaaaaaggatctcaagaagatcctttgatcttttctacggggtctgacgctcagtggaacgaaaactcacgttaagggattttggtcatgagattatcaaaaaggatcttcacctagatccttttaaattaaaaatgaagttttaaatcaatctaaagtatatatgagtaaacttggtctgacagttaccaatgcttaatcagtgaggcacctatctcagcgatctgtctatttcgttcatccatagttgcctgactccccgtcgtgtagataactacgatacgggagggcttaccatctggccccagtgctgcaatgataccgcgagaaccacgctcaccggctccagatttatcagcaataaaccagccagccggaagggccgagcgcagaagtggtcctgcaactttatccgcctccatccagtctattaattgttgccgggaagctagagtaagtagttcgccagttaatagtttgcgcaacgttgttgccattgctacaggcatcgtggtgtcacgctcgtcgtttggtatggcttcattcagctccggttcccaacgatcaaggcgagttacatgatcccccatgttgtgcaaaaaagcggttagctccttcggtcctccgatcgttgtcagaagtaagttggccgcagtgttatcactcatggttatggcagcactgcataattctcttactgtcatgccatccgtaagatgcttttctgtgactggtgagtactcaaccaagtcattctgagaatagtgtatgcggcgaccgagttgctcttgcccggcgtcaatacgggataataccgcgccacatagcagaactttaaaagtgctcatcattggaaaacgttcttcggggcgaaaactctcaaggatcttaccgctgttgagatccagttcgatgtaacccactcgtgcacccaactgatcttcagcatcttttactttcaccagcgtttctgggtgagcaaaaacaggaaggcaaaatgccgcaaaaaagggaataagggcgacacggaaatgttgaatactcatactcttcctttttcaatattattgaagcatttatcagggttattgtctcatgagcggatacatatttgaatgtatttagaaaaataaacaaataggggttccgcgcacatttccccgaaaagtgccacctgacgtctaagaaaccattattatcatgacattaacctataaaaataggcgtatcacgaggcccttttgtc

SEQ ID NO: 13 - DNA, 11039 bp, Artificial Sequence
  plasmid
ttgagatcctttttttctgcgcgtaatctgctgcttgcaaacaaaaaaaccaccgctaccagcggtggtttgtttgccggatcaagagctaccaactctttttccgaaggtaactggcttcagcagagcgcagataccaaatactgtccttctagtgtagccgtagttaggccaccacttcaagaactctgtagcaccgcctacatacctcgctctgctaatcctgttaccagtggctgctgccagtggcgataagtcgtgtcttaccgggttggactcaagacgatagttaccggataaggcgcagcggtcgggctgaacggggggttcgtgcacacagcccagcttggagcgaacgacctacaccgaactgagatacctacagcgtgagctatgagaaagcgccacgcttcccgaagggagaaaggcggacaggtatccggtaagcggcagggtcggaacaggagagcgcacgagggagcttccagggggaaacgcctggtatctttatagtcctgtcgggtttcgccacctctgacttgagcgtcgatttttgtgatgctcgtcaggggggcggagcctatggaaaaacgccagcaacgcggcctttttacggttcctggccttttgctggccttttgctcacatgttctttcctgcgttatcccctgattctgtggataaccgtattaccgccatgcatagatctaaatgagtcttcggacctcgcgggggccgcttaagcggtggttagggtttgtctgacgcggggggagggggaaggaacgaaacactctcattcggaggcggctcggggtttggtcttggtggccacgggcacgcagaagagcgccgcgatcctcttaagcacccccccgccctccgtggaggcgggggtttggtcggcgggtggtaactggcgggccgctgactcgggcgggtcgcgcgccccagagtgtgaccttttcggtctgctcgcagacccccgggcggcgccgccgcggcggcgacgggctcgctgggtcctaggctccatggggaccgtatacgtggacaggctctggagcatccgcacgactgcggtgatattaccggagaccttctgcgggacgagccgggtcacgcggctgacgcggagcgtccgttgggcgacaaacaccaggacggggcacaggtacactatcttgtcacccggaggcgcgagggactgcaggagcttcagggagtggcgcagctgcttcatccccgtggcccgttgctcgcgtttgctggcggtgtccccggaagaaatatatttgcatgtctttagttctatgatgacacaaaccccgcccagcgtcttgtcattggcgaattcgaacacgcagatgcagtcggggcggcgcggtcccaggtccacttcgcatattaaggtgacgcgtgtggcctcgaacaccgagcgaccctgcagcgacccgcttaaaagcttgattcttctgacacaacagtctcgaacttaagctgcagaagttggtcgtgaggcactgggcaggtaagtatcaaggttacaagacaggtttaaggagaccaatagaaactgggcttgtcgagacagagaagactcttgcgtttctgataggcacctattggtcttactgacatccactttgcctttctctccacaggtgtccactcccagttcaattacagctcttaaggctagagtacttaatacgactcactataggctagcctggcttgaggctcaggacgcaaatcttgaggatgttcagcgggagttttccgggctgcgagtaattggtgatgaggacgaggatggttcggaggatggggaattttcagacctggatctgtctgacagcgaccatgaaggggatgagggtgggggggctgttggagggggcaggagtctgcactccctgtattcactgagcgtcgtctaataaagatgtctattgatctcttttagtgtgaatcatgtctgacgaggggccaggtacaggacctggaaatggcctaggagagaagggagacacatctggaccagaaggctccggcggcagtggacctcaaagaagagggggtgataaccatggacgaggacggggaagaggacgaggacgaggaggcggaagaccaggagccccgggcggctcaggatcagggccaagacatagagatggtgtccggagaccccaaaaacgtccaagttgcattggctgcaaagggacccacggtggaacaggagcaggagcaggagcgggaggggcaggagcaggaggggcaggagcaggaggaggggcaggagcaggaggaggggcaggaggggcaggaggggcaggaggggcaggagcaggaggaggggcaggagcaggaggaggggcaggaggggcaggaggggcaggagcaggaggaggggcaggagcaggaggaggggcaggaggggcaggagcaggaggaggggcaggaggggcaggaggggcaggagcaggaggaggggcaggagcaggaggaggggcaggaggggcaggagcaggaggaggggcaggaggggcaggaggggcaggagcaggaggaggggcaggagcaggaggggcaggaggggcaggaggggcaggagcaggaggggcaggagcaggaggaggggcaggaggggcaggaggggcaggagcaggaggggcaggagcaggaggggcaggagcaggaggggcaggagcaggaggggcaggaggggcaggagcaggaggggcaggaggggcaggagcaggaggggcaggaggggcaggagcaggaggaggggcaggaggggcaggagcaggaggaggggcaggaggggcaggagcaggaggggcaggaggggcaggagcaggaggggcaggaggggcaggagcaggaggggcaggaggggcaggagcaggaggaggggcaggagcaggaggggcaggagcaggaggtggaggccggggtcgaggaggcagtggaggccggggtcgaggaggtagtggaggccggggtcgaggaggtagtggaggccgccggggtagaggacgtgaaagagccagggggggaagtcgtgaaagagccagggggagaggtcgtggacgtggagaaaagaggcccaggagtcccagtagtcagtcatcatcatccgggtctccaccgcgcaggccccctccaggtagaaggccatttttccaccctgtaggggaagccgattattttgaataccaccaagaaggtggcccagatggtgagcctgacgtgcccccgggagcgatagagcagggccccgcagatgacccaggagaaggcccaagcactggaccccggggtcagggtgatggaggcaggcgcaaaaaaggagggtggtttggaaagcatcgtggtcaaggaggttccaacccgaaatttgagaacattgcagaaggtttaagagctctcctggctaggagtcacgtagaaaggactaccgacgaaggaacttgggtcgccggtgtgttcgtatatggaggtagtaagacctccctttacaacctaaggcgaggaactgcccttgctattccacaatgtcgtcttacaccattgagtcgtctcccctttggaatggcccctggacccggcccacaacctggcccgctaagggagtccattgtctgttatttcatggtctttttacaaactcatatatttgctgaggttttgaaggatgcgattaaggaccttgttatgacaaagcccgctcctacctgcaatatcagggtgactgtgtgcagctttgacgatggagtagatttgcctccctggtttccacctatggtggaaggggctgccgcggagggtgatgacggagatgacggagatgaaggaggtgatggagatgagggtgaggaagggcaggagtgatgtaacttgttaggagacgccctcaatcgtattaaaagccgtgtattcccccgcactaaagaataaatccccagtagacatcatgcgtgctgttggtgtatttctggccatctgtcttgtcaccattttcgtcctcccaacatggggcaattgggcatacccatgttgtcacgtcactcagctccgcgctcaacaccttctcgcgttggaaaacattagcgacatttacctggtgagcaatcagacatgcgacggctttagcctggcctccttaaattcacctaagaatgggagcaaccagcaggaaaaggacaagcagcgaaaattcacgcccccttgggaggtggcggcatatgcaaaggatagcactcccactctactactgggtatcatatgctgactgtatatgcatgaggatagcatatgctacccggatacagattaggatagcatatactacccagatatagattaggatagcatatgctacccagatatagattaggatagcctatgctacccagatataaattaggatagcatatactacccagatatagattaggatagcatatgctacccagatatagattaggatagcctatgctacccagatatagattaggatagcatatgctacccagatatagattaggatagcatatgctatccagatatttgggtagtatatgctacccagatataaattaggatagcatatactaccctaatctctattaggatagcatatgctacccggatacagattaggatagcatatactacccagatatagattaggatagcatatgctacccagatatagattaggatagcctatgctacccagatataaattaggatagcatatactacccagatatagattaggatagcatatgctacccagatatagattaggatagcctatgctacccagatatagattaggatagcatatgctatccagatatttgggtagtatatgctacccatggcaacattagcccaccgtgctctcagcgacctcgtgaatatgaggaccaacaaccctgtgcttggcgctcaggcgcaagtgtgtgtaatttgtcctccagatcgcagcaatcgcgcccctatcttggcccgcccacctacttatgcaggtattccccggggtgccattagtggttttgtgggcaagtggtttgaccgcagtggttagcggggttacaatcagccaagttattacacccttattttacagtccaaaaccgcagggcggcgtgtgggggctgacgcgatcgctgttccttaggacccttttactaaccctaattcgatagcatatgcttcccgttgggtaacatatgctattgaattagggttagtctggatagtatatactactacccgggaagcatatgctacccgtttagggttaacaagggggccttataaacactattgctaatgccctcttgagggtccgcttatcggtagctacacaggcccctctgattgacgttggtgtagcctcccgtagtcttcctgggcccctgggaggtacatgtcccccagcattggtgtaagagcttcagccaagagttacacataaaggcaatgttgtgttgcagtccacagactgcaaagtctgctccaggatgaaagccactcagtgttggcaaatgtgcacatccatttataaggatgtcaactacagtcagagaacccctttgtgtttggtccccccccgtgtcacatgtggaacagggcccagttggcaagttgtaccaaccaactgaagggattacatgcactgccccgcgaagaaggggcagagatgtcgtagtcaggtttagttcgtccggggcggggatctcgacattgattattgactagttattaatagtaatcaattacggggtcattagttcatagcccatatatggagttccgcgttacataacttacggtaaatggcccgcctggctgaccgcccaacgacccccgcccattgacgtcaataatgacgtatgttcccatagtaacgccaatagggactttccattgacgtcaatgggtggagtatttacggtaaactgcccacttggcagtacatcaagtgtatcatatgccaagtacgccccctattgacgtcaatgacggtaaatggcccgcctggcattatgcccagtacatgaccttatgggactttcctacttggcagtacatctacgtattagtcatcgctattaccatggtcgaggtgagccccacgttctgcttcactctccccatctcccccccctccccacccccaattttgtatttatttattttttaattattttgtgcagcgatgggggcggggggggggggggggcgcgcgccaggcggggcggggcggggcgaggggcggggcggggcgaggcggagaggtgcggcggcagccaatcagagcggcgcgctccgaaagtttccttttatggcgaggcggcggcggcggcggccctataaaaagcgaagcgcgcggcgggcgggagtcgctgcgcgttgccctcgccccgtgccccgctccgccgccgcctcgcgccgcccgccccggctctgactgaccgcgttactcccacaggtgagcgggcgggacggcccttctcctccgggctgtaattagcgcttggtttaatgacggcttgtttcttttctgtggctgcgtgaaagccttgaggggctccgggagggccctttgtgcggggggagcggctcggggggtgcgtgcgtgtgtgtgtgcgtggggagcgccgcgtgcggctccgcgctgcccggcggctgtgagcgctgcgggcgcggcgcggggctttgtgcgctccgcagtgtgcgcgaggggagcgcggccgggggcggtgccccgcggtgcggggggggctgcgaggggaacaaaggctgcgtgcggggtgtgtgcgtgggggggtgagcagggggtgtgggcgcgtcggtcgggctgcaaccccccctgcacccccctccccgagttgctgagcacggcccggcttcgggtgcggggctccgtacggggcgtggcgcggggctcgccgtgccgggcggggggtggcggcaggtgggggtgccgggcggggcggggccgcctcgggccggggagggctcgggggaggggcgcggcggcccccggagcgccggcggctgtcgaggcgcggcgagccgcagccattgccttttatggtaatcgtgcgagagggcgcagggacttcctttgtcccaaatctgtgcggagccgaaatctgggaggcgccgccgcaccccctctagcgggcgcggggcgaagcggtgcggcgccggcaggaaggaaatgggcggggagggccttcgtgcgtcgccgcgccgccgtccccttctccctctccagcctcggggctgtccgcggggggacggctgccttcgggggggacggggcagggcggggttcggcttctggcgtgtgaccggcggctctagagcctctgctaaccatgttcatgccttcttctttttcctacagctcctgggcaacgtgctggttattgtgctgtctcatcattttggcaaagaattaaccctcactaaaggggtaccgggccccccctcgaatgactacgtccggcgttccatttggcatgacactacgaccaacacgatctcggttgtctcggcgcactccgtacagtagggatcgcctacctccttttgagacagagacccgcgctaccatactggaggatcatccgctgctgcccgaatgtaacactttgacaatgcacaacgtgagttacgtgcgaggtcttccctgcagtgtgggatttacgctgattcaggaatgggttgttccctgggatatggttctgacgcgggaggagcttgtaatcctgaggaagtgtatgcacgtgtgcctgtgttgtgccaacattgatatcatgacgagcatgatgatccatggttacgagtcctgggctctccactgtcattgttccagtcccggttccctgcagtgcatagccggcgggcaggttttggccagctggtttaggatggtggtggatggcgccatgtttaatcagaggtttatatggtaccgggaggtggtgaattacaacatgccaaaagaggtaatgtttatgtccagcgtgtttatgaggggtcgccacttaatctacctgcgcttgtggtatgatggccacgtgggttctgtggtccccgccatgagctttggatacagcgccttgcactgtgggattttgaacaatattgtggtgctgtgctgcagttactgtgctgatttaagtgagatcagggtgcgctgctgtgcccggaggacaaggcgtctcatgctgcgggcggtgcgaatcatcgctgaggagaccactgccatgttgtattcctgcaggacggagcggcggcggcagcagtttattcgcgcgctgctgcagcaccaccgccctatcctgatgcacgattatgactctacccccatgggccgcgactctagatcataatcagccataccacatttgtagaggttttacttgctttaaaaaacctcccacacctccccctgaacctgaaacataaaatgaatgcaattgttgttgttaacttgtttattgcagcttataatggttacaaataaagcaatagcatcacaaatttcacaaataaagcatttttttcactgcattctagttgtggtttgtccaaactcatcaatgtatcttaaggcgtaaattgtaagcgttaatattttgttaaaattcgcgttaaatttttgttaaatcagctcattttttaaccaataggccgaaatcggcaaaatcccttataaatcaaaagaatagaccgagatagggttgagtgttgttccagtttggaacaagagtccactattaaagaacgtggactccaacgtcaaagggcgaaaaaccgtctatcagggcgatggcccactacgtgaaccatcaccctaatcaagttttttggggtcgaggtgccgtaaagcactaaatcggaaccctaaagggagcccccgatttagagcttgacggggaaagccggcgaacgtggcgagaaaggaagggaagaaagcgaaaggagcgggcgctagggcgctggcaagtgtagcggtcacgctgcgcgtaaccaccacacccgccgcgcttaatgcgccgctacagggcgcgtcaggtggcacttttcggggaaatgtgcgcggaacccctatttgtttatttttctaaatacattcaaatatgtatccgctcatgagacaataaccctgataaatgcttcaataatattgaaaaaggaagagtcctgaggcggaaagaaccagctgtggaatgtgtgtcagttagggtgtggaaagtccccaggctccccagcaggcagaagtatgcaaagcatgcatctcaattagtcagcaaccaggtgtggaaagtccccaggctccccagcaggcagaagtatgcaaagcatgcatctcaattagtcagcaaccatagtcccgcccctaactccgcccatcccgcccctaactccgcccagttccgcccattctccgccccatggctgactaattttttttatttatgcagaggccgaggccgcctcggcctctgagctattccagaagtagtgaggaggcttttttggaggcctaggcttttgcaaagatcatcaagagacaggatgaggatcgtttcgcatgattgaacaagatggattgcacgcaggttctccggccgcttgggtggagaggctattcggctatgactgggcacaacagacaatcggctgctctgatgccgccgtgttccggctgtcagcgcaggggcgcccggttctttttgtcaagaccgacctgtccggtgccctgaatgaactgcaagacgaggcagcgcggctatcgtggctggccacgacgggcgttccttgcgcagctgtgctcgacgttgtcactgaagcgggaagggactggctgctattgggcgaagtgccggggcaggatctcctgtcatctcaccttgctcctgccgagaaagtatccatcatggctgatgcaatgcggcggctgcatacgcttgatccggctacctgcccattcgaccaccaagcgaaacatcgcatcgagcgagcacgtactcggatggaagccggtcttgtcgatcaggatgatctggacgaagagcatcaggggctcgcgccagccgaactgttcgccaggctcaaggcgagcatgcccgacggcgaggatctcgtcgtgacccatggcgatgcctgcttgccgaatatcatggtggaaaatggccgcttttctggattcatcgactgtggccggctgggtgtggcggaccgctatcaggacatagcgttggctacccgtgatattgctgaagagcttggcggcgaatgggctgaccgcttcctcgtgctttacggtatcgccgctcccgattcgcagcgcatcgccttctatcgccttcttgacgagttcttctgagcgggactctggggttcgaaatgaccgaccaagcgacgcccaacctgccatcacgagatttcgattccaccgccgccttctatgaaaggttgggcttcggaatcgttttccgggacgccggctggatgatcctccagcgcggggatctcatgctggagttcttcgcccaccctagggggaggctaactgaaacacggaaggagacaataccggaaggaacccgcgctatgacggcaataaaaagacagaataaaacgcacggtgttgggtcgtttgttcataaacgcggggttcggtcccagggctggcactctgtcgataccccaccgagaccccattggggccaatacgcccgcgtttcttccttttccccaccccaccccccaagttcgggtgaaggcccagggctcgcagccaacgtcggggcggcaggccctgccatagcctcaggttactcatatatactttagattgatttaaaacttcatttttaatttaaaaggatctaggtgaagatcctttttgataatctcatgaccaaaatcccttaacgtgagttttcgttccactgagcgtcagaccccgtagaaaagatcaaaggatcttc

SEQ ID NO: 14 - DNA, 11481 bp, Artificial Sequence
  plasmid
ggtacccaactccatgcttaacagtccccaggtacagcccaccctgcgtcgcaaccaggaacagctctacagcttcctggagcgccactcgccctacttccgcagccacagtgcgcagattaggagcgccacttctttttgtcacttgaaaaacatgtaaaaataatgtactaggagacactttcaataaaggcaaatgtttttatttgtacactctcgggtgattatttaccccccacccttgccgtctgcgccgtttaaaaatcaaaggggttctgccgcgcatcgctatgcgccactggcagggacacgttgcgatactggtgtttagtgctccacttaaactcaggcacaaccatccgcggcagctcggtgaagttttcactccacaggctgcgcaccatcaccaacgcgtttagcaggtcgggcgccgatatcttgaagtcgcagttggggcctccgccctgcgcgcgcgagttgcgatacacagggttgcagcactggaacactatcagcgccgggtggtgcacgctggccagcacgctcttgtcggagatcagatccgcgtccaggtcctccgcgttgctcagggcgaacggagtcaactttggtagctgccttcccaaaaagggtgcatgcccaggctttgagttgcactcgcaccgtagtggcatcagaaggtgaccgtgcccggtctgggcgttaggatacagcgcctgcatgaaagccttgatctgcttaaaagccacctgagcctttgcgccttcagagaagaacatgccgcaagacttgccggaaaactgattggccggacaggccgcgtcatgcacgcagcaccttgcgtcggtgttggagatctgcaccacatttcggccccaccggttcttcacgatcttggccttgctagactgctccttcagcgcgcgctgcccgttttcgctcgtcacatccatttcaatcacgtgctccttatttatcataatgctcccgtgtagacacttaagctcgccttcgatctcagcgcagcggtgcagccacaacgcgcagcccgtgggctcgtggtgcttgtaggttacctctgcaaacgactgcaggtacgcctgcaggaatcgccccatcatcgtcacaaaggtcttgttgctggtgaaggtcagctgcaacccgcggtgctcctcgtttagccaggtcttgcatacggccgccagagcttccacttggtcaggcagtagcttgaagtttgcctttagatcgttatccacgtggtacttgtccatcaacgcgcgcgcagcctccatgcccttctcccacgcagacacgatcggcaggctcagcgggtttatcaccgtgctttcactttccgcttcactggactcttccttttcctcttgcgtccgcataccccgcgccactgggtcgtcttcattcagccgccgcaccgtgcgcttacctcccttgccgtgcttgattagcaccggtgggttgctgaaacccaccatttgtagcgccacatcttctctttcttcctcgctgtccacgatcacctctggggatggcgggcgctcgggcttgggagaggggcgcttctttttctttttggacgcaatggccaaatccgccgtcgaggtcgatggccgcgggctgggtgtgcgcggcaccagcgcatcttgtgacgagtcttcttcgtcctcggactcgagacgccgcctcagccgcttttttgggggcgcgcggggaggcggcggcgacggcgacggggacgacacgtcctccatggttggtggacgtcgcgccgcaccgcgtccgcgctcgggggtggtttcgcgctgctcctcttcccgactggccatttccttctcctataggcagaaaaagatcatggagtcagtcgagaaggaggacagcctaaccgccccctttgagttcgccaccaccgcctccaccgatgccgccaacgcgcctaccaccttccccgtcgaggcacccccgcttgaggaggaggaagtgattatcgagcaggacccaggttttgtaagcgaagacgacgaggatcgctcagtaccaacagaggataaaaagcaagaccaggacgacgcagaggcaaacgaggaacaagtcgggcggggggaccaaaggcatggcgactacctagatgtgggagacgacgtgctgttgaagcatctgcagcgccagtgcgccattatctgcgacgcgttgcaagagcgcagcgatgtgcccctcgccatagcggatgtcagccttgcctacgaacgccacctgttctcaccgcgcgtaccccccaaacgccaagaaaacggcacatgcgagcccaacccgcgcctcaacttctaccccgtatttgccgtgccagaggtgcttgccacctatcacatctttttccaaaactgcaagatacccctatcctgccgtgccaaccgcagccgagcggacaagcagctggccttgcggcagggcgctgtcatacctgatatcgcctcgctcgacgaagtgccaaaaatctttgagggtcttggacgcgacgagaaacgcgcggcaaacgctctgcaacaagaaaacagcgaaaatgaaagtcactgtggagtgctggtggaacttgagggtgacaacgcgcgcctagccgtgctgaaacgcagcatcgaggtcacccactttgcctacccggcacttaacctaccccccaaggttatgagcacagtcatgagcgagctgatcgtgcgccgtgcacgacccctggagagggatgcaaacttgcaagaacaaaccgaggagggcctacccgcagttggcgatgagcagctggcgcgctggcttgagacgcgcgagcctgccgacttggaggagcgacgcaagctaatgatggccgcagtgcttgttaccgtggagcttgagtgcatgcagcggttctttgctgacccggagatgcagcgcaagctagaggaaacgttgcactacacctttcgccagggctacgtgcgccaggcctgcaaaatttccaacgtggagctctgcaacctggtctcctaccttggaattttgcacgaaaaccgcctcgggcaaaacgtgcttcattccacgctcaagggcgaggcgcgccgcgactacgtccgcgactgcgtttacttatttctgtgctacacctggcaaacggccatgggcgtgtggcagcaatgcctggaggagcgcaacctaaaggagctgcagaagctgctaaagcaaaacttgaaggacctatggacggccttcaacgagcgctccgtggccgcgcacctggcggacattatcttccccgaacgcctgcttaaaaccctgcaacagggtctgccagacttcaccagtcaaagcatgttgcaaaactttaggaactttatcctagagcgttcaggaattctgcccgccacctgctgtgcgcttcctagcgactttgtgcccattaagtaccgtgaatgccctccgccgctttggggtcactgctaccttctgcagctagccaactaccttgcctaccactccgacatcatggaagacgtgagcggtgacggcctactggagtgtcactgtcgctgcaacctatgcaccccgcaccgctccctggtctgcaattcgcaactgcttagcgaaagtcaaattatcggtacctttgagctgcagggtccctcgcctgacgaaaagtccgcggctccggggttgaaactcactccggggctgtggacgtcggcttaccttcgcaaatttgtacctgaggactaccacgcccacgagattaggttctacgaagaccaatcccgcccgccaaatgcggagcttaccgcctgcgtcattacccagggccacatccttggccaattgcaagccatcaacaaagcccgccaagagtttctgctacgaaagggacggggggtttacctggacccccagtccggcgaggagctcaacccaatccccccgccgccgcagccctatcagcagccgcgggcccttgcttcccaggatggcacccaaaaagaagctgcagctgccgccgccgccacccacggacgaggaggaatactgggacagtcaggcagaggaggttttggacgaggaggaggagatgatggaagactgggacagcctagacgaagcttccgaggccgaagaggtgtcagacgaaacaccgtcaccctcggtcgcattcccctcgccggcgccccagaaattggcaaccgttcccagcatcgctacaacctccgctcctcaggcgccgccggcactgcctgttcgccgacccaaccgtagatgggacaccactggaaccagggccggtaagtctaagcagccgccgccgttagcccaagagcaacaacagcgccaaggctaccgctcgtggcgcgggcacaagaacgccatagttgcttgcttgcaagactgtgggggcaacatctccttcgcccgccgctttcttctctaccatcacggcgtggccttcccccgtaacatcctgcattactaccgtcatctctacagcccctactgcaccggcggcagcggcagcggcagcaacagcagcggtcacacagaagcaaaggcgaccggatagcaagactctgacaaagcccaagaaatccacagcggcggcagcagcaggaggaggagcgctgcgtctggcgcccaacgaacccgtatcgacccgcgagcttagaaataggatttttcccactctgtatgctatatttcaacaaagcaggggccaagaacaagagctgaaaataaaaaacaggtctctgcgctccctcacccgcagctgcctgtatcacaaaagcgaagatcagcttcggcgcacgctggaagacgcggaggctctcttcagcaaatactgcgcgctgactcttaaggactagtttcgcgccctttctcaaatttaagcgcgaaaactacgtcatctccagcggccacacccggcgccagcacctgtcgtcagcgccattatgagcaaggaaattcccacgccctacatgtggagttaccagccacaaatgggacttgcggctggagctgcccaagactactcaacccgaataaactacatgagcgcgggaccccacatgatatcccgggtcaacggaatccgcgcccaccgaaaccgaattctcctcgaacaggcggctattaccaccacacctcgtaataaccttaatccccgtagttggcccgctgccctggtgtaccaggaaagtcccgctcccaccactgtggtacttcccagagacgcccaggccgaagttcagatgactaactcaggggcgcagcttgcgggcggctttcgtcacagggtgcggtcgcccgggcgttttagggcggagtaacttgcatgtattgggaattgtagtttttttaaaatgggaagtgacgtatcgtgggaaaacggaagtgaagatttgaggaagttgtgggttttttggctttcgtttctgggcgtaggttcgcgtgcggttttctgggtgttttttgtggactttaaccgttacgtcattttttagtcctatatatactcgctctgtacttggccctttttacactgtgactgattgagctggtgccgtgtcgagtggtgttttttaataggtttttttactggtaaggctgactgttatggctgccgctgtggaagcgctgtatgttgttctggagcgggagggtgctattttgcctaggcaggagggtttttcaggtgtttatgtgtttttctctcctattaattttgttatacctcctatgggggctgtaatgttgtctctacgcctgcgggtatgtattcccccgggctatttcggtcgctttttagcactgaccgatgttaaccaacctgatgtgtttaccgagtcttacattatgactccggacatgaccgaggaactgtcggtggtgctttttaatcacggtgaccagtttttttacggtcacgccggcatggccgtagtccgtcttatgcttataagggttgtttttcctgttgtaagacaggcttctaatgtttaaatgtttttttttttgttattttattttgtgtttaatgcaggaacccgcagacatgtttgagagaaaaatggtgtctttttctgtggtggttccggaacttacctgcctttatctgcatgagcatgactacgatgtgcttgcttttttgcgcgaggctttgcctgattttttgagcagcaccttgcattttatatcgccgcccatgcaacaagcttacataggggctacgctggttagcatagctccgagtatgcgtgtcataatcagtgtgggttcttttgtcatggttcctggcggggaagtggccgcgctggtccgtgcagacctgcacgattatgttcagctggccctgcgaagggacctacgggatcgcggtatttttgttaatgttccgcttttgaatcttatacaggtctgtgaggaacctgaatttttgcaatcatgattcgctgcttgaggctgaaggtggagggcgctctggagcagatttttacaatggccggacttaatattcgggatttgcttagagacatattgataaggtggcgagatgaaaattatttgggcatggttgaaggtgctggaatgtttatagaggagattcaccctgaagggtttagcctttacgtccacttggacgtgagggcagtttgccttttggaagccattgtgcaacatcttacaaatgccattatctgttctttggctgtagagtttgaccacgccaccggaggggagcgcgttcacttaatagatcttcattttgaggttttggataatcttttggaataaaaaaaaaaaaacatggttcttccagctcttcccgctcctcccgtgtgtgactcgcagaacgaatgtgtaggttggctgggtgtggcttattctgcggtggtggatgttatcagggcagcggcgcatgaaggagtttacatagaacccgaagccagggggcgcctggatgctttgagagagtggatatactacaactactacacagagcgagctaagcgacgagaccggagacgcagatctgtttgtcacgcccgcacctggttttgcttcaggaaatatgactacgtccggcgttccatttggcatgacactacgaccaacacgatctcggttgtctcggcgcactccgtacagtagggatcgcctacctccttttgagacagagacccgcgctaccatactggaggatcatccgctgctgcccgaatgtaacactttgacaatgcacaacgtgagttacgtgcgaggtcttccctgcagtgtgggatttacgctgattcaggaatgggttgttccctgggatatggttctgacgcgggaggagcttgtaatcctgaggaagtgtatgcacgtgtgcctgtgttgtgccaacattgatatcatgacgagcatgatgatccatggttacgagtcctgggctctccactgtcattgttccagtcccggttccctgcagtgcatagccggcgggcaggttttggccagctggtttaggatggtggtggatggcgccatgtttaatcagaggtttatatggtaccgggaggtggtgaattacaacatgccaaaagaggtaatgtttatgtccagcgtgtttatgaggggtcgccacttaatctacctgcgcttgtggtatgatggccacgtgggttctgtggtccccgccatgagctttggatacagcgccttgcactgtgggattttgaacaatattgtggtgctgtgctgcagttactgtgctgatttaagtgagatcagggtgcgctgctgtgcccggaggacaaggcgtctcatgctgcgggcggtgcgaatcatcgctgaggagaccactgccatgttgtattcctgcaggacggagcggcggcggcagcagtttattcgcgcgctgctgcagcaccaccgccctatcctgatgcacgattatgactctacccccatgtaggcgtggacttccccttcgccgcccgttgagcaaccgcaagttggacagcagcctgtggctcagcagctggacagcgacatgaacttaagcgagctgcccggggagtttattaatatcactgatgagcgtttggctcgacaggaaaccgtgtggaatataacacctaagaatatgtctgttacccatgatatgatgctttttaaggccagccggggagaaaggactgtgtactctgtgtgttgggagggaggtggcaggttgaatactagggttctgtgagtttgattaaggtacggtgatcaatataagctatgtggtggtggggctatactactgaatgaaaaatgacttgaaattttctgcaattgaaaaataaacacgttgaaacataacatgcaacaggttcacgattctttattcctgggcaatgtaggagaaggtgtaagagttggtagcaaaagtttcagtggtgtattttccactttcccaggaccatgtaaaagacatagagtaagtgcttacctcgctagtttctgtggattcactagaatcgatgtaggatgttgcccctctgacgcggtaggagaaggggagggtgccctgcatgtctgccgctgctcttgctcttgccgctgctgaggaggggggcgcatctgccgcagcaccggatgcatctgggaaaagcaagcggccgcacttaatgctttcgctttccagcctaaccgcttacgccgcgcgcggccagtggccaaaaaagctagcgcagcagccgccgcgcctggaaggaagccaaaaggagcgctcccccgttgtctgacgtcgcacacctgggttcgacacgcgggcggtaaccgcatggatcacggcggacggccggatccggggttcgaaccccggtcgtccgccatgatacccttgcgaatttatccaccagaccacggaagagtgcccgcttacaggctctccttttgcacggtctagagcgtcaacgactgcgcacgcctcaccggccagagcgtcccgaccatggagcactttttgccgctgcgcaacatctggaaccgcgtccgcgactttccgcgcgcctccaccaccgccgccggcatcacctggatgtccaggtacatctacggattacgtcgacgtttaaaccatatgatcagctcactcaaaggcggtaatacggttatccacagaatcaggggataacgcaggaaagaacatgtgagcaaaaggccagcaaaaggccaggaaccgtaaaaaggccgcgttgctggcgtttttccataggctccgcccccctgacgagcatcacaaaaatcgacgctcaagtcagaggtggcgaaacccgacaggactataaagataccaggcgtttccccctggaagctccctcgtgcgctctcctgttccgaccctgccgcttaccggatacctgtccgcctttctcccttcgggaagcgtggcgctttctcatagctcacgctgtaggtatctcagttcggtgtaggtcgttcgctccaagctgggctgtgtgcacgaaccccccgttcagcccgaccgctgcgccttatccggtaactatcgtcttgagtccaacccggtaagacacgacttatcgccactggcagcagccactggtaacaggattagcagagcgaggtatgtaggcggtgctacagagttcttgaagtggtggcctaactacggctacactagaagaacagtatttggtatctgcgctctgctgaagccagttaccttcggaaaaagagttggtagctcttgatccggcaaacaaaccaccgctggtagcggtggtttttttgtttgcaagcagcagattacgcgcagaaaaaaaggatctcaagaagatcctttgatcttttctacggggtctgacgctcagtggaacgaaaactcacgttaagggattttggtcatgagattatcaaaaaggatcttcacctagatccttttaaattaaaaatgaagttttaaatcaatctaaagtatatatgagtaaacttggtctgacagttaccaatgcttaatcagtgaggcacctatctcagcgatctgtctatttcgttcatccatagttgcctgactccccgtcgtgtagataactacgatacgggagggcttaccatctggccccagtgctgcaatgataccgcgagacccacgctcaccggctccagatttatcagcaataaaccagccagccggaagggccgagcgcagaagtggtcctgcaactttatccgcctccatccagtctattaattgttgccgggaagctagagtaagtagttcgccagttaatagtttgcgcaacgttgttgccattgctacaggcatcgtggtgtcacgctcgtcgtttggtatggcttcattcagctccggttcccaacgatcaaggcgagttacatgatcccccatgttgtgcaaaaaagcggttagctccttcggtcctccgatcgttgtcagaagtaagttggccgcagtgttatcactcatggttatggcagcactgcataattctcttactgtcatgccatccgtaagatgcttttctgtgactggtgagtactcaaccaagtcattctgagaatagtgtatgcggcgaccgagttgctcttgcccggcgtcaatacgggataataccgcgccacatagcagaactttaaaagtgctcatcattggaaaacgttcttcggggcgaaaactctcaaggatcttaccgctgttgagatccagttcgatgtaacccactcgtgcacccaactgatcttcagcatcttttactttcaccagcgtttctgggtgagcaaaaacaggaaggcaaaatgccgcaaaaaagggaataagggcgacacggaaatgttgaatactcatactcttcctttttcaatattattgaagcatttatcagggttattgtctcatgagcggatacatatttgaatgtatttagaaaaataaacaaataggggttccgcgcacatttccccgaaaagtgccacctaaattgtaagcgttaatattttgttaaaattcgcgttaaatttttgttaaatcagctcattttttaaccaataggccgaaatcggcaaaatcccttataaatcaaaagaatagaccgagatagggttgagtgttgttccagtttggaacaagagtccactattaaagaacgtggactccaacgtcaaagggcgaaaaaccgtctatcagggcgatggcccactacgtgaaccatcaccctaatcaagttttttggggtcgaggtgccgtaaagcactaaatcggaaccctaaagggagcccccgatttagagcttgacggggaaagccggcgaacgtggcgagaaaggaagggaagaaagcgaaaggagcgggcgctagggcgctggcaagtgtagcggtcacgctgcgcgtaaccaccacacccgccgcgcttaatgcgccgctacagggcgcgatggatcc

SEQ ID NO: 15 - DNA, 11483 bp, Artificial Sequence
  plasmid
ggtacccaactccatgcttaacagtccccaggtacagcccaccctgcgtcgcaaccaggaacagctctacagcttcctggagcgccactcgccctacttccgcagccacagtgcgcagattaggagcgccacttctttttgtcacttgaaaaacatgtaaaaataatgtactaggagacactttcaataaaggcaaatgtttttatttgtacactctcgggtgattatttaccccccacccttgccgtctgcgccgtttaaaaatcaaaggggttctgccgcgcatcgctatgcgccactggcagggacacgttgcgatactggtgtttagtgctccacttaaactcaggcacaaccatccgcggcagctcggtgaagttttcactccacaggctgcgcaccatcaccaacgcgtttagcaggtcgggcgccgatatcttgaagtcgcagttggggcctccgccctgcgcgcgcgagttgcgatacacagggttgcagcactggaacactatcagcgccgggtggtgcacgctggccagcacgctcttgtcggagatcagatccgcgtccaggtcctccgcgttgctcagggcgaacggagtcaactttggtagctgccttcccaaaaagggtgcatgcccaggctttgagttgcactcgcaccgtagtggcatcagaaggtgaccgtgcccggtctgggcgttaggatacagcgcctgcatgaaagccttgatctgcttaaaagccacctgagcctttgcgccttcagagaagaacatgccgcaagacttgccggaaaactgattggccggacaggccgcgtcatgcacgcagcaccttgcgtcggtgttggagatctgcaccacatttcggccccaccggttcttcacgatcttggccttgctagactgctccttcagcgcgcgctgcccgttttcgctcgtcacatccatttcaatcacgtgctccttatttatcataatgctcccgtgtagacacttaagctcgccttcgatctcagcgcagcggtgcagccacaacgcgcagcccgtgggctcgtggtgcttgtaggttacctctgcaaacgactgcaggtacgcctgcaggaatcgccccatcatcgtcacaaaggtcttgttgctggtgaaggtcagctgcaacccgcggtgctcctcgtttagccaggtcttgcatacggccgccagagcttccacttggtcaggcagtagcttgaagtttgcctttagatcgttatccacgtggtacttgtccatcaacgcgcgcgcagcctccatgcccttctcccacgcagacacgatcggcaggctcagcgggtttatcaccgtgctttcactttccgcttcactggactcttccttttcctcttgcgtccgcataccccgcgccactgggtcgtcttcattcagccgccgcaccgtgcgcttacctcccttgccgtgcttgattagcaccggtgggttgctgaaacccaccatttgtagcgccacatcttctctttcttcctcgctgtccacgatcacctctggggatggcgggcgctcgggcttgggagaggggcgcttctttttctttttggacgcaatggccaaatccgccgtcgaggtcgatggccgcgggctgggtgtgcgcggcaccagcgcatcttgtgacgagtcttcttcgtcctcggactcgagacgccgcctcagccgcttttttgggggcgcgcggggaggcggcggcgacggcgacggggacgacacgtcctccatggttggtggacgtcgcgccgcaccgcgtccgcgctcgggggtggtttcgcgctgctcctcttcccgactggccatttccttctcctataggcagaaaaagatcatggagtcagtcgagaaggaggacagcctaaccgccccctttgagttcgccaccaccgcctccaccgatgccgccaacgcgcctaccaccttccccgtcgaggcacccccgcttgaggaggaggaagtgattatcgagcaggacccaggttttgtaagcgaagacgacgaggatcgctcagtaccaacagaggataaaaagcaagaccaggacgacgcagaggcaaacgaggaacaagtcgggcggggggaccaaaggcatggcgactacctagatgtgggagacgacgtgctgttgaagcatctgcagcgccagtgcgccattatctgcgacgcgttgcaagagcgcagcgatgtgcccctcgccatagcggatgtcagccttgcctacgaacgccacctgttctcaccgcgcgtaccccccaaacgccaagaaaacggcacatgcgagcccaacccgcgcctcaacttctaccccgtatttgccgtgccagaggtgcttgccacctatcacatctttttccaaaactgcaagatacccctatcctgccgtgccaaccgcagccgagcggacaagcagctggccttgcggcagggcgctgtcatacctgatatcgcctcgctcgacgaagtgccaaaaatctttgagggtcttggacgcgacgagaaacgcgcggcaaacgctctgcaacaagaaaacagcgaaaatgaaagtcactgtggagtgctggtggaacttgagggtgacaacgcgcgcctagccgtgctgaaacgcagcatcgaggtcacccactttgcctacccggcacttaacctaccccccaaggttatgagcacagtcatgagcgagctgatcgtgcgccgtgcacgacccctggagagggatgcaaacttgcaagaacaaaccgaggagggcctacccgcagttggcgatgagcagctggcgcgctggcttgagacgcgcgagcctgccgacttggaggagcgacgcaagctaatgatggccgcagtgcttgttaccgtggagcttgagtgcatgcagcggttctttgctgacccggagatgcagcgcaagctagaggaaacgttgcactacacctttcgccagggctacgtgcgccaggcctgcaaaatttccaacgtggagctctgcaacctggtctcctaccttggaattttgcacgaaaaccgcctcgggcaaaacgtgcttcattccacgctcaagggcgaggcgcgccgcgactacgtccgcgactgcgtttacttatttctgtgctacacctggcaaacggccatgggcgtgtggcagcaatgcctggaggagcgcaacctaaaggagctgcagaagctgctaaagcaaaacttgaaggacctatggacggccttcaacgagcgctccgtggccgcgcacctggcggacattatcttccccgaacgcctgcttaaaaccctgcaacagggtctgccagacttcaccagtcaaagcatgttgcaaaactttaggaactttatcctagagcgttcaggaattctgcccgccacctgctgtgcgcttcctagcgactttgtgcccattaagtaccgtgaatgccctccgccgctttggggtcactgctaccttctgcagctagccaactaccttgcctaccactccgacatcatggaagacgtgagcggtgacggcctactggagtgtcactgtcgctgcaacctatgcaccccgcaccgctccctggtctgcaattcgcaactgcttagcgaaagtcaaattatcggtacctttgagctgcagggtccctcgcctgacgaaaagtccgcggctccggggttgaaactcactccggggctgtggacgtcggcttaccttcgcaaatttgtacctgaggactaccacgcccacgagattaggttctacgaagaccaatcccgcccgccaaatgcggagcttaccgcctgcgtcattacccagggccacatccttggccaattgcaagccatcaacaaagcccgccaagagtttctgctacgaaagggacggggggtttacctggacccccagtccggcgaggagctcaacccaatccccccgccgccgcagccctatcagcagccgcgggcccttgcttcccaggatggcacccaaaaagaagctgcagctgccgccgccgccacccacggacgaggaggaatactgggacagtcaggcagaggaggttttggacgaggaggaggagatgatggaagactgggacagcctagacgaagcttccgaggccgaagaggtgtcagacgaaacaccgtcaccctcggtcgcattcccctcgccggcgccccagaaattggcaaccgttcccagcatcgctacaacctccgctcctcaggcgccgccggcactgcctgttcgccgacccaaccgtagatgggacaccactggaaccagggccggtaagtctaagcagccgccgccgttagcccaagagcaacaacagcgccaaggctaccgctcgtggcgcgggcacaagaacgccatagttgcttgcttgcaagactgtgggggcaacatctccttcgcccgccgctttcttctctaccatcacggcgtggccttcccccgtaacatcctgcattactaccgtcatctctacagcccctactgcaccggcggcagcggcagcggcagcaacagcagcggtcacacagaagcaaaggcgaccggatagcaagactctgacaaagcccaagaaatccacagcggcggcagcagcaggaggaggagcgctgcgtctggcgcccaacgaacccgtatcgacccgcgagcttagaaataggatttttcccactctgtatgctatatttcaacaaagcaggggccaagaacaagagctgaaaataaaaaacaggtctctgcgctccctcacccgcagctgcctgtatcacaaaagcgaagatcagcttcggcgcacgctggaagacgcggaggctctcttcagcaaatactgcgcgctgactcttaaggactagtttcgcgccctttctcaaatttaagcgcgaaaactacgtcatctccagcggccacacccggcgccagcacctgtcgtcagcgccattatgagcaaggaaattcccacgccctacatgtggagttaccagccacaaatgggacttgcggctggagctgcccaagactactcaacccgaataaactacatgagcgcgggaccccacatgatatcccgggtcaacggaatccgcgcccaccgaaaccgaattctcctcgaacaggcggctattaccaccacacctcgtaataaccttaatccccgtagttggcccgctgccctggtgtaccaggaaagtcccgctcccaccactgtggtacttcccagagacgcccaggccgaagttcagatgactaactcaggggcgcagcttgcgggcggctttcgtcacagggtgcggtcgcccgggcgttttagggcggagtaacttgcatgtattgggaattgtagtttttttaaaatgggaagtgacgtatcgtgggaaaacggaagtgaagatttgaggaagttgtgggttttttggctttcgtttctgggcgtaggttcgcgtgcggttttctgggtgttttttgtggactttaaccgttacgtcattttttagtcctatatatactcgctctgtacttggccctttttacactgtgactgattgagctggtgccgtgtcgagtggtgttttttaataggtttttttactggtaaggctgactgttatggctgccgctgtggaagcgctgtatgttgttctggagcgggagggtgctattttgcctaggcaggagggtttttcaggtgtttatgtgtttttctctcctattaattttgttatacctcctatgggggctgtaatgttgtctctacgcctgcgggtatgtattcccccgggctatttcggtcgctttttagcactgaccgatgttaaccaacctgatgtgtttaccgagtcttacattatgactccggacatgaccgaggaactgtcggtggtgctttttaatcacggtgaccagtttttttacggtcacgccggcatggccgtagtccgtcttatgcttataagggttgtttttcctgttgtaagacaggcttctaatgtttaaatgtttttttttttgttattttattttgtgtttaatgcaggaacccgcagacatgtttgagagaaaaatggtgtctttttctgtggtggttccggaacttacctgcctttatctgcatgagcatgactacgatgtgcttgcttttttgcgcgaggctttgcctgattttttgagcagcaccttgcattttatatcgccgcccatgcaacaagcttacataggggctacgctggttagcatagctccgagtatgcgtgtcataatcagtgtgggttcttttgtcatggttcctggcggggaagtggccgcgctggtccgtgcagacctgcacgattatgttcagctggccctgcgaagggacctacgggatcgcggtatttttgttaatgttccgcttttgaatcttatacaggtctgtgaggaacctgaatttttgcaatcatgattcgctgcttgaggctgaaggtggagggcgctctggagcagatttttacaatggccggacttaatattcgggatttgcttagagacatattgataaggtggcgagatgaaaattatttgggcatggttgaaggtgctggaatgtttatagaggagattcaccctgaagggtttagcctttacgtccacttggacgtgagggcagtttgccttttggaagccattgtgcaacatcttacaaatgccattatctgttctttggctgtagagtttgaccacgccaccggaggggagcgcgttcacttaatagatcttcattttgaggttttggataatcttttggaataaaaaaaaaaaaacatggttcttccagctcttcccgctcctcccgtgtgtgactcgcagaacgaatgtgtaggttggctgggtgtggcttattctgcggtggtggatgttatcagggcagcggcgcatgaaggagtttacatagaacccgaagccagggggcgcctggatgctttgagagagtggatatactacaactactacacagagcgagctaagcgacgagaccggagacgcagatctgtttgtcacgcccgcacctggttttgcttcaggaaatatgactacgtccggcgttccatttggcatgacactacgaccaacacgatctcggttgtctcggcgcactccgtacagtagggatcgcctacctccttttgagacagagacccgcgctaccatactggaggatcatccgctgctgcccgaatgtaacactttgacaatgcacaacgtgagttacgtgcgaggtcttccctgcagtgtgggatttacgctgattcaggaatgggttgttccctgggatatggttctgacgcgggaggagcttgtaatcctgaggaagtgtatgcacgtgtgcctgtgttgtgccaacattgatatcatgacgagcatgatgatccatggttacgagtcctgggctctccactgtcattgttccagtcccggttccctgcagtgcatagccggcgggcaggttttggccagctggtttaggatggtggtggatggcgccatgtttaatcagaggtttatatggtaccgggaggtggtgaattacaacatgccaaaagaggtaatgtttatgtccagcgtgtttatgaggggtcgccacttaatctacctgcgcttgtggtatgatggccacgtgggttctgtggtccccgccatgagctttggatacagcgccttgcactgtgggattttgaacaatattgtggtgctgtgctgcagttactgtgctgatttaagtgagatcagggtgcgctgctgtgcccggaggacaaggcgtctcatgctgcgggcggtgcgaatcatcgctgaggagaccactgccatgttgtattcctgcaggacggagcggcggcggcagcagtttattcgcgcgctgctgcagcaccaccgccctatcctgatgcacgattatgactctacccccatgtaggcgtggacttccccttcgccgcccgttgagcaaccgcaagttggacagcagcctgtggctcagcagctggacagcgacatgaacttaagcgagctgcccggggagtttattaatatcactgatgagcgtttggctcgacaggaaaccgtgtggaatataacacctaagaatatgtctgttacccatgatatgatgctttttaaggccagccggggagaaaggactgtgtactctgtgtgttgggagggaggtggcaggttgaatactagggttctgtgagtttgattaaggtacggtgatcaatataagctatgtggtggtggggctatactactgaatgaaaaatgacttgaaattttctgcaattgaaaaataaacacgttgaaacataacatgcaacaggttcacgattctttattcctgggcaatgtaggagaaggtgtaagagttggtagcaaaagtttcagtggtgtattttccactttcccaggaccatgtaaaagacatagagtaagtgcttacctcgctagtttctgtggattcactagaatcgatgtaggatgttgcccctcctgacgcggtaggagaaggggagggtgccctgcatgtctgccgctgctcttgctcttgccgctgctgaggaggggggcgcatctgccgcagcaccggatgcatctgggaaaagcaaaaaaggggctcgtccctgtttccggaggaatttgcaagcggggtcttgcatgacggggaggcaaacccccgttcgccgcagtccggccggcccgagactcgaaccgggggtcctgcgactcaacccttggaaaataaccctccggctacagggagcgagccacttaatgctttcgctttccagcctaaccgcttacgccgcgcgcggccagtggccaaaaaagctagcgcagcagccgccgcgcctggaaggaagccgcggccgcgcttacaggctctccttttgcacggtctagagcgtcaacgactgcgcacgcctcaccggccagagcgtcccgaccatggagcactttttgccgctgcgcaacatctggaaccgcgtccgcgactttccgcgcgcctccaccaccgccgccggcatcacctggatgtccaggtacatctacggattacgtcgacgtttaaaccatatgatcagctcactcaaaggcggtaatacggttatccacagaatcaggggataacgcaggaaagaacatgtgagcaaaaggccagcaaaaggccaggaaccgtaaaaaggccgcgttgctggcgtttttccataggctccgcccccctgacgagcatcacaaaaatcgacgctcaagtcagaggtggcgaaacccgacaggactataaagataccaggcgtttccccctggaagctccctcgtgcgctctcctgttccgaccctgccgcttaccggatacctgtccgcctttctcccttcgggaagcgtggcgctttctcatagctcacgctgtaggtatctcagttcggtgtaggtcgttcgctccaagctgggctgtgtgcacgaaccccccgttcagcccgaccgctgcgccttatccggtaactatcgtcttgagtccaacccggtaagacacgacttatcgccactggcagcagccactggtaacaggattagcagagcgaggtatgtaggcggtgctacagagttcttgaagtggtggcctaactacggctacactagaagaacagtatttggtatctgcgctctgctgaagccagttaccttcggaaaaagagttggtagctcttgatccggcaaacaaaccaccgctggtagcggtggtttttttgtttgcaagcagcagattacgcgcagaaaaaaaggatctcaagaagatcctttgatcttttctacggggtctgacgctcagtggaacgaaaactcacgttaagggattttggtcatgagattatcaaaaaggatcttcacctagatccttttaaattaaaaatgaagttttaaatcaatctaaagtatatatgagtaaacttggtctgacagttaccaatgcttaatcagtgaggcacctatctcagcgatctgtctatttcgttcatccatagttgcctgactccccgtcgtgtagataactacgatacgggagggcttaccatctggccccagtgctgcaatgataccgcgagacccacgctcaccggctccagatttatcagcaataaaccagccagccggaagggccgagcgcagaagtggtcctgcaactttatccgcctccatccagtctattaattgttgccgggaagctagagtaagtagttcgccagttaatagtttgcgcaacgttgttgccattgctacaggcatcgtggtgtcacgctcgtcgtttggtatggcttcattcagctccggttcccaacgatcaaggcgagttacatgatcccccatgttgtgcaaaaaagcggttagctccttcggtcctccgatcgttgtcagaagtaagttggccgcagtgttatcactcatggttatggcagcactgcataattctcttactgtcatgccatccgtaagatgcttttctgtgactggtgagtactcaaccaagtcattctgagaatagtgtatgcggcgaccgagttgctcttgcccggcgtcaatacgggataataccgcgccacatagcagaactttaaaagtgctcatcattggaaaacgttcttcggggcgaaaactctcaaggatcttaccgctgttgagatccagttcgatgtaacccactcgtgcacccaactgatcttcagcatcttttactttcaccagcgtttctgggtgagcaaaaacaggaaggcaaaatgccgcaaaaaagggaataagggcgacacggaaatgttgaatactcatactcttcctttttcaatattattgaagcatttatcagggttattgtctcatgagcggatacatatttgaatgtatttagaaaaataaacaaataggggttccgcgcacatttccccgaaaagtgccacctaaattgtaagcgttaatattttgttaaaattcgcgttaaatttttgttaaatcagctcattttttaaccaataggccgaaatcggcaaaatcccttataaatcaaaagaatagaccgagatagggttgagtgttgttccagtttggaacaagagtccactattaaagaacgtggactccaacgtcaaagggcgaaaaaccgtctatcagggcgatggcccactacgtgaaccatcaccctaatcaagttttttggggtcgaggtgccgtaaagcactaaatcggaaccctaaagggagcccccgatttagagcttgacggggaaagccggcgaacgtggcgagaaaggaagggaagaaagcgaaaggagcgggcgctagggcgctggcaagtgtagcggtcacgctgcgcgtaaccaccacacccgccgcgcttaatgcgccgctacagggcgcgatggatcc

SEQ ID NO: 16 - DNA, 7622 bp, Artificial Sequence
  plasmid
agcgcccaatacgcaaaccgcctctccccgcgcgttggccgattcattaatgcagctggcacgacaggtttcccgactggaaagcgggcagtgagcgcaacgcaattaatgtgagttagctcactcattaggcaccccaggctttacactttatgcttccggctcgtatgttgtgtggaattgtgagcggataacaatttcacacaggaaacagctatgaccatgattacgaattgcctgcaggcagctgcgcgctcgctcgctcactgaggccgcccgggcaaagcccgggcgtcgggcgacctttggtcgcccggcctcagtgagcgagcgagcgcgcagagagggagtggccaactccatcactaggggttcctatcgatatcaagctttaatagtaatcaattacggggtcattagttcatagcccatatatggagttccgcgttacataacttacggtaaatggcccgcctggctgaccgcccaacgacccccgcccattgacgtcaataatgacgtatgttcccatagtaacgccaatagggactttccattgacgtcaatgggtggagtatttacggtaaactgcccacttggcagtacatcaagtgtatcatatgccaagtacgccccctattgacgtcaatgacggtaaatggcccgcctggcattatgcccagtacatgaccttatgggactttcctacttggcagtacatctacgtattagtcatcgctattaccatggtgatgcggttttggcagtacatcaatgggcgtggatagcggtttgactcacggggatttccaagtctccaccccattgacgtcaatgggagtttgttttggcaccaaaatcaacgggactttccaaaatgtcgtaacaactccgccccattgacgcaaatgggcggtaggcgtgtacggtgggaggtctatataagcagagctggtttagtggatatccttaagggcccagccggcctcgcgagaattctctagaacgccgccatgaccatgattacggattcactggccgtcgttttacaacgtcgtgactgggaaaaccctggcgttacccaacttaatcgccttgcagcacatccccctttcgccagctggcgtaatagcgaagaggcccgcaccgatcgcccttcccaacagttgcgcagcctgaatggcgaatggcgctttgcctggtttccggcaccagaagcggtgccggaaagctggctggagtgcgatcttcctgaggccgatactgtcgtcgtcccctcaaactggcagatgcacggttacgatgcgcccatctacaccaacgtgacctatcccattacggtcaatccgccgtttgttcccacggagaatccgacgggttgttactcgctcacatttaatgttgatgaaagctggctacaggaaggccagacgcgaattatttttgatggcgttaactcggcgtttcatctgtggtgcaacgggcgctgggtcggttacggccaggacagtcgtttgccgtctgaatttgacctgagcgcatttttacgcgccggagaaaaccgcctcgcggtgatggtgctgcgctggagtgacggcagttatctggaagatcaggatatgtggcggatgagcggcattttccgtgacgtctcgttgctgcataaaccgactacacaaatcagcgatttccatgttgccactcgctttaatgatgatttcagccgcgctgtactggaggctgaagttcagatgtgcggcgagttgcgtgactacctacgggtaacagtttctttatggcagggtgaaacgcaggtcgccagcggcaccgcgcctttcggcggtgaaattatcgatgagcgtggtggttatgccgatcgcgtcacactacgtctgaacgtcgaaaacccgaaactgtggagcgccgaaatcccgaatctctatcgtgcggtggttgaactgcacaccgccgacggcacgctgattgaagcagaagcctgcgatgtcggtttccgcgaggtgcggattgaaaatggtctgctgctgctgaacggcaagccgttgctgattcgaggcgttaaccgtcacgagcatcatcctctgcatggtcaggtcatggatgagcagacgatggtgcaggatatcctgctgatgaagcagaacaactttaacgccgtgcgctgttcgcattatccgaaccatccgctgtggtacacgctgtgcgaccgctacggcctgtatgtggtggatgaagccaatattgaaacccacggcatggtgccaatgaatcgtctgaccgatgatccgcgctggctaccggcgatgagcgaacgcgtaacgcgaatggtgcagcgcgatcgtaatcacccgagtgtgatcatctggtcgctggggaatgaatcaggccacggcgctaatcacgacgcgctgtatcgctggatcaaatctgtcgatccttcccgcccggtgcagtatgaaggcggcggagccgacaccacggccaccgatattatttgcccgatgtacgcgcgcgtggatgaagaccagcccttcccggctgtgccgaaatggtccatcaaaaaatggctttcgctacctggagagacgcgcccgctgatcctttgcgaatacgcccacgcgatgggtaacagtcttggcggtttcgctaaatactggcaggcgtttcgtcagtatccccgtttacagggcggcttcgtctgggactgggtggatcagtcgctgattaaatatgatgaaaacggcaacccgtggtcggcttacggcggtgattttggcgatacgccgaacgatcgccagttctgtatgaacggtctggtctttgccgaccgcacgccgcatccagcgctgacggaagcaaaacaccagcagcagtttttccagttccgtttatccgggcaaaccatcgaagtgaccagcgaatacctgttccgtcatagcgataacgagctcctgcactggatggtggcgctggatggtaagccgctggcaagcggtgaagtgcctctggatgtcgctccacaaggtaaacagttgattgaactgcctgaactaccgcagccggagagcgccgggcaactctggctcacagtacgcgtagtgcaaccgaacgcgaccgcatggtcagaagccgggcacatcagcgcctggcagcagtggcgtctggcggaaaacctcagtgtgacgctccccgccgcgtcccacgccatcccgcatctgaccaccagcgaaatggatttttgcatcgagctgggtaataagcgttggcaatttaaccgccagtcaggctttctttcacagatgtggattggcgataaaaaacaactgctgacgccgctgcgcgatcagttcacccgtgcaccgctggataacgacattggcgtaagtgaagcgacccgcattgaccctaacgcctgggtcgaacgctggaaggcggcgggccattaccaggccgaagcagcgttgttgcagtgcacggcagatacacttgctgatgcggtgctgattacgaccgctcacgcgtggcagcatcaggggaaaaccttatttatcagccggaaaacctaccggattgatggtagtggtcaaatggcgattaccgttgatgttgaagtggcgagcgatacaccgcatccggcgcggattggcctgaactgccagctggcgcaggtagcagagcgggtaaactggctcggattagggccgcaagaaaactatcccgaccgccttactgccgcctgttttgaccgctgggatctgccattgtcagacatgtataccccgtacgtcttcccgagcgaaaacggtctgcgctgcgggacgcgcgaattgaattatggcccacaccagtggcgcggcgacttccagttcaacatcagccgctacagtcaacagcaactgatggaaaccagccatcgccatctgctgcacgcggaagaaggcacatggctgaatatcgacggtttccatatggggattggtggcgacgactcctggagcccgtcagtatcggcggaattccagctgagcgccggtcgctaccattaccagttggtctggtgtcaaaaataaagctgacactagtgcggatccacgggtggcatccctgtgacccctccccagtgcctctcctggccctggaagttgccactccagtgcccaccagccttgtcctaataaaattaagttgcatcattttgtctgactaggtgtccttctataatattatggggtggaggggggtggtatggagcaaggggcaagttgggaagacaacctgtagggcctgcggggtctattgggaaccaagctggagtgcagtggcacaatcttggctcactgcaatctccgcctcctgggttcaagcgattctcctgcctcagcctcccgagttgttgggattccaggcatgcatgaccaggctcagctaatttttgtttttttggtagagacggggtttcaccatattggccaggctggtctccaactcctaatctcaggtgatctacccaccttggcctcccaaattgctgggattacaggcgtgaaccactgctcccttccctgtccttatcgatagatctaggaacccctagtgatggagttggccactccctctctgcgcgctcgctcgctcactgaggccgggcgaccaaaggtcgcccgacgcccgggctttgcccgggcggcctcagtgagcgagcgagcgcgcagctgcctgcaggcagcttggcactggccgtcgttttacaacgtcgtgactgggaaaaccctggcgttacccaacttaatcgccttgcagcacatccccctttcgccagctggcgtaatagcgaagaggcccgcaccgatcgcccttcccaacagttgcgcagcctgaatggcgaatggcgcctgatgcggtattttctccttacgcatctgtgcggtatttcacaccgcatacgtcaaagcaaccatagtacgcgccctgtagcggcgcattaagcgcggcgggtgtggtggttacgcgcagcgtgaccgctacacttgccagcgccctagcgcccgctcctttcgctttcttcccttcctttctcgccacgttcgccggctttccccgtcaagctctaaatcgggggctccctttagggttccgatttagtgctttacggcacctcgaccccaaaaaacttgatttgggtgatggttcacgtagtgggccatcgccctgatagacggtttttcgccctttgacgttggagtccacgttctttaatagtggactcttgttccaaactggaacaacactcaaccctatctcgggctattcttttgatttataagggattttgccgatttcggcctattggttaaaaaatgagctgatttaacaaaaatttaacgcgaattttaacaaaatattaacgtttacaattttatggtgcactctcagtacaatctgctctgatgccgcatagttaagccagccccgacacccgccaacacccgctgacgcgccctgacgggcttgtctgctcccggcatccgcttacagacaagctgtgaccgtctccgggagctgcatgtgtcagaggttttcaccgtcatcaccgaaacgcgcgagacgaaagggcctcgtgatacgcctatttttataggttaatgtcatgataataatggtttcttagacgtcaggtggcacttttcggggaaatgtgcgcggaacccctatttgtttatttttctaaatacattcaaatatgtatccgctcatgagacaataaccctgataaatgcttcaataatattgaaaaaggaagagtatgagtattcaacatttccgtgtcgcccttattcccttttttgcggcattttgccttcctgtttttgctcacccagaaacgctggtgaaagtaaaagatgctgaagatcagttgggtgcacgagtgggttacatcgaactggatctcaacagcggtaagatccttgagagttttcgccccgaagaacgttttccaatgatgagcacttttaaagttctgctatgtggcgcggtattatcccgtattgacgccgggcaagagcaactcggtcgccgcatacactattctcagaatgacttggttgagtactcaccagtcacagaaaagcatcttacggatggcatgacagtaagagaattatgcagtgctgccataaccatgagtgataacactgcggccaacttacttctgacaacgatcggaggaccgaaggagctaaccgcttttttgcacaacatgggggatcatgtaactcgccttgatcgttgggaaccggagctgaatgaagccataccaaacgacgagcgtgacaccacgatgcctgtagcaatggcaacaacgttgcgcaaactattaactggcgaactacttactctagcttcccggcaacaattaatagactggatggaggcggataaagttgcaggaccacttctgcgctcggcccttccggctggctggtttattgctgataaatctggagccggtgagcgtgggtctcgcggtatcattgcagcactggggccagatggtaagccctcccgtatcgtagttatctacacgacggggagtcaggcaactatggatgaacgaaatagacagatcgctgagataggtgcctcactgattaagcattggtaactgtcagaccaagtttactcatatatactttagattgatttaaaacttcatttttaatttaaaaggatctaggtgaagatcctttttgataatctcatgaccaaaatcccttaacgtgagttttcgttccactgagcgtcagaccccgtagaaaagatcaaaggatcttcttgagatcctttttttctgcgcgtaatctgctgcttgcaaacaaaaaaaccaccgctaccagcggtggtttgtttgccggatcaagagctaccaactctttttccgaaggtaactggcttcagcagagcgcagataccaaatactgttcttctagtgtagccgtagttaggccaccacttcaagaactctgtagcaccgcctacatacctcgctctgctaatcctgttaccagtggctgctgccagtggcgataagtcgtgtcttaccgggttggactcaagacgatagttaccggataaggcgcagcggtcgggctgaacggggggttcgtgcacacagcccagcttggagcgaacgacctacaccgaactgagatacctacagcgtgagctatgagaaagcgccacgcttcccgaagggagaaaggcggacaggtatccggtaagcggcagggtcggaacaggagagcgcacgagggagcttccagggggaaacgcctggtatctttatagtcctgtcgggtttcgccacctctgacttgagcgtcgatttttgtgatgctcgtcaggggggcggagcctatggaaaaacgccagcaacgcggcctttttacggttcctggccttttgctggccttttgctcacatgttctttcctgcgttatcccctgattctgtggataaccgtattaccgcctttgagtgagctgataccgctcgccgcagccgaacgaccgagcgcagcgagtcagtgagcgaggaagcggaag

SEQ ID NO: 17 - DNA, 21 bp, Artificial Sequence
  primer
ggaacccctagtgatggagtt

SEQ ID NO: 18 - DNA, 16 bp, Artificial Sequence
  primer
cggcctcagtgagcga

SEQ ID NO: 19 - DNA, 21 bp, Artificial Sequence
  probe
cactccctctctgcgcgctcg

SEQ ID NO: 20 - DNA, 2367 bp, Artificial Sequence
  plasmid
gcggccgctacgtcgacgtttaaaccatatgatcagctcactcaaaggcggtaatacggttatccacagaatcaggggataacgcaggaaagaacatgtgagcaaaaggccagcaaaaggccaggaaccgtaaaaaggccgcgttgctggcgtttttccataggctccgcccccctgacgagcatcacaaaaatcgacgctcaagtcagaggtggcgaaacccgacaggactataaagataccaggcgtttccccctggaagctccctcgtgcgctctcctgttccgaccctgccgcttaccggatacctgtccgcctttctcccttcgggaagcgtggcgctttctcatagctcacgctgtaggtatctcagttcggtgtaggtcgttcgctccaagctgggctgtgtgcacgaaccccccgttcagcccgaccgctgcgccttatccggtaactatcgtcttgagtccaacccggtaagacacgacttatcgccactggcagcagccactggtaacaggattagcagagcgaggtatgtaggcggtgctacagagttcttgaagtggtggcctaactacggctacactagaagaacagtatttggtatctgcgctctgctgaagccagttaccttcggaaaaagagttggtagctcttgatccggcaaacaaaccaccgctggtagcggtggtttttttgtttgcaagcagcagattacgcgcagaaaaaaaggatctcaagaagatcctttgatcttttctacggggtctgacgctcagtggaacgaaaactcacgttaagggattttggtcatgagattatcaaaaaggatcttcacctagatccttttaaattaaaaatgaagttttaaatcaatctaaagtatatatgagtaaacttggtctgacagttaccaatgcttaatcagtgaggcacctatctcagcgatctgtctatttcgttcatccatagttgcctgactccccgtcgtgtagataactacgatacgggagggcttaccatctggccccagtgctgcaatgataccgcgagacccacgctcaccggctccagatttatcagcaataaaccagccagccggaagggccgagcgcagaagtggtcctgcaactttatccgcctccatccagtctattaattgttgccgggaagctagagtaagtagttcgccagttaatagtttgcgcaacgttgttgccattgctacaggcatcgtggtgtcacgctcgtcgtttggtatggcttcattcagctccggttcccaacgatcaaggcgagttacatgatcccccatgttgtgcaaaaaagcggttagctccttcggtcctccgatcgttgtcagaagtaagttggccgcagtgttatcactcatggttatggcagcactgcataattctcttactgtcatgccatccgtaagatgcttttctgtgactggtgagtactcaaccaagtcattctgagaatagtgtatgcggcgaccgagttgctcttgcccggcgtcaatacgggataataccgcgccacatagcagaactttaaaagtgctcatcattggaaaacgttcttcggggcgaaaactctcaaggatcttaccgctgttgagatccagttcgatgtaacccactcgtgcacccaactgatcttcagcatcttttactttcaccagcgtttctgggtgagcaaaaacaggaaggcaaaatgccgcaaaaaagggaataagggcgacacggaaatgttgaatactcatactcttcctttttcaatattattgaagcatttatcagggttattgtctcatgagcggatacatatttgaatgtatttagaaaaataaacaaataggggttccgcgcacatttccccgaaaagtgccacctaaattgtaagcgttaatattttgttaaaattcgcgttaaatttttgttaaatcagctcattttttaaccaataggccgaaatcggcaaaatcccttataaatcaaaagaatagaccgagatagggttgagtgttgttccagtttggaacaagagtccactattaaagaacgtggactccaacgtcaaagggcgaaaaaccgtctatcagggcgatggcccactacgtgaaccatcaccctaatcaagttttttggggtcgaggtgccgtaaagcactaaatcggaaccctaaagggagcccccgatttagagcttgacggggaaagccggcgaacgtggcgagaaaggaagggaagaaagcgaaaggagcgggcgctagggcgctggcaagtgtagcggtcacgctgcgcgtaaccaccacacccgccgcgcttaatgcgccgctacagggcgcgatggatcc

SEQ ID NO: 21 - DNA, 2968 bp, Artificial Sequence
  plasmid
tcgcgcgtttcggtgatgacggtgaaaacctctgacacatgcagctcccggagactgtcacagcttgtctgtaagcggatgccgggagcagacaagcccgtcagggcgcgtcagcgggtgttggcgggtgtcggggctggcttaactatgcggcatcagagcagattgtactgagagtgcaccatatgcggtgtgaaataccgcacagatgcgtaaggagaaaataccgcatcaggcgccattcgccattcaggctgcgcaactgttgggaagggcgatcggtgcgggcctcttcgctattacgccagctggcgaaagggggatgtgctgcaaggcgattaagttgggtaacgccagggttttcccagtcacgacgttgtaaaacgacggccagtgaattgacgcgtattgggatatcccaatggcgcgccgagcttggcgtaatcatggtcatagctgtttcctgtgtgaaattgttatccgctcacaattccacacaacatacgagccggaagcataaagtgtaaagcctggggtgcctaatgagtgagctaactcacattaattgcgttgcgctcactgcccgctttccagtcgggaaacctgtcgtgccagctgcattaatgaatcggccaacgcgcggggagaggcggtttgcgtattgggcgctgttccgcttcctcgctcactgactcgctgcgctcggtcgttcggctgcggcgagcggtatcagctcactcaaaggcggtaatacggttatccacagaatcaggggataacgcaggaaagaacatgtgagcaaaaggccagcaaaaggccaggaaccgtaaaaaggccgcgttgctggcgtttttccataggctccgcccccctgacgagcatcacaaaaatcgacgctcaagtcagaggtggcgaaacccgacaggactataaagataccaggcgtttccccctggaagctccctcgtgcgctctcctgttccgaccctgccgcttaccggatacctgtccgcctttctcccttcgggaagcgtggcgctttctcatagctcacgctgtaggtatctcagttcggtgtaggtcgttcgctccaagctgggctgtgtgcacgaaccccccgttcagcccgaccgctgcgccttatccggtaactatcgtcttgagtccaacccggtaagacacgacttatcgccactggcagcagccactggtaacaggattagcagagcgaggtatgtaggcggtgctacagagttcttgaagtggtggcctaactacggctacactagaagaacagtatttggtatctgcgctctgctgaagccagttaccttcggaaaaagagttggtagctcttgatccggcaaacaaaccaccgctggtagcggtggtttttttgtttgcaagcagcagatgcggccgcaatatttgcatgtcgctatgtgttctgggaaatcaccataaacgtgaaatccctatcagtgatagagacttataagttccctatcagtgatagagaaccggtgggcactcttccgtggtctggtggataaattcgcaagggtatcatggcggacgaccggggttcgaaccccggatccggccgtccgccgtgatccatgcggttaccgcccgcgtgtcgaacccaggtgtgcgacgtcagacaacgggggagcgctcctttttgaattccactttggccgcggctcgagtacgcgcagaaaaaaaggatctcaagaagatcctttgatcttttctacggggtctgacgctcagtggaacgaaaactcacgttaagggattttggtcatgagattatcaaaaaggatcttcacctagatccttttaaattaaaaatgaagttttaaatcaatctaaagtatatatgagtaaacttggtctgacagttaccaatgcttaatcagtgaggcacctatctcagcgatctgtctatttcgttcatccatagttgcctgactccccgtcgtgtagataactacgatacgggagggcttaccatctggccccagtgctgcaatgataccgcgagaaccacgctcaccggctccagatttatcagcaataaaccagccagccggaagggccgagcgcagaagtggtcctgcaactttatccgcctccatccagtctattaattgttgccgggaagctagagtaagtagttcgccagttaatagtttgcgcaacgttgttgccattgctacaggcatcgtggtgtcacgctcgtcgtttggtatggcttcattcagctccggttcccaacgatcaaggcgagttacatgatcccccatgttgtgcaaaaaagcggttagctccttcggtcctccgatcgttgtcagaagtaagttggccgcagtgttatcactcatggttatggcagcactgcataattctcttactgtcatgccatccgtaagatgcttttctgtgactggtgagtactcaaccaagtcattctgagaatagtgtatgcggcgaccgagttgctcttgcccggcgtcaatacgggataataccgcgccacatagcagaactttaaaagtgctcatcattggaaaacgttcttcggggcgaaaactctcaaggatcttaccgctgttgagatccagttcgatgtaacccactcgtgcacccaactgatcttcagcatcttttactttcaccagcgtttctgggtgagcaaaaacaggaaggcaaaatgccgcaaaaaagggaataagggcgacacggaaatgttgaatactcatactcttcctttttcaatattattgaagcatttatcagggttattgtctcatgagcggatacatatttgaatgtatttagaaaaataaacaaataggggttccgcgcacatttccccgaaaagtgccacctgacgtctaagaaaccattattatcatgacattaacctataaaaataggcgtatcacgaggcccttttgtc

SEQ ID NO: 22 - DNA, 6159 bp, Artificial Sequence
  plasmid
tcgcgcgtttcggtgatgacggtgaaaacctctgacacatgcagctcccggagactgtcacagcttgtctgtaagcggatgccgggagcagacaagcccgtcagggcgcgtcagcgggtgttggcgggtgtcggggctggcttaactatgcggcatcagagcagattgtactgagagtgcaccatatgcggtgtgaaataccgcacagatgcgtaaggagaaaataccgcatcaggcgccattcgccattcaggctgcgcaactgttgggaagggcgatcggtgcgggcctcttcgctattacgccagctggcgaaagggggatgtgctgcaaggcgattaagttgggtaacgccagggttttcccagtcacgacgttgtaaaacgacggccagtgaattgacgcgtattgggatgaggagcttggcccattgcatacgttgtatccatatcataatatgtacatttatattggctcatgtccaacattaccgccatgttgacattgattattgactagttattaatagtaatcaattacggggtcattagttcatagcccatatatggagttccgcgttacataacttacggtaaatggcccgcctggctgaccgcccaacgacccccgcccattgacgtcaataatgacgtatgttcccatagtaacgccaatagggactttccattgacgtcaatgggtggagtatttacggtaaactgcccacttggcagtacatcaagtgtatcatatgccaagtacgccccctattgacgtcaatgacggtaaatggcccgcctggcattatgcccagtacatgaccttatgggactttcctacttggcagtacatctacgtattagtcatcgctattaccatggtgatgcggttttggcagtacatcaatgggcgtggatagcggtttgactcacggggatttccaagtctccaccccattgacgtcaatgggagtttgttttggcaccaaaatcaacgggactttccaaaatgtcgtaacaactccgccccattgacgcaaatgggcggtaggcgtgtacggtgggaggtctatataagcagagctcgtttagtgaaccgtcagatcgcctggagacgccatccacgctgttttgacctccatagaagacaccgggaccgatccagcctccgcggccccgaattcaccatgtctagattagataaaagtaaagtgattaacagcgcattagagctgcttaatgaggtcggaatcgaaggtttaacaacccgtaaactcgcccagaagctaggtgtagagcagcctacattgtattggcacgtgcgcaacaagcagactcttatgaacatgctttcagaggcaatactggcgaagcatcacacccgttcagcaccgttaccgactgagagttggcagcagtttctccaggaaaatgctctgagtttccgtaaagcattactggtccatcgtgatggagcccgattgcatatagggacctctcctacgcccccccagtttgaacaagcagaggcgcaactacgctgtctatgcgatgcagggttttcggtcgaggaggctcttttcattctgcaatctatcagccattttacgttgggtgcagtattagaggagcaagcaacaaaccagatagaaaataatcatgtgatagacgctgcaccaccattattacaagaggcatttaatattcaggcgagaacctctgctgaaatggccttccatttcgggctgaaatcattaatatttggattttctgcacagttagatgaaaaaaagcatacacccattgaggatggtaataaaccaaaaaagaagagaaagctagcagtgtcagtgacatttgaagatgtggctgtgctctttactcgggacgagtggaagaagctggatctgtctcagagaagcctgtaccgtgaggtgatgctggagaattacagcaacctggcctccatggcaggattcctgtttaccaaaccaaaggtgatctccctgttgcagcaaggagaggatccctggtaaatcgatctgagaacttcagggtgagtttggggacccttgattgttctttctttttcgctattgtaaaattcatgttatatggagggggcaaagttttcagggtgttgtttagaatgggaagatgtcccttgtatcaccatggaccctcatgataattttgtttctttcactttctactctgttgacaaccattgtctcctcttattttcttttcattttctgtaactttttcgttaaactttagcttgcatttgtaacgaatttttaaattcacttttgtttatttgtcagattgtaagtactttctctaatcacttttttttcaaggcaatcagggtatattatattgtacttcagcacagttttagagaacaattgttataattaaatgataaggtagaatatttctgcatataaattctggctggcgtggaaatattcttattggtagaaacaactacaccctggtcatcatcctgcctttctctttatggttacaatgatatacactgtttgagatgaggataaaatactctgagtccaaaccgggcccctctgctaaccatgttcatgccttcttctctttcctacagctcctgggcaacgtgctggttgttgtgctgtctcatcattttggcaaagaattcactcctcaggtgcaggctgcctatcagaaggtggtggctggtgtggccaatgccctggctcacaaataccactgagatctttttccctctgccaaaaattatggggacatcatgaagccccttgagcatctgacttctggctaataaaggaaatttattttcattgcaatagtgtgttggaattttttgtgtctctcactcggaaggacatatgggagggcaaatcatttaaaacatcagaatgagtatttggtttagagtttggcaacatatgcccatatgctggctgccatgaacaaaggttggctataaagaggtcatcagtatatgaaacagccccctgctgtccattccttattccatagaaaagccttgacttgaggttagattttttttatattttgttttgtgttatttttttctttaacatccctaaaattttccttacatgttttactagccagatttttcctcctctcctgactactcccagtcatagctgtccctcttctcttatgaactcgactgaagctcacatttccccgaaaagtgccacctgacgtaactataacggtcctaaggtagcgaaagctcagatctctttcgtcttcacttgagtttactccctatcagtgatagagaacgtatgtcgagtttactccctatcagtgatagagaacgatgtcgagtttactccctatcagtgatagagaacgtatgtcgagtttactccctatcagtgatagagaacgtatgtcgagtttactccctatcagtgatagagaacgtatgtcgagtttatccctatcagtgatagagaacgtatgtcgagtttactccctatcagtgatagagaacgtatgtcgaggtaggcgtgtacggtcatatgcttaccgtaacttgaaagtatttcgatttcttggctttatatatcttgtggaaaggacgactcgaggggcactcttccgtggtctggtggataaattcgcaagggtatcatggcggacgaccggggttcgaaccccggatccggccgtccgccgtgatccatgcggttaccgcccgcgtgtcgaacccaggtgtgcgacgtcagacaacgggggagcgctccttttaagcttatctatgtcgggtgcggagaaagaggtaatgaaatggcattatgggtattatgggtctgcattaatgagcttggcgagattttcaggagctaaggaagctatcccaatggcgcgccgagcttggcgtaatcatggtcatagctgtttcctgtgtgaaattgttatccgctcacaattccacacaacatacgagccggaagcataaagtgtaaagcctggggtgcctaatgagtgagctaactcacattaattgcgttgcgctcactgcccgctttccagtcgggaaacctgtcgtgccagctgcattaatgaatcggccaacgcgcggggagaggcggtttgcgtattgggcgctgttccgcttcctcgctcactgactcgctgcgctcggtcgttcggctgcggcgagcggtatcagctcactcaaaggcggtaatacggttatccacagaatcaggggataacgcaggaaagaacatgtgagcaaaaggccagcaaaaggccaggaaccgtaaaaaggccgcgttgctggcgtttttccataggctccgcccccctgacgagcatcacaaaaatcgacgctcaagtcagaggtggcgaaacccgacaggactataaagataccaggcgtttccccctggaagctccctcgtgcgctctcctgttccgaccctgccgcttaccggatacctgtccgcctttctcccttcgggaagcgtggcgctttctcatagctcacgctgtaggtatctcagttcggtgtaggtcgttcgctccaagctgggctgtgtgcacgaaccccccgttcagcccgaccgctgcgccttatccggtaactatcgtcttgagtccaacccggtaagacacgacttatcgccactggcagcagccactggtaacaggattagcagagcgaggtatgtaggcggtgctacagagttcttgaagtggtggcctaactacggctacactagaagaacagtatttggtatctgcgctctgctgaagccagttaccttcggaaaaagagttggtagctcttgatccggcaaacaaaccaccgctggtagcggtggtttttttgtttgcaagcagcagattacgcgcagaaaaaaaggatctcaagaagatcctttgatcttttctacggggtctgacgctcagtggaacgaaaactcacgttaagggattttggtcatgagattatcaaaaaggatcttcacctagatccttttaaattaaaaatgaagttttaaatcaatctaaagtatatatgagtaaacttggtctgacagttaccaatgcttaatcagtgaggcacctatctcagcgatctgtctatttcgttcatccatagttgcctgactccccgtcgtgtagataactacgatacgggagggcttaccatctggccccagtgctgcaatgataccgcgagaaccacgctcaccggctccagatttatcagcaataaaccagccagccggaagggccgagcgcagaagtggtcctgcaactttatccgcctccatccagtctattaattgttgccgggaagctagagtaagtagttcgccagttaatagtttgcgcaacgttgttgccattgctacaggcatcgtggtgtcacgctcgtcgtttggtatggcttcattcagctccggttcccaacgatcaaggcgagttacatgatcccccatgttgtgcaaaaaagcggttagctccttcggtcctccgatcgttgtcagaagtaagttggccgcagtgttatcactcatggttatggcagcactgcataattctcttactgtcatgccatccgtaagatgcttttctgtgactggtgagtactcaaccaagtcattctgagaatagtgtatgcggcgaccgagttgctcttgcccggcgtcaatacgggataataccgcgccacatagcagaactttaaaagtgctcatcattggaaaacgttcttcggggcgaaaactctcaaggatcttaccgctgttgagatccagttcgatgtaacccactcgtgcacccaactgatcttcagcatcttttactttcaccagcgtttctgggtgagcaaaaacaggaaggcaaaatgccgcaaaaaagggaataagggcgacacggaaatgttgaatactcatactcttcctttttcaatattattgaagcatttatcagggttattgtctcatgagcggatacatatttgaatgtatttagaaaaataaacaaataggggttccgcgcacatttccccgaaaagtgccacctgacgtctaagaaaccattattatcatgacattaacctataaaaataggcgtatcacgaggcccttttgtc

SEQ ID NO: 23 - DNA, 9808 bp, Artificial Sequence
  plasmid
tggaagggctaattcactcccaaagaagacaagatatccttgatctgtggatctaccacacacaaggctacttccctgattagcagaactacacaccagggccaggggtcagatatccactgacctttggatggtgctacaagctagtaccagttgagccagataaggtagaagaggccaataaaggagagaacaccagcttgttacaccctgtgagcctgcatgggatggatgacccggagagagaagtgttagagtggaggtttgacagccgcctagcatttcatcacgtggcccgagagctgcatccggagtacttcaagaactgctgatatcgagcttgctacaagggactttccgctggggactttccagggaggcgtggcctgggcgggactggggagtggcgagccctcagatcctgcatataagcagctgctttttgcctgtactgggtctctctggttagaccagatctgagcctgggagctctctggctaactagggaacccactgcttaagcctcaataaagcttgccttgagtgcttcaagtagtgtgtgcccgtctgttgtgtgactctggtaactagagatccctcagacccttttagtcagtgtggaaaatctctagcagtggcgcccgaacagggacttgaaagcgaaagggaaaccagaggagctctctcgacgcaggactcggcttgctgaagcgcgcacggcaagaggcgaggggcggcgactggtgagtacgccaaaaattttgactagcggaggctagaaggagagagatgggtgcgagagcgtcagtattaagcgggggagaattagatcgcgatgggaaaaaattcggttaaggccagggggaaagaaaaaatataaattaaaacatatagtatgggcaagcagggagctagaacgattcgcagttaatcctggcctgttagaaacatcagaaggctgtagacaaatactgggacagctacaaccatcccttcagacaggatcagaagaacttagatcattatataatacagtagcaaccctctattgtgtgcatcaaaggatagagataaaagacaccaaggaagctttagacaagatagaggaagagcaaaacaaaagtaagaccaccgcacagcaagcggccggccgctgatcttcagacctggaggaggagatatgagggacaattggagaagtgaattatataaatataaagtagtaaaaattgaaccattaggagtagcacccaccaaggcaaagagaagagtggtgcagagagaaaaaagagcagtgggaataggagctttgttccttgggttcttgggagcagcaggaagcactatgggcgcagcgtcaatgacgctgacggtacaggccagacaattattgtctggtatagtgcagcagcagaacaatttgctgagggctattgaggcgcaacagcatctgttgcaactcacagtctggggcatcaagcagctccaggcaagaatcctggctgtggaaagatacctaaaggatcaacagctcctggggatttggggttgctctggaaaactcatttgcaccactgctgtgccttggaatgctagttggagtaataaatctctggaacagatttggaatcacacgacctggatggagtgggacagagaaattaacaattacacaagcttaatacactccttaattgaagaatcgcaaaaccagcaagaaaagaatgaacaagaattattggaattagataaatgggcaagtttgtggaattggtttaacataacaaattggctgtggtatataaaattattcataatgatagtaggaggcttggtaggtttaagaatagtttttgctgtactttctatagtgaatagagttaggcagggatattcaccattatcgtttcagacccacctcccaaccccgaggggacccgacaggcccgaaggaatagaagaagaaggtggagagagagacagagacagatccattcgattagtgaacggatctcgacggtatcgcctttaaaagaaaaggggggattggggggtacagtgcaggggaaagaatagtagacataatagcaacagacatacaaactaaagaattacaaaaacaaattacaaaaattcaaaattttcgggtttattacagggacagcagagatccagtttatcgagatccagtttatcgtgacattgattattgactagttattaatagtaatcaattacggggtcattagttcatagcccatatatggagttccgcgttacataacttacggtaaatggcccgcctggctgaccgcccaacgacccccgcccattgacgtcaataatgacgtatgttcccatagtaacgccaatagggactttccattgacgtcaatgggtggagtatttacggtaaactgcccacttggcagtacatcaagtgtatcatatgccaagtacgccccctattgacgtcaatgacggtaaatggcccgcctggcattatgcccagtacatgaccttatgggactttcctacttggcagtacatctacgtattagtcatcgctattaccatggtgatgcggttttggcagtacatcaatgggcgtggatagcggtttgactcacggggatttccaagtctccaccccattgacgtcaatgggagtttgttttggcaccaaaatcaacgggactttccaaaatgtcgtaacaactccgccccattgacgcaaatgggcggtaggcgtgtacggtgggaggtctatataagcagagctcgtttagtgaaccgtcagatcgcctggagacgccatccacgctgttttgacctccatagaagacaccgggaccgatccagcctccgcggccccgaattcaccatgtctagattagataaaagtaaagtgattaacagcgcattagagctgcttaatgaggtcggaatcgaaggtttaacaacccgtaaactcgcccagaagctaggtgtagagcagcctacattgtattggcacgtgcgcaacaagcagactcttatgaacatgctttcagaggcaatactggcgaagcatcacacccgttcagcaccgttaccgactgagagttggcagcagtttctccaggaaaatgctctgagtttccgtaaagcattactggtccatcgtgatggagcccgattgcatatagggacctctcctacgcccccccagtttgaacaagcagaggcgcaactacgctgtctatgcgatgcagggttttcggtcgaggaggctcttttcattctgcaatctatcagccattttacgttgggtgcagtattagaggagcaagcaacaaaccagatagaaaataatcatgtgatagacgctgcaccaccattattacaagaggcatttaatattcaggcgagaacctctgctgaaatggccttccatttcgggctgaaatcattaatatttggattttctgcacagttagatgaaaaaaagcatacacccattgaggatggtaataaaccaaaaaagaagagaaagctagcagtgtcagtgacatttgaagatgtggctgtgctctttactcgggacgagtggaagaagctggatctgtctcagagaagcctgtaccgtgaggtgatgctggagaattacagcaacctggcctccatggcaggattcctgtttaccaaaccaaaggtgatctccctgttgcagcaaggagaggatccctggtaaatcgatctgagaacttcagggtgagtttggggacccttgattgttctttctttttcgctattgtaaaattcatgttatatggagggggcaaagttttcagggtgttgtttagaatgggaagatgtcccttgtatcaccatggaccctcatgataattttgtttctttcactttctactctgttgacaaccattgtctcctcttattttcttttcattttctgtaactttttcgttaaactttagcttgcatttgtaacgaatttttaaattcacttttgtttatttgtcagattgtaagtactttctctaatcacttttttttcaaggcaatcagggtatattatattgtacttcagcacagttttagagaacaattgttataattaaatgataaggtagaatatttctgcatataaattctggctggcgtggaaatattcttattggtagaaacaactacaccctggtcatcatcctgcctttctctttatggttacaatgatatacactgtttgagatgaggataaaatactctgagtccaaaccgggcccctctgctaaccatgttcatgccttcttctctttcctacagctcctgggcaacgtgctggttgttgtgctgtctcatcattttggcaaagaattcactcctcaggtgcaggctgcctatcagaaggtggtggctggtgtggccaatgccctggctcacaaataccactgagatctttttccctctgccaaaaattatggggacatcatgaagccccttgagcatctgacttctggctaataaaggaaatttattttcattgcaatagtgtgttggaattttttgtgtctctcactctagagcggccgcggatccaattctaccgggtaggggaggcgcttttcccaaggcagtctggagcatgcgctttagcagccccgctgggcacttggcgctacacaagtggcctctggcctcgcacacattccacatccaccggtaggcgccaaccggctccgttctttggtggccccttcgcgccaccttctactcctcccctagtcaggaagttcccccccgccccgcagctcgcgtcgtgcaggacgtgacaaatggaagtagcacgtctcactagtctcgtgcagatggacagcaccgctgagcaatggaagcgggtaggcctttggggcagcggccaatagcagctttgctccttcgctttctgggctcagaggctgggaaggggtgggtccgggggcgggctcaggggcgggctcaggggcggggcgggcgcccgaaggtcctccggaggcccggcattctgcacgcttcaaaagcgcacgtctgccgcgctgttctcctcttcctcatctccgggcctttcgacctgcagttaacgccgccatggatagatccggaaagcctgaactcaccgcgacgtctgtcgagaagtttctgatcgaaaagttcgacagcgtctccgacctgatgcagctctcggagggcgaagaatctcgtgctttcagcttcgatgtaggagggcgtggatatgtcctgcgggtaaatagctgcgccgatggtttctacaaagatcgttatgtttatcggcactttgcatcggccgcgctcccgattccggaagtgcttgacattggggaattcagcgagagcctgacctattgcatctcccgccgtgcacagggtgtcacgttgcaagacctgcctgaaaccgaactgcccgctgttctgcagccggtcgcggaggccatggatgcgatcgctgcggccgatcttagccagacgagcgggttcggcccattcggaccgcaaggaatcggtcaatacactacatggcgtgatttcatatgcgcgattgctgatccccatgtgtatcactggcaaactgtgatggacgacaccgtcagtgcgtccgtcgcgcaggctctcgatgagctgatgctttgggccgaggactgccccgaagtccggcacctcgtgcacgcggatttcggctccaacaatgtcctgacggacaatggccgcataacagcggtcattgactggagcgaggcgatgttcggggattcccaatacgaggtcgccaacatcttcttctggaggccgtggttggcttgtatggagcagcagacgcgctacttcgagcggaggcatccggagcttgcaggatcgccgcggctccgggcgtatatgctccgcattggtcttgaccaactctatcagagcttggttgacggcaatttcgatgatgcagcttgggcgcagggtcgatgcgacgcaatcgtccgatccggagccgggactgtcgggcgtacacaaatcgcccgcagaagcgcggccgtctggaccgatggctgtgtagaagtactcgccgatagtggaaaccgacgccccagcactcgtccgagggcaaaggaatagacgcgtctggaacaatcaacctctggattacaaaatttgtgaaagattgactggtattcttaactatgttgctccttttacgctatgtggatacgctgctttaatgcctttgtatcatgctattgcttcccgtatggctttcattttctcctccttgtataaatcctggttgctgtctctttatgaggagttgtggcccgttgtcaggcaacgtggcgtggtgtgcactgtgtttgctgacgcaacccccactggttggggcattgccaccacctgtcagctcctttccgggactttcgctttccccctccctattgccacggcggaactcatcgccgcctgccttgcccgctgctggacaggggctcggctgttgggcactgacaattccgtggtgttgtcggggaagctgacgtcctttccatggctgctcgcctgtgttgccacctggattctgcgcgggacgtccttctgctacgtcccttcggccctcaatccagcggaccttccttcccgcggcctgctgccggctctgcggcctcttccgcgtcttcgccttcgccctcagacgagtcggatctccctttgggccgcctccccgcctggaattaattctgcagtcgagacctagaaaaacatggagcaatcacaagtagcaatacagcagctaccaatgctgattgtgcctggctagaagcacaagaggaggaggaggtgggttttccagtcacacctcaggtacctttaagaccaatgacttacaaggcagctgtagatcttagccactttttaaaagaaaagaggggactggaagggctaattcactcccaacgaagacaagatctgctttttgcttgtactgggtctctctggttagaccagatctgagcctgggagctctctggctaactagggaacccactgcttaagcctcaataaagcttgccttgagtgcttcaagtagtgtgtgcccgtctgttgtgtgactctggtaactagagatccctcagacccttttagtcagtgtggaaaatctctagcagtagtagttcatgtcatcttattattcagtatttataacttgcaaagaaatgaatatcagagagtgagaggccttgacattgctagcgttttaccgtcgacctctagctagagcttggcgtaatcatggtcatagctgtttcctgtgtgaaattgttatccgctcacaattccacacaacatacgagccggaagcataaagtgtaaagcctggggtgcctaatgagtgagctaactcacattaattgcgttgcgctcactgcccgctttccagtcgggaaacctgtcgtgccagctgcattaatgaatcggccaacgcgcggggagaggcggtttgcgtattgggcgctcttccgcttcctcgctcactgactcgctgcgctcggtcgttcggctgcggcgagcggtatcagctcactcaaaggcggtaatacggttatccacagaatcaggggataacgcaggaaagaacatgtgagcaaaaggccagcaaaaggccaggaaccgtaaaaaggccgcgttgctggcgtttttccataggctccgcccccctgacgagcatcacaaaaatcgacgctcaagtcagaggtggcgaaacccgacaggactataaagataccaggcgtttccccctggaagctccctcgtgcgctctcctgttccgaccctgccgcttaccggatacctgtccgcctttctcccttcgggaagcgtggcgctttctcatagctcacgctgtaggtatctcagttcggtgtaggtcgttcgctccaagctgggctgtgtgcacgaaccccccgttcagcccgaccgctgcgccttatccggtaactatcgtcttgagtccaacccggtaagacacgacttatcgccactggcagcagccactggtaacaggattagcagagcgaggtatgtaggcggtgctacagagttcttgaagtggtggcctaactacggctacactagaagaacagtatttggtatctgcgctctgctgaagccagttaccttcggaaaaagagttggtagctcttgatccggcaaacaaaccaccgctggtagcggtggtttttttgtttgcaagcagcagattacgcgcagaaaaaaaggatctcaagaagatcctttgatcttttctacggggtctgacgctcagtggaacgaaaactcacgttaagggattttggtcatgagattatcaaaaaggatcttcacctagatccttttaaattaaaaatgaagttttaaatcaatctaaagtatatatgagtaaacttggtctgacagttaccaatgcttaatcagtgaggcacctatctcagcgatctgtctatttcgttcatccatagttgcctgactccccgtcgtgtagataactacgatacgggagggcttaccatctggccccagtgctgcaatgataccgcgagacccacgctcaccggctccagatttatcagcaataaaccagccagccggaagggccgagcgcagaagtggtcctgcaactttatccgcctccatccagtctattaattgttgccgggaagctagagtaagtagttcgccagttaatagtttgcgcaacgttgttgccattgctacaggcatcgtggtgtcacgctcgtcgtttggtatggcttcattcagctccggttcccaacgatcaaggcgagttacatgatcccccatgttgtgcaaaaaagcggttagctccttcggtcctccgatcgttgtcagaagtaagttggccgcagtgttatcactcatggttatggcagcactgcataattctcttactgtcatgccatccgtaagatgcttttctgtgactggtgagtactcaaccaagtcattctgagaatagtgtatgcggcgaccgagttgctcttgcccggcgtcaatacgggataataccgcgccacatagcagaactttaaaagtgctcatcattggaaaacgttcttcggggcgaaaactctcaaggatcttaccgctgttgagatccagttcgatgtaacccactcgtgcacccaactgatcttcagcatcttttactttcaccagcgtttctgggtgagcaaaaacaggaaggcaaaatgccgcaaaaaagggaataagggcgacacggaaatgttgaatactcatactcttcctttttcaatattattgaagcatttatcagggttattgtctcatgagcggatacatatttgaatgtatttagaaaaataaacaaataggggttccgcgcacatttccccgaaaagtgccacctgacgtcgacggatcgggagatcaacttgtttattgcagcttataatggttacaaataaagcaatagcatcacaaatttcacaaataaagcatttttttcactgcattctagttgtggtttgtccaaactcatcaatgtatcttatcatgtctggatcaactggataactcaagctaaccaaaatcatcccaaacttcccaccccataccctattaccactgccaattacctgtggtttcatttactctaaacctgtgattcctctgaattattttcattttaaagaaattgtatttgttaaatatgtactacaaacttagtagt

SEQ ID NO: 24 - DNA, 30 bp, Artificial Sequence
  primer
taagcggccgcacccgccgtctggatcatg

SEQ ID NO: 25 - DNA, 30 bp, Artificial Sequence
  primer
taagcggccgcggcggctgcgcagatcaga

SEQ ID NO: 26 - DNA, 30 bp, Artificial Sequence
  primer
taagcggccgcttgcttgttaatcaataaa

SEQ ID NO: 27 - DNA, 30 bp, Artificial Sequence
  primer
taagcggccgcttcagagagagtgtcctcg

SEQ ID NO: 28 - DNA, 30 bp, Artificial Sequence
  primer
taagcggccgcgttttagggcggagtaact

SEQ ID NO: 29 - DNA, 30 bp, Artificial Sequence
  primer
taagcggccgcggatccatcgcgccctgta

SEQ ID NO: 30 - DNA, 30 bp, Artificial Sequence
  primer
taagcggccgcggatgttgcccctcctgac

SEQ ID NO: 31 - DNA, 30 bp, Artificial Sequence
  primer
taagcggccgcgcccgggcgaccgcaccct

SEQ ID NO: 32 - DNA, 30 bp, Artificial Sequence
  primer
taagcggccgctacgtcgacgtttaaacca

SEQ ID NO: 33 - DNA, 30 bp, Artificial Sequence
  primer
taagcggccgctagtgaatccacagaaact

SEQ ID NO: 34 - DNA, 30 bp, Artificial Sequence
  primer
taagcggccgcacttaatgctttcgctttc

SEQ ID NO: 35 - DNA, 30 bp, Artificial Sequence
  primer
taagcggccgcttgcttttcccagatgcat

SEQ ID NO: 36 - DNA, 30 bp, Artificial Sequence
  primer
taagcggccgcgcttacaggctctcctttt

SEQ ID NO: 37 - DNA, 30 bp, Artificial Sequence
  primer
taagcggccgcggcttccttccaggcgcgg

SEQ ID NO: 38 - DNA, 9665 bp, Artificial Sequence
  plasmid
tcgcgcgtttcggtgatgacggtgaaaacctctgacacatgcagctcccggagactgtcacagcttgtctgtaagcggatgccgggagcagacaagcccgtcagggcgcgtcagcgggtgttggcgggtgtcggggctggcttaactatgcggcatcagagcagattgtactgagagtgcaccatatgcggtgtgaaataccgcacagatgcgtaaggagaaaataccgcatcaggcgccattcgccattcaggctgcgcaactgttgggaagggcgatcggtgcgggcctcttcgctattacgccagctggcgaaagggggatgtgctgcaaggcgattaagttgggtaacgccagggttttcccagtcacgacgttgtaaaacgacggccagtgaattgacgcgtattgggatgacattgattattgactagttattaatagtaatcaattacggggtcattagttcatagcccatatatggagttccgcgttacataacttacggtaaatggcccgcctggctgaccgcccaacgacccccgcccattgacgtcaataatgacgtatgttcccatagtaacgccaatagggactttccattgacgtcaatgggtggagtatttacggtaaactgcccacttggcagtacatcaagtgtatcatatgccaagtacgccccctattgacgtcaatgacggtaaatggcccgcctggcattatgcccagtacatgaccttatgggactttcctacttggcagtacatctacgtattagtcatcgctattaccatggtgatgcggttttggcagtacatcaatgggcgtggatagcggtttgactcacggggatttccaagtctccaccccattgacgtcaatgggagtttgttttggaaccaaaatcaacgggactttccaaaatgtcgtaacaactccgccccattgacgcaaatgggcggtaggcgtgtacggtgggaggtctatataagcagagctctccctatcagtgatagagatctccctatcagtgatagagatcgtcgacgagctcgtttagtgaaccgtcagatcgcctggagacgccatccacgctgttttgacctccatagaagacaccgggaccgatccagcctccggactctagcgtttaaacttaagcttgccaccatgactacgtccggcgttccatttggcatgacactacgaccaacacgatctcggttgtctcggcgcactccgtacagtagggatcgcctacctccttttgagacagagacccgcgctaccatactggaggatcatccgctgctgcccgaatgtaacactttgacaatgcacaacgtgagttacgtgcgaggtcttccctgcagtgtgggatttacgctgattcaggaatgggttgttccctgggatatggttctgacgcgggaggagcttgtaatcctgaggaagtgtatgcacgtgtgcctgtgttgtgccaacattgatatcatgacgagcatgatgatccatggttacgagtcctgggctctccactgtcattgttccagtcccggttccctgcagtgcatagccggcgggcaggttttggccagctggtttaggatggtggtggatggcgccatgtttaatcagaggtttatatggtaccgggaggtggtgaattacaacatgccaaaagaggtaatgtttatgtccagcgtgtttatgaggggtcgccacttaatctacctgcgcttgtggtatgatggccacgtgggttctgtggtccccgccatgagctttggatacagcgccttgcactgtgggattttgaacaatattgtggtgctgtgctgcagttactgtgctgatttaagtgagatcagggtgcgctgctgtgcccggaggacaaggcgtctcatgctgcgggcggtgcgaatcatcgctgaggagaccactgccatgttgtattcctgcaggacggagcggcggcggcagcagtttattcgcgcgctgctgcagcaccaccgccctatcctgatgcacgattatgactctacccccatgtaggcggccgctcgagtctagagggcccgtttaaacccgctgatcagcctcgactgtgccttctagttgccagccatctgttgtttgcccctcccccgtgccttccttgaccctggaaggtgccactcccactgtcctttcctaataaaatgaggaaattgcatcgcattgtctgagtaggtgtcattctattctggggggtggggtggggcaggacagcaagggggaggattgggaagacaatagcaggcatgctggggatgcggtgggctctatggatccgtattgggatgcggccgcaatatttgcatgtcgctatgtgttctgggaaatcaccataaacgtgaaatccctatcagtgatagagacttataagttccctatcagtgatagagaaccggtgggcactcttccgtggtctggtggataaattcgcaagggtatcatggcggacgaccggggttcgaaccccggatccggccgtccgccgtgatccatgcggttaccgcccgcgtgtcgaacccaggtgtgcgacgtcagacaacgggggagcgctcctttttgaattccactttggccgcggctcgaggacattgattattgactagttattaatagtaatcaattacggggtcattagttcatagcccatatatggagttccgcgttacataacttacggtaaatggcccgcctggctgaccgcccaacgacccccgcccattgacgtcaataatgacgtatgttcccatagtaacgccaatagggactttccattgacgtcaatgggtggagtatttacggtaaactgcccacttggcagtacatcaagtgtatcatatgccaagtacgccccctattgacgtcaatgacggtaaatggcccgcctggcattatgcccagtacatgaccttatgggactttcctacttggcagtacatctacgtattagtcatcgctattaccatggtgatgcggttttggcagtacatcaatgggcgtggatagcggtttgactcacggggatttccaagtctccaccccattgacgtcaatgggagtttgttttggcaccaaaatcaacgggactttccaaaatgtcgtaacaactccgccccattgacgcaaatgggcggtaggcgtgtacggtgggaggtctatataagcagagctcgtttagtgaaccgtcagatcgcctggagacgccatccacgctgttttgacctccatagaagacaccgggaccgatccagcctccgcggccccgaattcaccatgtctagattagataaaagtaaagtgattaacagcgcattagagctgcttaatgaggtcggaatcgaaggtttaacaacccgtaaactcgcccagaagctaggtgtagagcagcctacattgtattggcacgtgcgcaacaagcagactcttatgaacatgctttcagaggcaatactggcgaagcatcacacccgttcagcaccgttaccgactgagagttggcagcagtttctccaggaaaatgctctgagtttccgtaaagcattactggtccatcgtgatggagcccgattgcatatagggacctctcctacgcccccccagtttgaacaagcagaggcgcaactacgctgtctatgcgatgcagggttttcggtcgaggaggctcttttcattctgcaatctatcagccattttacgttgggtgcagtattagaggagcaagcaacaaaccagatagaaaataatcatgtgatagacgctgcaccaccattattacaagaggcatttaatattcaggcgagaacctctgctgaaatggccttccatttcgggctgaaatcattaatatttggattttctgcacagttagatgaaaaaaagcatacacccattgaggatggtaataaaccaaaaaagaagagaaagctagcagtgtcagtgacatttgaagatgtggctgtgctctttactcgggacgagtggaagaagctggatctgtctcagagaagcctgtaccgtgaggtgatgctggagaattacagcaacctggcctccatggcaggattcctgtttaccaaaccaaaggtgatctccctgttgcagcaaggagaggatccctggtaaatcgatctgagaacttcagggtgagtttggggacccttgattgttctttctttttcgctattgtaaaattcatgttatatggagggggcaaagttttcagggtgttgtttagaatgggaagatgtcccttgtatcaccatggaccctcatgataattttgtttctttcactttctactctgttgacaaccattgtctcctcttattttcttttcattttctgtaactttttcgttaaactttagcttgcatttgtaacgaatttttaaattcacttttgtttatttgtcagattgtaagtactttctctaatcacttttttttcaaggcaatcagggtatattatattgtacttcagcacagttttagagaacaattgttataattaaatgataaggtagaatatttctgcatataaattctggctggcgtggaaatattcttattggtagaaacaactacaccctggtcatcatcctgcctttctctttatggttacaatgatatacactgtttgagatgaggataaaatactctgagtccaaaccgggcccctctgctaaccatgttcatgccttcttctctttcctacagctcctgggcaacgtgctggttgttgtgctgtctcatcattttggcaaagaattcactcctcaggtgcaggctgcctatcagaaggtggtggctggtgtggccaatgccctggctcacaaataccactgagatctttttccctctgccaaaaattatggggacatcatgaagccccttgagcatctgacttctggctaataaaggaaatttattttcattgcaatagtgtgttggaattttttgtgtctctcactctagagcggccgcggatccaattctaccgggtaggggaggcgcttttcccaaggcagtctggagcatgcgctttagcagccccgctgggcacttggcgctacacaagtggcctctggcctcgcacacattccacatccaccggtaggcgccaaccggctccgttctttggtggccccttcgcgccaccttctactcctcccctagtcaggaagttcccccccgccccgcagctcgcgtcgtgcaggacgtgacaaatggaagtagcacgtctcactagtctcgtgcagatggacagcaccgctgagcaatggaagcgggtaggcctttggggcagcggccaatagcagctttgctccttcgctttctgggctcagaggctgggaaggggtgggtccgggggcgggctcaggggcgggctcaggggcggggcgggcgcccgaaggtcctccggaggcccggcattctgcacgcttcaaaagcgcacgtctgccgcgctgttctcctcttcctcatctccgggcctttcgacctgcagttaacgccgccatggatagatccggaaagcctgaactcaccgcgacgtctgtcgagaagtttctgatcgaaaagttcgacagcgtctccgacctgatgcagctctcggagggcgaagaatctcgtgctttcagcttcgatgtaggagggcgtggatatgtcctgcgggtaaatagctgcgccgatggtttctacaaagatcgttatgtttatcggcactttgcatcggccgcgctcccgattccggaagtgcttgacattggggaattcagcgagagcctgacctattgcatctcccgccgtgcacagggtgtcacgttgcaagacctgcctgaaaccgaactgcccgctgttctgcagccggtcgcggaggccatggatgcgatcgctgcggccgatcttagccagacgagcgggttcggcccattcggaccgcaaggaatcggtcaatacactacatggcgtgatttcatatgcgcgattgctgatccccatgtgtatcactggcaaactgtgatggacgacaccgtcagtgcgtccgtcgcgcaggctctcgatgagctgatgctttgggccgaggactgccccgaagtccggcacctcgtgcacgcggatttcggctccaacaatgtcctgacggacaatggccgcataacagcggtcattgactggagcgaggcgatgttcggggattcccaatacgaggtcgccaacatcttcttctggaggccgtggttggcttgtatggagcagcagacgcgctacttcgagcggaggcatccggagcttgcaggatcgccgcggctccgggcgtatatgctccgcattggtcttgaccaactctatcagagcttggttgacggcaatttcgatgatgcagcttgggcgcagggtcgatgcgacgcaatcgtccgatccggagccgggactgtcgggcgtacacaaatcgcccgcagaagcgcggccgtctggaccgatggctgtgtagaagtactcgccgatagtggaaaccgacgccccagcactcgtccgagggcaaaggaatagacgcgtctggaacaatcaacctctggattacaaaatttgtgaaagattgactggtattcttaactatgttgctccttttacgctatgtggatacgctgctttaatgcctttgtatcatgctattgcttcccgtatggctttcattttctcctccttgtataaatcctggttgctgtctctttatgaggagttgtggcccgttgtcaggcaacgtggcgtggtgtgcactgtgtttgctgacgcaacccccactggttggggcattgccaccacctgtcagctcctttccgggactttcgctttccccctccctattgccacggcggaactcatcgccgcctgccttgcccgctgctggacaggggctcggctgttgggcactgacaattccgtggtgttgtcggggaagctgacgtcctttccatggctgctcgcctgtgttgccacctggattctgcgcgggacgtccttctgctacgtcccttcggccctcaatccagcggaccttccttcccgcggcctgctgccggctctgcggcctcttccgcgtcttcgccttcgccctcagacgagtcggatctccctttgggccgcctccccgcctggaattaattctgcagtcgagacctagaaaaacatggagcaatcacaagtagcaatacagcagctaccaatgctgattgtgcctggctagaagcacaagaggaggaggaggtgggttttccagtcacacctcaggtacctttaagaccaatgacttacaaggcagctgtagatcttagccactttttaaaagaaaagaggggaccaatggcgcgccgagcttggcgtaatcatggtcatagctgtttcctgtgtgaaattgttatccgctcacaattccacacaacatacgagccggaagcataaagtgtaaagcctggggtgcctaatgagtgagctaactcacattaattgcgttgcgctcactgcccgctttccagtcgggaaacctgtcgtgccagctgcattaatgaatcggccaacgcgcggggagaggcggtttgcgtattgggcgctgttccgcttcctcgctcactgactcgctgcgctcggtcgttcggctgcggcgagcggtatcagctcactcaaaggcggtaatacggttatccacagaatcaggggataacgcaggaaagaacatgtgagcaaaaggccagcaaaaggccaggaaccgtaaaaaggccgcgttgctggcgtttttccataggctccgcccccctgacgagcatcacaaaaatcgacgctcaagtcagaggtggcgaaacccgacaggactataaagataccaggcgtttccccctggaagctccctcgtgcgctctcctgttccgaccctgccgcttaccggatacctgtccgcctttctcccttcgggaagcgtggcgctttctcatagctcacgctgtaggtatctcagttcggtgtaggtcgttcgctccaagctgggctgtgtgcacgaaccccccgttcagcccgaccgctgcgccttatccggtaactatcgtcttgagtccaacccggtaagacacgacttatcgccactggcagcagccactggtaacaggattagcagagcgaggtatgtaggcggtgctacagagttcttgaagtggtggcctaactacggctacactagaagaacagtatttggtatctgcgctctgctgaagccagttaccttcggaaaaagagttggtagctcttgatccggcaaacaaaccaccgctggtagcggtggtttttttgtttgcaagcagcagattacgcgcagaaaaaaaggatctcaagaagatcctttgatcttttctacggggtctgacgctcagtggaacgaaaactcacgttaagggattttggtcatgagattatcaaaaaggatcttcacctagatccttttaaattaaaaatgaagttttaaatcaatctaaagtatatatgagtaaacttggtctgacagttaccaatgcttaatcagtgaggcacctatctcagcgatctgtctatttcgttcatccatagttgcctgactccccgtcgtgtagataactacgatacgggagggcttaccatctggccccagtgctgcaatgataccgcgagaaccacgctcaccggctccagatttatcagcaataaaccagccagccggaagggccgagcgcagaagtggtcctgcaactttatccgcctccatccagtctattaattgttgccgggaagctagagtaagtagttcgccagttaatagtttgcgcaacgttgttgccattgctacaggcatcgtggtgtcacgctcgtcgtttggtatggcttcattcagctccggttcccaacgatcaaggcgagttacatgatcccccatgttgtgcaaaaaagcggttagctccttcggtcctccgatcgttgtcagaagtaagttggccgcagtgttatcactcatggttatggcagcactgcataattctcttactgtcatgccatccgtaagatgcttttctgtgactggtgagtactcaaccaagtcattctgagaatagtgtatgcggcgaccgagttgctcttgcccggcgtcaatacgggataataccgcgccacatagcagaactttaaaagtgctcatcattggaaaacgttcttcggggcgaaaactctcaaggatcttaccgctgttgagatccagttcgatgtaacccactcgtgcacccaactgatcttcagcatcttttactttcaccagcgtttctgggtgagcaaaaacaggaaggcaaaatgccgcaaaaaagggaataagggcgacacggaaatgttgaatactcatactcttcctttttcaatattattgaagcatttatcagggttattgtctcatgagcggatacatatttgaatgtatttagaaaaataaacaaataggggttccgcgcacatttccccgaaaagtgccacctgacgtctaagaaaccattattatcatgacattaacctataaaaataggcgtatcacgaggcccttttgtc

SEQ ID NO: 39 - DNA, 11389 bp, Artificial Sequence
  plasmid
tgtacactactagggacaggattggtgacagaaaagccccatccttaggcctcctccttcctagtctcctgatattgggtctaacccccacctcctgttaggcagattccttatctggtgacacacccccatttcctggagccatctctctccttgccagaacctctaaggtttgcttacgatggagccagagaggatcctgggagggagagcttggcagggggtgggagggaagggggggatgcgtgacctgcccggttctcagtggccaccctgcgctaccctctcccagaacctgagctgctctgacgcggctgtctggtgcgtttcactgatcctggtgctgcagcttccttacacttcccaagaggagaagcagtttggaaaaacaaaatcagaataagttggtcctgagttctaactttggctcttcacctttctagtccccaatttatattgttcctccgtgcgtcagttttacctgtgagataaggccagtagccagccccgtcctggcagggctgtggtgaggaggggggtgtccgtgtggaaaactccctttgtgagaatggtgcgtcctaggtgttcaccaggtcgtggccgcctctactccctttctctttctccatccttctttccttaaagagtccccagtgctatctgggacatattcctccgcccagagcagggtcccgcttccctaaggccctgctctgggcttctgggtttgagtccttggcaagcccaggagaggcgctcaggcttccctgtcccccttcctcgtccaccatctcatgcccctggctctcctgccccttccctacaggggttcctggctctgctctctcgagatgcatgcgtcaattttacgcagactatctttctagggttaatctagctgcatcaggatcatatcgtcgggtcttttttccggctcagtcatcgcccaagctggcgctatctgggcatcggggaggaagaagcccgtgccttttcccgcgaggttgaagcggcatggaaagagtttgccgaggatgactgctgctgcattgacgttgagcgaaaacgcacgtttaccatgatgattcgggaaggtgtggccatgcacgcctttaacggtgaactgttcgttcaggccacctgggataccagttcgtcgcggcttttccggacacagttccggatggtcagcccgaagcgcatcagcaacccgaacaataccggcgacagccggaactgccgtgccggtgtgcagattaatgacagcggtgcggcgctgggatattacgtcagcgaggacgggtatcctggctggatgccgcagaaatggacatggataccccgtgagttacccggcgggcgcgcttggcgtaatcatggtcatagctgtttcctgtgtgaaattgttatccgctcacaattccacacaacatacgagccggaagcataaagtgtaaagcctggggtgcctaatgagtgagctaactcacattaattgcgttgcgctcactgcccgctttccagtcgggaaacctgtcgtgccagctgcattaatgaatcggccaacgcgcggggagaggcggtttgcgtattgggcgctcttccgcttcctcgctcactgactcgctgcgctcggtcgttcggctgcggcgagcggtatcagctcactcaaaggcggtaatacggttatccacagaatcaggggataacgcaggaaagaacatgtgagcaaaaggccagcaaaaggccaggaaccgtaaaaaggccgcgttgctggcgtttttccataggctccgcccccctgacgagcatcacaaaaatcgacgctcaagtcagaggtggcgaaacccgacaggactataaagataccaggcgtttccccctggaagctccctcgtgcgctctcctgttccgaccctgccgcttaccggatacctgtccgcctttctcccttcgggaagcgtggcgctttctcatagctcacgctgtaggtatctcagttcggtgtaggtcgttcgctccaagctgggctgtgtgcacgaaccccccgttcagcccgaccgctgcgccttatccggtaactatcgtcttgagtccaacccggtaagacacgacttatcgccactggcagcagccactggtaacaggattagcagagcgaggtatgtaggcggtgctacagagttcttgaagtggtggcctaactacggctacactagaaggacagtatttggtatctgcgctctgctgaagccagttaccttcggaaaaagagttggtagctcttgatccggcaaacaaaccaccgctggtagcggtggtttttttgtttgcaagcagcagattacgcgcagaaaaaaaggatctcaagaagatcctttgatcttttctacggggtctgacgctcagtggaacgaaaactcacgttaagggattttggtcatgagattatcaaaaaggatcttcacctagatccttttaaattaaaaatgaagttttaaatcaatctaaagtatatatgagtaaacttggtctgacagttaccaatgcttaatcagtgaggcacctatctcagcgatctgtctatttcgttcatccatagttgcctgactccccgtcgtgtagataactacgatacgggagggcttaccatctggccccagtgctgcaatgataccgcgagacccacgctcaccggctccagatttatcagcaataaaccagccagccggaagggccgagcgcagaagtggtcctgcaactttatccgcctccatccagtctattaattgttgccgggaagctagagtaagtagttcgccagttaatagtttgcgcaacgttgttgccattgctacaggcatcgtggtgtcacgctcgtcgtttggtatggcttcattcagctccggttcccaacgatcaaggcgagttacatgatcccccatgttgtgcaaaaaagcggttagctccttcggtcctccgatcgttgtcagaagtaagttggccgcagtgttatcactcatggttatggcagcactgcataattctcttactgtcatgccatccgtaagatgcttttctgtgactggtgagtactcaaccaagtcattctgagaatagtgtatgcggcgaccgagttgctcttgcccggcgtcaatacgggataataccgcgccacatagcagaactttaaaagtgctcatcattggaaaacgttcttcggggcgaaaactctcaaggatcttaccgctgttgagatccagttcgatgtaacccactcgtgcacccaactgatcttcagcatcttttactttcaccagcgtttctgggtgagcaaaaacaggaaggcaaaatgccgcaaaaaagggaataagggcgacacggaaatgttgaatactcatactcttcctttttcaatattattgaagcatttatcagggttattgtctcatgagcggatacatatttgaatgtatttagaaaaataaacaaataggggttccgcgcacatttccccgaaaagtgccacctaaattgtaagcgttaatattttgttaaaattcgcgttaaatttttgttaaatcagctcattttttaaccaataggccgaaatcggcaaaatcccttataaatcaaaagaatagaccgagatagggttgagtgttgttccagtttggaacaagagtccactattaaagaacgtggactccaacgtcaaagggcgaaaaaccgtctatcagggcgatggcccactacgtgaaccatcaccctaatcaagttttttggggtcgaggtgccgtaaagcactaaatcggaaccctaaagggagcccccgatttagagcttgacggggaaagccggcgaacgtggcgagaaaggaagggaagaaagcgaaaggagcgggcgctagggcgctggcaagtgtagcggtcacgctgcgcgtaaccaccacacccgccgcgcttaatgcgccgctacagggcgcgtcccattcgccattcaggctgcgcaactgttgggaagggcgatcggtgcgggcctcttcgctattacgccagctggcgaaagggggatgtgctgcaaggcgattaagttgggtaacgccagggttttcccagtcacgacgttgtaaaacgacggccagtgagcgcgcctcgttcattcacgtttttgaacccgtggaggacgggcagactcgcggtgcaaatgtgttttacagcgtgatggagcagatgaagatgctcgacacgctgcagaacacgcagctagattaaccctagaaagataatcatattgtgacgtacgttaaagataatcatgcgtaaaattgacgcatgtgttttatcggtctgtatatcgaggtttatttattaatttgaatagatattaagttttattatatttacacttacatactaataataaattcaacaaacaatttatttatgtttatttatttattaaaaaaaaacaaaaactcaaaatttcttctataaagtaacaaaacttttatgagggacagcccccccccaaagcccccagggatgtaattacgtccctcccccgctagggggcagcagcgagccgcccggggctccgctccggtccggcgctccccccgcatccccgagccggcagcgtgcggggacagcccgggcacggggaaggtggcacgggatcgctttcctctgaacgcttctcgctgctctttgagcctgcagacacctggggggatacggggaaaaggcctccaaggcctactagtaacggccgccagtgtgctggaattcgcccttggtacctgctttctctgaccagcattctctcccctgggcctgtgccgctttctgtctgcagcttgtggcctgggtcacctctacggctggcccagatccttccctgccgcctccttcaggttccgtcttcctccactccctcttccccttgctctctgctgtgttgctgcccaaggatgctctttccggagcacttccttctcggcgctgcaccacgtgatgtcctctgagcggatcctccccgtgtctgggtcctctccgggcatctctcctccctcacccaaccccatgccgtcttcactcgctgggttcccttttccttctccttctggggcctgtgccatctctcgtttcttaggatggccttctccgacggatgtctcccttgcgtcccgcctccccttcttgtaggcctgcatcatcaccgtttttctggacaaccccaaagtaccccgtctccctggctttagccacctctccatcctcttgctttctttgcctggacaccccgttctcctgtggattcgggtcacctctcactcctttcatttgggcagctcccctaccccccttacctctctagtctgtgctagctcttccagccccctgtcatggcatcttccaggggtccgagagctcagctagtcttcttcctccaacccgggcccctatgtccacttcaggacagcatgtttgctgcctccagggatcctgtgtccccgagctgggaccaccttatattcccagggccggttaatgtggctctggttctgggtacttttatctgtcccctccaccccacagtggggcacgcgtaagggcgaattctgcagatatccatcacactggcggccgctcgagcatgcatctagtattatgcccagtacatgaccttatgggactttcctacttggcagtacatctacgtattagtcatcgctattaccatggtgatgcggttttggcagtacatcaatgggcgtggatagcggtttgactcacggggatttccaagtctccaccccattgacgtcaatgggagtttgttttggcaccaaaatcaacgggactttccaaaatgtcgtaacaactccgccccattgacgcaaatgggcggtaggcgtgtacggtgggaggtctatataagcagagctcgtttagtgaaccgtcagatcgcctggagacgccatccacgctgttttgacctccatagaagattctagaatggcccttagtaagcacggcctgactaaggacatgaccatgaagtaccatatggagggctcggtggacgggcacaagttcgtgattacgggccacgggaacggcaacccattcgaggggaaacagacaatgaacctgtgtgtggtggaaggcggacccctgcccttctcggaggacatcctgtccgcaacctttgactacggcaatcgcgtgttcacagagtatccacagggtatggtggatttctttaagaacagctgtcccgcaggatacacctggcaccgcagcctgctcttcgaggacggggcggtgtgtaccacctccgctgatatcaccgtgtccgtcgaggagaactgcttctaccacaacagcaaattccacggcgtgaactttcctgccgacgggcctgtgatgaagaaaatgactacgaattgggagcccagctgcgagaaaatcatcccggtccctcgtcagggaatcttgaagggcgacatcgcaatgtacctcctgctcaaggacgggggaagataccgatgccagttcgataccatctacaaggcaaagtccgatcccaaggagatgccagagtggcacttcatccagcacaaactcacccgcgaggaccgctcagatgccaagaaccagaagtggcaactggtcgagcacgccgtggcatcccgtagcgccctgccagggtaattcgaatttaaatcggatccctgtgccttctagttgccagccatctgttgtttgcccctcccccgtgccttccttgaccctggaaggtgccactcccactgtcctttcctaataaaatgaggaaattgcatcgcattgtctgagtaggtgtcattctattctggggggtggggtggggcaggacagcaagggggaggattgggaagacaatagcaggcatgctggggatgcggtgggctctatggagatctctgatctgcgcagccgccatgccggggttttacgagattgtgattaaggtccccagcgaccttgacgagcatctgcccggcatttctgacagctttgtgaactgggtggccgagaaggaatgggagttgccgccagattctgacatggatctgaatctgattgagcaggcacccctgaccgtggccgagaagctgcagcgcgactttctgacggaatggcgccgtgtgagtaaggccccggaggcccttttctttgtgcaatttgagaagggagagagctacttccacatgcacgtgctcgtggaaaccaccggggtgaaatccatggttttgggacgtttcctgagtcagattcgcgaaaaactgattcagagaatttaccgcgggatcgagccgactttgccaaactggttcgcggtcacaaagaccagaaatggcgccggaggcgggaacaaggtggtggatgagtgctacatccccaattacttgctccccaaaacccagcctgagctccagtgggcgtggactaatatggaacagtatttaagcgcctgtttgaatctcacggagcgtaaacggttggtggcgcagcatctgacgcacgtgtcgcagacgcaggagcagaacaaagagaatcagaatcccaattctgatgcgccggtgatcagatcaaaaacttcagccaggtacatggagctggtcgggtggctcgtggacaaggggattacctcggagaagcagtggatccaggaggaccaggcctcatacatctccttcaatgcggcctccaactcgcggtcccaaatcaaggctgccttggacaatgcgggaaagattatgagcctgactaaaaccgcccccgactacctggtgggccagcagcccgtggaggacatttccagcaatcggatttataaaattttggaactaaacgggtacgatccccaatatgcggcttccgtctttctgggatgggccacgaaaaagttcggcaagaggaacaccatctggctgtttgggcctgcaactaccgggaagaccaacatcgcggaggccatagcccacactgtgcccttctacgggtgcgtaaactggaccaatgagaactttcccttcaacgactgtgtcgacaagatggtgatctggtgggaggaggggaagatgaccgccaaggtcgtggagtcggccaaagccattctcggaggaagcaaggtgcgcgtggaccagaaatgcaagtcctcggcccagatagacccgactcccgtgatcgtcacctccaacaccaacatgtgcgccgtgattgacgggaactcaacgaccttcgaacaccagcagccgttgcaagaccggatgttcaaatttgaactcacccgccgtctggatcatgactttgggaaggtcaccaagcaggaagtcaaagactttttccggtgggcaaaggatcacgtggttgaggtggagcatgaattctacgtcaaaaagggtggagccaagaaaagacccgcccccagtgacgcagatataagtgagcccaaacgggtgcgcgagtcagttgcgcagccatcgacgtcagacgcggaagcttcgatcaactacgcagacaggtaccaaaacaaatgttctcgtcacgtgggcatgaatctgatgctgtttccctgcagacaatgcgagagaatgaatcagaattcaaatatctgcttcactcacggacagaaagactgtttagagtgctttcccgtgtcagaatctcaacccgtttctgtcgtcaaaaaggcgtatcagaaactgtgctacattcatcatatcatgggaaaggtgccagacgcttgcactgcctgcgatctggtcaatgtggatttggatgactgcatctttgaacaataaatgatttaaatcaggtatgtcttttgttgatcaccctccagattggttggaagaagttggtgaaggtcttcgcgagtttttgggccttgaagcgggcccaccgaaaccaaaacccaatcagcagcatcaagatcaagcccgtggtcttgtgctgcctggttataactatctcggacccggaaacggtctcgatcgaggagagcctgtcaacagggcagacgaggtcgcgcgagagcacgacatctcgtacaacgagcagcttgaggcgggagacaacccctacctcaagtacaaccacgcggacgccgagtttcaggagaagctcgccgacgacacatccttcgggggaaacctcggaaaggcagtctttcaggccaagaaaagggttctcgaaccttttggcctggttgaagagggtgctaagacggcccctaccggaaagcggatagacgaccactttccaaaaagaaagaaggctcggaccgaagaggactccaagccttccacctcgtcagacgccgaagctggacccagcggatcccagcagctgcaaatcccagcccaaccagcctcaagtttgggagctgatacaatgtctgcgggaggtggcggcccattgggcgacaataaccaaggtgccgatggagtgggcaatgcctcgggagattggcattgcgattccacgtggatgggggacagagtcgtcaccaagtccacccgaacctgggtgctgcccagctacaacaaccaccagtaccgagagatcaaaagcggctccgtcgacggaagcaacgccaacgcctactttggatacagcaccccctgggggtactttgactttaaccgcttccacagccactggagcccccgagactggcaaagactcatcaacaactactggggcttcagaccccggtccctcagagtcaaaatcttcaacattcaagtcaaagaggtcacggtgcaggactccaccaccaccatcgccaacaacctcacctccaccgtccaagtgtttacggacgacgactaccagctgccctacgtcgtcggcaacgggaccgagggatgcctgccggccttccctccgcaggtctttacgctgccgcagtacggttacgcgacgctgaaccgcgacaacacagaaaatcccaccgagaggagcagcttcttctgcctagagtactttcccagcaagatgctgagaacgggcaacaactttgagtttacctacaactttgaggaggtgcccttccactccagcttcgctcccagtcagaacctgttcaagctggccaacccgctggtggaccagtacttgtaccgcttcgtgagcacaaataacactggcggagtccagttcaacaagaacctggccgggagatacgccaacacctacaaaaactggttcccggggcccatgggccgaacccagggctggaacctgggctccggggtcaaccgcgccagtgtcagcgccttcgccacgaccaataggatggagctcgagggcgcgagttaccaggtgcccccgcagccgaacggcatgaccaacaacctccagggcagcaacacctatgccctggagaacactatgatcttcaacagccagccggcgaacccgggcaccaccgccacgtacctcgagggcaacatgctcatcaccagcgagagcgagacgcagccggtgaaccgcgtggcgtacaacgtcggcgggcagatggccaccaacaaccagagctccaccactgcccccgcgaccggcacgtacaacctccaggaaatcgtgcccggcagcgtgtggatggagagggacgtgtacctccaaggacccatctgggccaagatcccagagacgggggcgcactttcacccctctccggccatgggcggattcggactcaaacacccaccgcccatgatgctcatcaagaacacgcctgtgcccggaaatatcaccagcttctcggacgtgcccgtcagcagcttcatcacccagtacagcaccgggcaggtcaccgtggagatggagtgggagctcaagaaggaaaactccaagaggtggaacccagagatccagtacacaaacaactacaacgacccccagtttgtggactttgccccggacagcaccggggaatacagaaccaccagacctatcggaacccgataccttacccgacccctttaattgcttgttaatcaataaaccgtttaattcgtttcagttgaactttggtctctgcgtatttctttcttatctagtttccatggctacgtagataagtagcatggcgggttaatcattaactacagcccgggcgtttaaacagcgggcggaggggtggagtcgtgacgtgaattacgtcatagggttagggaggtcctgtattagaggtcacgtgagtgttttgcgacattttgcgacaccatgtggtctcgctgggggggggggcccgagtgagcacgcagggtctccattttgaagcgggaggtttgaacgagcgctggcgcgctcactggccgtcgttttac

SEQ ID NO: 40 - DNA, 11589 bp, Artificial Sequence
  plasmid
tgtacactactagggacaggattggtgacagaaaagccccatccttaggcctcctccttcctagtctcctgatattgggtctaacccccacctcctgttaggcagattccttatctggtgacacacccccatttcctggagccatctctctccttgccagaacctctaaggtttgcttacgatggagccagagaggatcctgggagggagagcttggcagggggtgggagggaagggggggatgcgtgacctgcccggttctcagtggccaccctgcgctaccctctcccagaacctgagctgctctgacgcggctgtctggtgcgtttcactgatcctggtgctgcagcttccttacacttcccaagaggagaagcagtttggaaaaacaaaatcagaataagttggtcctgagttctaactttggctcttcacctttctagtccccaatttatattgttcctccgtgcgtcagttttacctgtgagataaggccagtagccagccccgtcctggcagggctgtggtgaggaggggggtgtccgtgtggaaaactccctttgtgagaatggtgcgtcctaggtgttcaccaggtcgtggccgcctctactccctttctctttctccatccttctttccttaaagagtccccagtgctatctgggacatattcctccgcccagagcagggtcccgcttccctaaggccctgctctgggcttctgggtttgagtccttggcaagcccaggagaggcgctcaggcttccctgtcccccttcctcgtccaccatctcatgcccctggctctcctgccccttccctacaggggttcctggctctgctctctcgagatgcatgcgtcaattttacgcagactatctttctagggttaatctagctgcatcaggatcatatcgtcgggtcttttttccggctcagtcatcgcccaagctggcgctatctgggcatcggggaggaagaagcccgtgccttttcccgcgaggttgaagcggcatggaaagagtttgccgaggatgactgctgctgcattgacgttgagcgaaaacgcacgtttaccatgatgattcgggaaggtgtggccatgcacgcctttaacggtgaactgttcgttcaggccacctgggataccagttcgtcgcggcttttccggacacagttccggatggtcagcccgaagcgcatcagcaacccgaacaataccggcgacagccggaactgccgtgccggtgtgcagattaatgacagcggtgcggcgctgggatattacgtcagcgaggacgggtatcctggctggatgccgcagaaatggacatggataccccgtgagttacccggcgggcgcgcttggcgtaatcatggtcatagctgtttcctgtgtgaaattgttatccgctcacaattccacacaacatacgagccggaagcataaagtgtaaagcctggggtgcctaatgagtgagctaactcacattaattgcgttgcgctcactgcccgctttccagtcgggaaacctgtcgtgccagctgcattaatgaatcggccaacgcgcggggagaggcggtttgcgtattgggcgctcttccgcttcctcgctcactgactcgctgcgctcggtcgttcggctgcggcgagcggtatcagctcactcaaaggcggtaatacggttatccacagaatcaggggataacgcaggaaagaacatgtgagcaaaaggccagcaaaaggccaggaaccgtaaaaaggccgcgttgctggcgtttttccataggctccgcccccctgacgagcatcacaaaaatcgacgctcaagtcagaggtggcgaaacccgacaggactataaagataccaggcgtttccccctggaagctccctcgtgcgctctcctgttccgaccctgccgcttaccggatacctgtccgcctttctcccttcgggaagcgtggcgctttctcatagctcacgctgtaggtatctcagttcggtgtaggtcgttcgctccaagctgggctgtgtgcacgaaccccccgttcagcccgaccgctgcgccttatccggtaactatcgtcttgagtccaacccggtaagacacgacttatcgccactggcagcagccactggtaacaggattagcagagcgaggtatgtaggcggtgctacagagttcttgaagtggtggcctaactacggctacactagaaggacagtatttggtatctgcgctctgctgaagccagttaccttcggaaaaagagttggtagctcttgatccggcaaacaaaccaccgctggtagcggtggtttttttgtttgcaagcagcagattacgcgcagaaaaaaaggatctcaagaagatcctttgatcttttctacggggtctgacgctcagtggaacgaaaactcacgttaagggattttggtcatgagattatcaaaaaggatcttcacctagatccttttaaattaaaaatgaagttttaaatcaatctaaagtatatatgagtaaacttggtctgacagttaccaatgcttaatcagtgaggcacctatctcagcgatctgtctatttcgttcatccatagttgcctgactccccgtcgtgtagataactacgatacgggagggcttaccatctggccccagtgctgcaatgataccgcgagacccacgctcaccggctccagatttatcagcaataaaccagccagccggaagggccgagcgcagaagtggtcctgcaactttatccgcctccatccagtctattaattgttgccgggaagctagagtaagtagttcgccagttaatagtttgcgcaacgttgttgccattgctacaggcatcgtggtgtcacgctcgtcgtttggtatggcttcattcagctccggttcccaacgatcaaggcgagttacatgatcccccatgttgtgcaaaaaagcggttagctccttcggtcctccgatcgttgtcagaagtaagttggccgcagtgttatcactcatggttatggcagcactgcataattctcttactgtcatgccatccgtaagatgcttttctgtgactggtgagtactcaaccaagtcattctgagaatagtgtatgcggcgaccgagttgctcttgcccggcgtcaatacgggataataccgcgccacatagcagaactttaaaagtgctcatcattggaaaacgttcttcggggcgaaaactctcaaggatcttaccgctgttgagatccagttcgatgtaacccactcgtgcacccaactgatcttcagcatcttttactttcaccagcgtttctgggtgagcaaaaacaggaaggcaaaatgccgcaaaaaagggaataagggcgacacggaaatgttgaatactcatactcttcctttttcaatattattgaagcatttatcagggttattgtctcatgagcggatacatatttgaatgtatttagaaaaataaacaaataggggttccgcgcacatttccccgaaaagtgccacctaaattgtaagcgttaatattttgttaaaattcgcgttaaatttttgttaaatcagctcattttttaaccaataggccgaaatcggcaaaatcccttataaatcaaaagaatagaccgagatagggttgagtgttgttccagtttggaacaagagtccactattaaagaacgtggactccaacgtcaaagggcgaaaaaccgtctatcagggcgatggcccactacgtgaaccatcaccctaatcaagttttttggggtcgaggtgccgtaaagcactaaatcggaaccctaaagggagcccccgatttagagcttgacggggaaagccggcgaacgtggcgagaaaggaagggaagaaagcgaaaggagcgggcgctagggcgctggcaagtgtagcggtcacgctgcgcgtaaccaccacacccgccgcgcttaatgcgccgctacagggcgcgtcccattcgccattcaggctgcgcaactgttgggaagggcgatcggtgcgggcctcttcgctattacgccagctggcgaaagggggatgtgctgcaaggcgattaagttgggtaacgccagggttttcccagtcacgacgttgtaaaacgacggccagtgagcgcgcctcgttcattcacgtttttgaacccgtggaggacgggcagactcgcggtgcaaatgtgttttacagcgtgatggagcagatgaagatgctcgacacgctgcagaacacgcagctagattaaccctagaaagataatcatattgtgacgtacgttaaagataatcatgcgtaaaattgacgcatgtgttttatcggtctgtatatcgaggtttatttattaatttgaatagatattaagttttattatatttacacttacatactaataataaattcaacaaacaatttatttatgtttatttatttattaaaaaaaaacaaaaactcaaaatttcttctataaagtaacaaaacttttatgagggacagcccccccccaaagcccccagggatgtaattacgtccctcccccgctagggggcagcagcgagccgcccggggctccgctccggtccggcgctccccccgcatccccgagccggcagcgtgcggggacagcccgggcacggggaaggtggcacgggatcgctttcctctgaacgcttctcgctgctctttgagcctgcagacacctggggggatacggggaaaaggcctccaaggcctactagtaacggccgccagtgtgctggaattcgcccttggtacctgctttctctgaccagcattctctcccctgggcctgtgccgctttctgtctgcagcttgtggcctgggtcacctctacggctggcccagatccttccctgccgcctccttcaggttccgtcttcctccactccctcttccccttgctctctgctgtgttgctgcccaaggatgctctttccggagcacttccttctcggcgctgcaccacgtgatgtcctctgagcggatcctccccgtgtctgggtcctctccgggcatctctcctccctcacccaaccccatgccgtcttcactcgctgggttcccttttccttctccttctggggcctgtgccatctctcgtttcttaggatggccttctccgacggatgtctcccttgcgtcccgcctccccttcttgtaggcctgcatcatcaccgtttttctggacaaccccaaagtaccccgtctccctggctttagccacctctccatcctcttgctttctttgcctggacaccccgttctcctgtggattcgggtcacctctcactcctttcatttgggcagctcccctaccccccttacctctctagtctgtgctagctcttccagccccctgtcatggcatcttccaggggtccgagagctcagctagtcttcttcctccaacccgggcccctatgtccacttcaggacagcatgtttgctgcctccagggatcctgtgtccccgagctgggaccaccttatattcccagggccggttaatgtggctctggttctgggtacttttatctgtcccctccaccccacagtggggcacgcgtaagggcgaattctgcagatatccatcacactggcggccgctcgagcatgcatctagtattatgcccagtacatgaccttatgggactttcctacttggcagtacatctacgtattagtcatcgctattaccatggtgatgcggttttggcagtacatcaatgggcgtggatagcggtttgactcacggggatttccaagtctccaccccattgacgtcaatgggagtttgttttggcaccaaaatcaacgggactttccaaaatgtcgtaacaactccgccccattgacgcaaatgggcggtaggcgtgtacggtgggaggtctatataagcagagctcgtttagtgaaccgtcagatcgcctggagacgccatccacgctgttttgacctccatagaagattctagaatggcccttagtaagcacggcctgactaaggacatgaccatgaagtaccatatggagggctcggtggacgggcacaagttcgtgattacgggccacgggaacggcaacccattcgaggggaaacagacaatgaacctgtgtgtggtggaaggcggacccctgcccttctcggaggacatcctgtccgcaacctttgactacggcaatcgcgtgttcacagagtatccacagggtatggtggatttctttaagaacagctgtcccgcaggatacacctggcaccgcagcctgctcttcgaggacggggcggtgtgtaccacctccgctgatatcaccgtgtccgtcgaggagaactgcttctaccacaacagcaaattccacggcgtgaactttcctgccgacgggcctgtgatgaagaaaatgactacgaattgggagcccagctgcgagaaaatcatcccggtccctcgtcagggaatcttgaagggcgacatcgcaatgtacctcctgctcaaggacgggggaagataccgatgccagttcgataccatctacaaggcaaagtccgatcccaaggagatgccagagtggcacttcatccagcacaaactcacccgcgaggaccgctcagatgccaagaaccagaagtggcaactggtcgagcacgccgtggcatcccgtagcgccctgccagggtaattcgaatttaaatcggatccctgtgccttctagttgccagccatctgttgtttgcccctcccccgtgccttccttgaccctggaaggtgccactcccactgtcctttcctaataaaatgaggaaattgcatcgcattgtctgagtaggtgtcattctattctggggggtggggtggggcaggacagcaagggggaggattgggaagacaatagcaggcatgctggggatgcggtgggctctatggagatctgtttaaacaccggtgcgatcgcggcgcgcccctcagcatcgatggaggggtggagtcgtgacgtgaattacgtcatagggttagggaggtcctgtattagaggtcacgtgagtgttttgcgacattttgcgacaccatgtggtcacgctgggtatttaagcccgagtgagcacgcagggtctccattttgaagcgggaggtttgaacgcgcagccgccatgccggggttttacgagattgtgattaaggtccccagcgaccttgacgagcatctgcccggcatttctgacagctttgtgaactgggtggccgagaaggaatgggagttgccgccagattctgacatggatctgaatctgattgagcaggcacccctgaccgtggccgagaagctgcagcgcgactttctgacggaatggcgccgtgtgagtaaggccccggaggcccttttctttgtgcaatttgagaagggagagagctacttccacatgcacgtgctcgtggaaaccaccggggtgaaatccatggttttgggacgtttcctgagtcagattcgcgaaaaactgattcagagaatttaccgcgggatcgagccgactttgccaaactggttcgcggtcacaaagaccagaaatggcgccggaggcgggaacaaggtggtggatgagtgctacatccccaattacttgctccccaaaacccagcctgagctccagtgggcgtggactaatatggaacagtatttaagcgcctgtttgaatctcacggagcgtaaacggttggtggcgcagcatctgacgcacgtgtcgcagacgcaggagcagaacaaagagaatcagaatcccaattctgatgcgccggtgatcagatcaaaaacttcagccaggtacatggagctggtcgggtggctcgtggacaaggggattacctcggagaagcagtggatccaggaggaccaggcctcatacatctccttcaatgcggcctccaactcgcggtcccaaatcaaggctgccttggacaatgcgggaaagattatgagcctgactaaaaccgcccccgactacctggtgggccagcagcccgtggaggacatttccagcaatcggatttataaaattttggaactaaacgggtacgatccccaatatgcggcttccgtctttctgggatgggccacgaaaaagttcggcaagaggaacaccatctggctgtttgggcctgcaactaccgggaagaccaacatcgcggaggccatagcccacactgtgcccttctacgggtgcgtaaactggaccaatgagaactttcccttcaacgactgtgtcgacaagatggtgatctggtgggaggaggggaagatgaccgccaaggtcgtggagtcggccaaagccattctcggaggaagcaaggtgcgcgtggaccagaaatgcaagtcctcggcccagatagacccgactcccgtgatcgtcacctccaacaccaacatgtgcgccgtgattgacgggaactcaacgaccttcgaacaccagcagccgttgcaagaccggatgttcaaatttgaactcacccgccgtctggatcatgactttgggaaggtcaccaagcaggaagtcaaagactttttccggtgggcaaaggatcacgtggttgaggtggagcatgaattctacgtcaaaaagggtggagccaagaaaagacccgcccccagtgacgcagatataagtgagcccaaacgggtgcgcgagtcagttgcgcagccatcgacgtcagacgcggaagcttcgatcaactacgcagacaggtaccaaaacaaatgttctcgtcacgtgggcatgaatctgatgctgtttccctgcagacaatgcgagagaatgaatcagaattcaaatatctgcttcactcacggacagaaagactgtttagagtgctttcccgtgtcagaatctcaacccgtttctgtcgtcaaaaaggcgtatcagaaactgtgctacattcatcatatcatgggaaaggtgccagacgcttgcactgcctgcgatctggtcaatgtggatttggatgactgcatctttgaacaataaatgatttaaatcaggtatgtcttttgttgatcaccctccagattggttggaagaagttggtgaaggtcttcgcgagtttttgggccttgaagcgggcccaccgaaaccaaaacccaatcagcagcatcaagatcaagcccgtggtcttgtgctgcctggttataactatctcggacccggaaacggtctcgatcgaggagagcctgtcaacagggcagacgaggtcgcgcgagagcacgacatctcgtacaacgagcagcttgaggcgggagacaacccctacctcaagtacaaccacgcggacgccgagtttcaggagaagctcgccgacgacacatccttcgggggaaacctcggaaaggcagtctttcaggccaagaaaagggttctcgaaccttttggcctggttgaagagggtgctaagacggcccctaccggaaagcggatagacgaccactttccaaaaagaaagaaggctcggaccgaagaggactccaagccttccacctcgtcagacgccgaagctggacccagcggatcccagcagctgcaaatcccagcccaaccagcctcaagtttgggagctgatacaatgtctgcgggaggtggcggcccattgggcgacaataaccaaggtgccgatggagtgggcaatgcctcgggagattggcattgcgattccacgtggatgggggacagagtcgtcaccaagtccacccgaacctgggtgctgcccagctacaacaaccaccagtaccgagagatcaaaagcggctccgtcgacggaagcaacgccaacgcctactttggatacagcaccccctgggggtactttgactttaaccgcttccacagccactggagcccccgagactggcaaagactcatcaacaactactggggcttcagaccccggtccctcagagtcaaaatcttcaacattcaagtcaaagaggtcacggtgcaggactccaccaccaccatcgccaacaacctcacctccaccgtccaagtgtttacggacgacgactaccagctgccctacgtcgtcggcaacgggaccgagggatgcctgccggccttccctccgcaggtctttacgctgccgcagtacggttacgcgacgctgaaccgcgacaacacagaaaatcccaccgagaggagcagcttcttctgcctagagtactttcccagcaagatgctgagaacgggcaacaactttgagtttacctacaactttgaggaggtgcccttccactccagcttcgctcccagtcagaacctgttcaagctggccaacccgctggtggaccagtacttgtaccgcttcgtgagcacaaataacactggcggagtccagttcaacaagaacctggccgggagatacgccaacacctacaaaaactggttcccggggcccatgggccgaacccagggctggaacctgggctccggggtcaaccgcgccagtgtcagcgccttcgccacgaccaataggatggagctcgagggcgcgagttaccaggtgcccccgcagccgaacggcatgaccaacaacctccagggcagcaacacctatgccctggagaacactatgatcttcaacagccagccggcgaacccgggcaccaccgccacgtacctcgagggcaacatgctcatcaccagcgagagcgagacgcagccggtgaaccgcgtggcgtacaacgtcggcgggcagatggccaccaacaaccagagctccaccactgcccccgcgaccggcacgtacaacctccaggaaatcgtgcccggcagcgtgtggatggagagggacgtgtacctccaaggacccatctgggccaagatcccagagacgggggcgcactttcacccctctccggccatgggcggattcggactcaaacacccaccgcccatgatgctcatcaagaacacgcctgtgcccggaaatatcaccagcttctcggacgtgcccgtcagcagcttcatcacccagtacagcaccgggcaggtcaccgtggagatggagtgggagctcaagaaggaaaactccaagaggtggaacccagagatccagtacacaaacaactacaacgacccccagtttgtggactttgccccggacagcaccggggaatacagaaccaccagacctatcggaacccgataccttacccgacccctttaattgcttgttaatcaataaaccgtttaattcgtttcagttgaactttggtctctgcgtatttctttcttatctagtttccatggctacgtagataagtagcatggcgggttaatcattaactacagcccgggcgtttaaacagcgggcggaggggtggagtcgtgacgtgaattacgtcatagggttagggaggtcctgtattagaggtcacgtgagtgttttgcgacattttgcgacaccatgtggtctcgctgggggggggggcccgagtgagcacgcagggtctccattttgaagcgggaggtttgaacgagcgctggcgcgctcactggccgtcgttttac

SEQ ID NO: 41 - DNA, 12308 bp, Artificial Sequence
  plasmid
tcgcgcgtttcggtgatgacggtgaaaacctctgacacatgcagctcccggagactgtcacagcttgtctgtaagcggatgccgggagcagacaagcccgtcagggcgcgtcagcgggtgttggcgggtgtcggggctggcttaactatgcggcatcagagcagattgtactgagagtgcaccatatgcggtgtgaaataccgcacagatgcgtaaggagaaaataccgcatcaggcgccattcgccattcaggctgcgcaactgttgggaagggcgatcggtgcgggcctcttcgctattacgccagctggcgaaagggggatgtgctgcaaggcgattaagttgggtaacgccagggttttcccagtcacgacgttgtaaaacgacggccagtgaattgacgcgtattgggatgaaacaccgtcttctttaaccctagaaagatagtctgcgtaaaattgacgcatgcattcttgaaatattgctctctctttctaaatagcgcgaatccgtcgctgtgcatttaggacatctcagtcgccgcttggagctcccgtgaggcgtgcttgtcaatgcggtaagtgtcactgattttgaactataacgaccgcgtgagtcaaaatgacgcatgattatcttttacgtgacttttaagatttaactcatacgataattatattgttatttcatgttctacttacgtgataacttattatatatatattttcttgttatagatagcggccgcggctccgccccgggttcccaccgcctgaagggcgagacaagcccgacctgctacaggcactcgtgggggtgggggaggagcgggggtcggtccggctggtttgtgggtgggaggcgcttgttctccaaaaaccggcgcgagctgcaatcctgagggagctgcggtggaggaggtggagagaaggccgcacccttctgggcagggggaggggagtgccgcaatacctttatgggagttctctgctgcctcccgtcttgtaaggaccgccctgggcctggaagaagccctccctcctttcctcctcgcgtgatctcgtcatcgcctccatgtcgagtcgcttctcgaataacttcgtatagcatacattatacgaagttatactagcaggaaacagctatgaccatgattacgaattgcctgcaggcagctgcgcgctcgctcgctcactgaggccgcccgggcaaagcccgggcgtcgggcgacctttggtcgcccggcctcagtgagcgagcgagcgcgcagagagggagtggccaactccatcactaggggttcctatcgatatcaagctttaatagtaatcaattacggggtcattagttcatagcccatatatggagttccgcgttacataacttacggtaaatggcccgcctggctgaccgcccaacgacccccgcccattgacgtcaataatgacgtatgttcccatagtaacgccaatagggactttccattgacgtcaatgggtggagtatttacggtaaactgcccacttggcagtacatcaagtgtatcatatgccaagtacgccccctattgacgtcaatgacggtaaatggcccgcctggcattatgcccagtacatgaccttatgggactttcctacttggcagtacatctacgtattagtcatcgctattaccatggtgatgcggttttggcagtacatcaatgggcgtggatagcggtttgactcacggggatttccaagtctccaccccattgacgtcaatgggagtttgttttggcaccaaaatcaacgggactttccaaaatgtcgtaacaactccgccccattgacgcaaatgggcggtaggcgtgtacggtgggaggtctatataagcagagctggtttagtggatatccttaagggcccagccggcctcgcgagaattctctagcaagctgtgaccggcgcctacgctagacgccaccatggagagcgacgagagcggcctgcccgccatggagatcgagtgccgcatcaccggcaccctgaacggcgtggagttcgagctggtgggcggcggagagggcacccccaagcagggccgcatgaccaacaagatgaagagcaccaaaggcgccctgaccttcagcccctacctgctgagccacgtgatgggctacggcttctaccacttcggcacctaccccagcggctacgagaaccccttcctgcacgccatcaacaacggcggctacaccaacacccgcatcgagaagtacgaggacggcggcgtgctgcacgtgagcttcagctaccgctacgaggccggccgcgtgatcggcgacttcaaggtggtgggcaccggcttccccgaggacagcgtgatcttcaccgacaagatcatccgcagcaacgccaccgtggagcacctgcaccccatgggcgataacgtgctggtgggcagcttcgcccgcaccttcagcctgcgcgacggcggctactacagcttcgtggtggacagccacatgcacttcaagagcgccatccaccccagcatcctgcagaacgggggccccatgttcgccttccgccgcgtggaggagctgcacagcaacaccgagctgggcatcgtggagtaccagcacgccttcaagacccccatcgccttcgccagatcccgcgctcagtcgtccaattctgccgtggacggcaccgccggacccggctccaccggatctcgcgagggcagaggaagtcttctaacatgcggtgacgtggaggagaatcccggccctatgaccgagtacaagcccacggtgcgcctcgccacccgcgacgacgtccccagggccgtacgcaccctcgccgccgcgttcgccgactaccccgccacgcgccacaccgtcgatccggaccgccacatcgagcgggtcaccgagctgcaagaactcttcctcacgcgcgtcgggctcgacatcggcaaggtgtgggtcgcggacgacggcgccgcggtggcggtctggaccacgccggagagcgtcgaagcgggggcggtgttcgccgagatcggcccgcgcatggccgagttgagcggttcccggctggccgcgcagcaacagatggaaggcctcctggcgccgcaccggcccaaggagcccgcgtggttcctggccaccgtcggcgtctcgcccgaccaccagggcaagggtctgggcagcgccgtcgtgctccccggagtggaggcggccgagcgcgccggggtgcccgccttcctggagacctccgcgccccgcaacctccccttctacgagcggctcggcttcaccgtcaccgccgacgtcgaggtgcccgaaggaccgcgcacctggtgcatgacccgcaagcccggtgcctgaaatcaacctctggattacaaaatttgtgaaagattgactggtattcttaactatgttgctccttttacgctatgtggatacgctgctttaatgcctttgtatcagttgatccacgggtggcatccctgtgacccctccccagtgcctctcctggccctggaagttgccactccagtgcccaccagccttgtcctaataaaattaagttgcatcattttgtctgactaggtgtccttctataatattatggggtggaggggggtggtatggagcaaggggcaagttgggaagacaacctgtagggcctgcggggtctattgggaaccaagctggagtgcagtggcacaatcttggctcactgcaatctccgcctcctgggttcaagcgattctcctgcctcagcctcccgagttgttgggattccaggcatgcatgaccaggctcagctaatttttgtttttttggtagagacggggtttcaccatattggccaggctggtctccaactcctaatctcaggtgatctacccaccttggcctcccaaattgctgggattacaggcgtgaaccactgctcccttccctgtccttatcgatagatctaggaacccctagtgatggagttggccactccctctctgcgcgctcgctcgctcactgaggccgggcgaccaaaggtcgcccgacgcccgggctttgcccgggcggcctcagtgagcgagcgagcgcgcagctgcctgcaggcagcttggcactggccgtcgttttactcgacaagcttataacttcgtataggatactttatacgaagttatgcccgggcgaccgcaccctgtgacgaaagccgcccgcaagctgcgcccctgagttagtcatctgaacttcggcctgggcgtctctgggaagtaccacagtggtgggagcgggactttcctggtacaccagggcagcgggccaactacggggattaaggttattacgaggtgtggtggtaatagccgcctgttcgaggagaattcggtttcggtgggcgcggattccgttgacccgggatatcatgtggggtcccgcgctcatgtagtttattcgggttgagtagtcttgggcagctccagccgcaagtcccatttgtggctggtaactccacatgtagggcgtgggaatttccttgctcataatggcgctgacgacaggtgctggcgccgggtgtggccgctggagatgacgtagttttcgcgcttaaatttgagaaagggcgcgaaactagtccttaagagtcagcgcgcagtatttgctgaagagagcctccgcgtcttccagcgtgcgccgaagctgatcttcgcttttgtgatacaggcagctgcgggtgagggagcgcagagacctgttttttattttcagctcttgttcttggcccctgctttgttgaaatatagcatacagagtgggaaaaatcctatttctaagctcgcgggtcgatacgggttcgttgggcgccagacgcagcgctcctcctcctgctgctgccgccgctgtggatttcttgggctttgtcagagtcttgctatccggtcgcctttgcttctgtgtgaccgctgctgttgctgccgctgccgctgccgccggtgcagtaggggctgtagagatgacggtagtaatgcaggatgttacgggggaaggccacgccgtgatggtagagaagaaagcggcgggcgaaggagatgttgcccccacagtcttgcaagcaagcaactatggcgttcttgtgcccgcgccacgagcggtagccttggcgctgttgttgctcttgggctaacggcggcggctgcttagacttaccggccctggttccagtggtgtcccatctacggttgggtcggcgaacaggcagtgccggcggcgcctgaggagcggaggttgtagcgatgctgggaacggttgccaatttctggggcgccggcgaggggaatgcgaccgagggtgacggtgtttcgtctgacacctcttcggcctcggaagcttcgtctaggctgtcccagtcttccatcatctcctcctcctcgtccaaaacctcctctgcctgactgtcccagtattcctcctcgtccgtgggtggcggcggcggcagctgcagcttctttttgggtgccatcctgggaagcaagggcccgcggctgctgatagggctgcggcggcggggggattgggttgagctcctcgccggactgggggtccaggtaaaccccccgtccctttcgtagcagaaactcttggcgggctttgttgatggcttgcaattggccaaggatgtggccctgggtaatgacgcaggcggtaagctccgcatttggcgggcgggattggtcttcgtagaacctaatctcgtgggcgtggtagtcctcaggtacaaatttgcgaaggtaagccgacgtccacagccccggagtgagtttcaaccccggagccgcggacttttcgtcaggcgagggaccctgcagctcaaaggtaccgataatttgactttcgctaagcagttgcgaattgcagaccagggagcggtgcggggtgcataggttgcagcgacagtgacactccagtaggccgtcaccgctcacgtcttccatgatgtcggagtggtaggcaaggtagttggctagctgcagaaggtagcagtgaccccaaagcggcggagggcattcacggtacttaatgggcacaaagtcgctaggaagcgcacagcaggtggcgggcagaattcctgaacgctctaggataaagttcctaaagttttgcaacatgctttgactggtgaagtctggcagaccctgttgcagggttttaagcaggcgttcggggaagataatgtccgccaggtgcgcggccacggagcgctcgttgaaggccgtccataggtccttcaagttttgctttagcagcttctgcagctcctttaggttgcgctcctccaggcattgctgccacacgcccatggccgtttgccaggtgtagcacagaaataagtaaacgcagtcgcggacgtagtcgcggcgcgcctcgcccttgagcgtggaatgaagcacgttttgcccgaggcggttttcgtgcaaaattccaaggtaggagaccaggttgcagagctccacgttggaaattttgcaggcctggcgcacgtagccctggcgaaaggtgtagtgcaacgtttcctctagcttgcgctgcatctccgggtcagcaaagaaccgctgcatgcactcaagctccacggtaacaagcactgcggccatcattagcttgcgtcgctcctccaagtcggcaggctcgcgcgtctcaagccagcgcgccagctgctcatcgccaactgcgggtaggccctcctcggtttgttcttgcaagtttgcatccctctccaggggtcgtgcacggcgcacgatcagctcgctcatgactgtgctcataaccttggggggtaggttaagtgccgggtaggcaaagtgggtgacctcgatgctgcgtttcagcacggctaggcgcgcgttgtcaccctcaagttccaccagcactccacagtgactttcattttcgctgttttcttgttgcagagcgtttgccgcgcgtttctcgtcgcgtccaagaccctcaaagatttttggcacttcgtcgagcgaggcgatatcaggtatgacagcgccctgccgcaaggccagctgcttgtccgctcggctgcggttggcacggcaggataggggtatcttgcagttttggaaaaagatgtgataggtggcaagcacctctggcacggcaaatacggggtagaagttgaggcgcgggttgggctcgcatgtgccgttttcttggcgtttggggggtacgcgcggtgagaacaggtggcgttcgtaggcaaggctgacatccgctatggcgaggggcacatcgctgcgctcttgcaacgcgtcgcagataatggcgcactggcgctgcagatgcttcaacagcacgtcgtctcccacatctaggtagtcgccatgcctttggtccccccgcccgacttgttcctcgtttgcctctgcgtcgtcctggtcttgctttttatcctctgttggtactgagcgatcctcgtcgtcttcgcttacaaaacctgggtcctgctcgataatcacttcctcctcctcaagcgggggtgcctcgacggggaaggtggtaggcgcgttggcggcatcggtggaggcggtggtggcgaactcaaagggggcggttaggctgtcctccttctcgactgactccatgatctttttctgcctataggagaaggaaatggccagtcgggaagaggagcagcgcgaaaccacccccgagcgcggacgcggtgcggcgcgacgtccaccaaccatggaggacgtgtcgtccccgtcgccgtcgccgccgcctccccgcgcgcccccaaaaaagcggctgaggcggcgtctcgagtccgaggacgaagaagactcgtcacaagatgcgctggtgccgcgcacacccagcccgcggccatcgacctcgacggcggatttggccattgcgtccaaaaagaaaaagaagcgcccctctcccaagcccgagcgcccgccatccccagaggtgatcgtggacagcgaggaagaaagagaagatgtggcgctacaaatggtgggtttcagcaacccaccggtgctaatcaagcacggcaagggaggtaagcgcacggtgcggcggctgaatgaagacgacccagtggcgcggggtatgcggacgcaagaggaaaaggaagagtccagtgaagcggaaagtgaaagcacggtgataaacccgctgagcctgccgatcgtgtctgcgtgggagaagggcatggaggctgcgcgcgcgttgatggacaagtaccacgtggataacgatctaaaggcaaacttcaagctactgcctgaccaagtggaagctctggcggccgtatgcaagacctggctaaacgaggagcaccgcgggttgcagctgaccttcaccagcaacaagacctttgtgacgatgatggggcgattcctgcaggcgtacctgcagtcgtttgcagaggtaacctacaagcaccacgagcccacgggctgcgcgttgtggctgcaccgctgcgctgagatcgaaggcgagcttaagtgtctacacgggagcattatgataaataaggagcacgtgattgaaatggatgtgacgagcgaaaacgggcagcgcgcgctgaaggagcagtctagcaaggccaagatcgtgaagaaccggtggggccgaaatgtggtgcagatctccaacaccgacgcaaggtgctgcgtgcatgacgcggcctgtccggccaatcagttttccggcaagtcttgcggcatgttcttctctgaaggcgcaaaggctcaggtggcttttaagcagatcaaggctttcatgcaggcgctgtatcctaacgcccagaccgggcacggtcaccttctgatgccactacggtgcgagtgcaactcaaagcctgggcatgcaccctttttgggaaggcagctaccaaagttgactccgttcgccctgagcaacgcggaggacctggacgcggatctgatctccgacaagagcgtgctggccagcgtgcaccacccggcgctgatagtgttccagtgctgcaaccctgtgtatcgcaactcgcgcgcgcagggcggaggccccaactgcgacttcaagatatcggcgcccgacctgctaaacgcgttggtgatggtgcgcagcctgtggagtgaaaacttcaccgagctgccgcggatggttgtgcctgagtttaagtggagcactaaacaccagtatcgcaacgtgtccctgccagtggcgcatagcgatgcgcggcagaacccctttgatttttaaacggcgcagacggcaagggtggggggtaaataatcacccgagagtgtacaaataaaaacatttgcctttattgaaagtgtctcctagtacattatttttacatgtttttcaagtgacaaaaagaagtggcgctcctaatctgcgcactgtggctgcggaagtagggcgagtggcgctccaggaagctgtagagctgttcctggttgcgacgcagggtgggctgtacctggggactgttaagcatggagttgggtaccttatgggcgggattcttttgcctaggcttaaggggctaacttggtccctgggcgttgccctgcaggggagtgagcagctgtaagatttgaggggcgactccgattagtttatcttcccacggactagagttggtgtcgaggttattgtaataagggtggggtagggaaatggagcttagtcattcacctggggctgattttatgcaacgagactgcggattatcactacttatcatttttggagcatttttctagagctagcgtcgacttttgttactttatagaagaaattttgagtttttgtttttttttaataaataaataaacataaataaattgtttgttgaatttattattagtatgtaagtgtaaatataataaaacttaatatctattcaaattaataaataaacctcgatatacagaccgataaaacacatgcgtcaattttacgcatgattatctttaacgtacgtcacaatatgattatctttctagggttaagaagacgttttagatcccaatggcgcgccgagcttggcgtaatcatggtcatagctgtttcctgtgtgaaattgttatccgctcacaattccacacaacatacgagccggaagcataaagtgtaaagcctggggtgcctaatgagtgagctaactcacattaattgcgttgcgctcactgcccgctttccagtcgggaaacctgtcgtgccagctgcattaatgaatcggccaacgcgcggggagaggcggtttgcgtattgggcgctgttccgcttcctcgctcactgactcgctgcgctcggtcgttcggctgcggcgagcggtatcagctcactcaaaggcggtaatacggttatccacagaatcaggggataacgcaggaaagaacatgtgagcaaaaggccagcaaaaggccaggaaccgtaaaaaggccgcgttgctggcgtttttccataggctccgcccccctgacgagcatcacaaaaatcgacgctcaagtcagaggtggcgaaacccgacaggactataaagataccaggcgtttccccctggaagctccctcgtgcgctctcctgttccgaccctgccgcttaccggatacctgtccgcctttctcccttcgggaagcgtggcgctttctcatagctcacgctgtaggtatctcagttcggtgtaggtcgttcgctccaagctgggctgtgtgcacgaaccccccgttcagcccgaccgctgcgccttatccggtaactatcgtcttgagtccaacccggtaagacacgacttatcgccactggcagcagccactggtaacaggattagcagagcgaggtatgtaggcggtgctacagagttcttgaagtggtggcctaactacggctacactagaagaacagtatttggtatctgcgctctgctgaagccagttaccttcggaaaaagagttggtagctcttgatccggcaaacaaaccaccgctggtagcggtggtttttttgtttgcaagcagcagattacgcgcagaaaaaaaggatctcaagaagatcctttgatcttttctacggggtctgacgctcagtggaacgaaaactcacgttaagggattttggtcatgagattatcaaaaaggatcttcacctagatccttttaaattaaaaatgaagttttaaatcaatctaaagtatatatgagtaaacttggtctgacagttaccaatgcttaatcagtgaggcacctatctcagcgatctgtctatttcgttcatccatagttgcctgactccccgtcgtgtagataactacgatacgggagggcttaccatctggccccagtgctgcaatgataccgcgagaaccacgctcaccggctccagatttatcagcaataaaccagccagccggaagggccgagcgcagaagtggtcctgcaactttatccgcctccatccagtctattaattgttgccgggaagctagagtaagtagttcgccagttaatagtttgcgcaacgttgttgccattgctacaggcatcgtggtgtcacgctcgtcgtttggtatggcttcattcagctccggttcccaacgatcaaggcgagttacatgatcccccatgttgtgcaaaaaagcggttagctccttcggtcctccgatcgttgtcagaagtaagttggccgcagtgttatcactcatggttatggcagcactgcataattctcttactgtcatgccatccgtaagatgcttttctgtgactggtgagtactcaaccaagtcattctgagaatagtgtatgcggcgaccgagttgctcttgcccggcgtcaatacgggataataccgcgccacatagcagaactttaaaagtgctcatcattggaaaacgttcttcggggcgaaaactctcaaggatcttaccgctgttgagatccagttcgatgtaacccactcgtgcacccaactgatcttcagcatcttttactttcaccagcgtttctgggtgagcaaaaacaggaaggcaaaatgccgcaaaaaagggaataagggcgacacggaaatgttgaatactcatactcttcctttttcaatattattgaagcatttatcagggttattgtctcatgagcggatacatatttgaatgtatttagaaaaataaacaaataggggttccgcgcacatttccccgaaaagtgccacctgacgtctaagaaaccattattatcatgacattaacctataaaaataggcgtatcacgaggcccttttgtc

SEQ ID NO: 42 - DNA, 5494 bp, Artificial Sequence
  plasmid
tcgcgcgtttcggtgatgacggtgaaaacctctgacacatgcagctcccggagactgtcacagcttgtctgtaagcggatgccgggagcagacaagcccgtcagggcgcgtcagcgggtgttggcgggtgtcggggctggcttaactatgcggcatcagagcagattgtactgagagtgcaccatatgcggtgtgaaataccgcacagatgcgtaaggagaaaataccgcatcaggcgccattcgccattcaggctgcgcaactgttgggaagggcgatcggtgcgggcctcttcgctattacgccagctggcgaaagggggatgtgctgcaaggcgattaagttgggtaacgccagggttttcccagtcacgacgttgtaaaacgacggccagtgaattgacgcgtattgggatcctgcaggtcgttacataacttacggtaaatggcccgcctggctgaccgcccaacgacccccgcccattgacgtcaataatgacgtatgttcccatagtaacgccaatagggactttccattgacgtcaatgggtggagtatttacggtaaactgcccacttggcagtacatcaagtgtatcatatgccaagtacgccccctattgacgtcaatgacggtaaatggcccgcctggcattatgcccagtacatgaccttatgggactttcctacttggcagtacatctacgtattagtcatcgctattaccatggtgatgcggttttggcagtacatcaatgggcgtggatagcggtttgactcacggggatttccaagtctccaccccattgacgtcaatgggagtttgttttggcaccaaaatcaacgggactttccaaaatgtcgtaacaactccgccccattgacgcaaatgggcggtaggcgtgtacggtgggaggtctatataagcagagctcgtttagtgaaccgtcagatcgcctggagacgccatccacgctgttttgacctccatagaagacaccgggaccgatccagcctccggactctagaggatccggtactagaggaactgaaaaaccagaaagttaactggtaagtttagtctttttgtcttttatttcaggtcccggatccggtggtggtgcaaatcaaagaactgctcctcagtggatgttgcctttacttctaggcctgtacggaagtgttacttctgctctaaaagctgcggaattgtacccgcgggcccaccatgtacccatacgatgttccagattacgctcttatggccatggaggcccgaattcggtcgaccatgggtagttctttagacgatgagcatatcctctctgctcttctgcaaagcgatgacgagcttgttggtgaggattctgacagtgaaatatcagatcacgtaagtgaagatgacgtccagagcgatacagaagaagcgtttatagatgaggtacatgaagtgcagccaacgtcaagcggtagtgaaatattagacgaacaaaatgttattgaacaaccaggttcttcattggcttctaacagaatcttgaccttgccacagaggactattagaggtaagaataaacattgttggtcaacttcaaagtccacgaggcgtagccgagtctctgcactgaacattgtcagatctcaaagaggtccgacgcgtatgtgccgcaatatatatgacccacttttatgcttcaaactattttttactgatgagataatttcggaaattgtaaaatggacaaatgctgagatatcattgaaacgtcgggaatctatgacaggtgctacatttcgtgacacgaatgaagatgaaatctatgctttctttggtattctggtaatgacagcagtgagaaaagataaccacatgtccacagatgacctctttgatcgatctttgtcaatggtgtacgtctctgtaatgagtcgtgatcgttttgattttttgatacgatgtcttagaatggatgacaaaagtatacggcccacacttcgagaaaacgatgtatttactcctgttagaaaaatatgggatctctttatccatcagtgcatacaaaattacactccaggggctcatttgaccatagatgaacagttacttggttttagaggacggtgtccgtttaggatgtatatcccaaacaagccaagtaagtatggaataaaaatcctcatgatgtgtgacagtggtacgaagtatatgataaatggaatgccttatttgggaagaggaacacagaccaacggagtaccactcggtgaatactacgtgaaggagttatcaaagcctgtgcacggtagttgtcgtaatattacgtgtgacaattggttcacctcaatccctttggcaaaaaacttactacaagaaccgtataagttaaccattgtgggaaccgtgcgatcaaacaaacgcgagataccggaagtactgaaaaacagtcgctccaggccagtgggaacatcgatgttttgttttgacggaccccttactctcgtctcatataaaccgaagccagctaagatggtatacttattatcatcttgtgatgaggatgcttctatcaacgaaagtaccggtaaaccgcaaatggttatgtattataatcaaactaaaggcggagtggacacgctagaccaaatgtgttctgtgatgacctgcagtaggaagacgaataggtggcctatggcattattgtacggaatgataaacattgcctgcataaattcttttattatatacagccataatgtcagtagcaagggagaaaaggttcaaagtcgcaaaaaatttatgagaaacctttacatgagcctgacgtcatcgtttatgcgtaagcgtttagaagctcctactttgaagagatatttgcgcgataatatctctaatattttgccaaatgaagtgcctggtacatcagatgacagtactgaagagccagtaatgaaaaaacgtacttactgtacttactgcccctctaaaataaggcgaaaggcaaatgcatcgtgcaaaaaatgcaaaaaagttatttgtcgagagcataatattgatatgtgccaaagttgtttctgagagatctctcgaggtaccgcggccgcggggatccagacatgataagatacattgatgagtttggacaaaccacaactagaatgcagtgaaaaaaatgctttatttgtgaaatttgtgatgctattgctttatttgtaaccattataagctgcaataaacaagttatcccaatggcgcgccgagcttggcgtaatcatggtcatagctgtttcctgtgtgaaattgttatccgctcacaattccacacaacatacgagccggaagcataaagtgtaaagcctggggtgcctaatgagtgagctaactcacattaattgcgttgcgctcactgcccgctttccagtcgggaaacctgtcgtgccagctgcattaatgaatcggccaacgcgcggggagaggcggtttgcgtattgggcgctgttccgcttcctcgctcactgactcgctgcgctcggtcgttcggctgcggcgagcggtatcagctcactcaaaggcggtaatacggttatccacagaatcaggggataacgcaggaaagaacatgtgagcaaaaggccagcaaaaggccaggaaccgtaaaaaggccgcgttgctggcgtttttccataggctccgcccccctgacgagcatcacaaaaatcgacgctcaagtcagaggtggcgaaacccgacaggactataaagataccaggcgtttccccctggaagctccctcgtgcgctctcctgttccgaccctgccgcttaccggatacctgtccgcctttctcccttcgggaagcgtggcgctttctcatagctcacgctgtaggtatctcagttcggtgtaggtcgttcgctccaagctgggctgtgtgcacgaaccccccgttcagcccgaccgctgcgccttatccggtaactatcgtcttgagtccaacccggtaagacacgacttatcgccactggcagcagccactggtaacaggattagcagagcgaggtatgtaggcggtgctacagagttcttgaagtggtggcctaactacggctacactagaagaacagtatttggtatctgcgctctgctgaagccagttaccttcggaaaaagagttggtagctcttgatccggcaaacaaaccaccgctggtagcggtggtttttttgtttgcaagcagcagattacgcgcagaaaaaaaggatctcaagaagatcctttgatcttttctacggggtctgacgctcagtggaacgaaaactcacgttaagggattttggtcatgagattatcaaaaaggatcttcacctagatccttttaaattaaaaatgaagttttaaatcaatctaaagtatatatgagtaaacttggtctgacagttaccaatgcttaatcagtgaggcacctatctcagcgatctgtctatttcgttcatccatagttgcctgactccccgtcgtgtagataactacgatacgggagggcttaccatctggccccagtgctgcaatgataccgcgagaaccacgctcaccggctccagatttatcagcaataaaccagccagccggaagggccgagcgcagaagtggtcctgcaactttatccgcctccatccagtctattaattgttgccgggaagctagagtaagtagttcgccagttaatagtttgcgcaacgttgttgccattgctacaggcatcgtggtgtcacgctcgtcgtttggtatggcttcattcagctccggttcccaacgatcaaggcgagttacatgatcccccatgttgtgcaaaaaagcggttagctccttcggtcctccgatcgttgtcagaagtaagttggccgcagtgttatcactcatggttatggcagcactgcataattctcttactgtcatgccatccgtaagatgcttttctgtgactggtgagtactcaaccaagtcattctgagaatagtgtatgcggcgaccgagttgctcttgcccggcgtcaatacgggataataccgcgccacatagcagaactttaaaagtgctcatcattggaaaacgttcttcggggcgaaaactctcaaggatcttaccgctgttgagatccagttcgatgtaacccactcgtgcacccaactgatcttcagcatcttttactttcaccagcgtttctgggtgagcaaaaacaggaaggcaaaatgccgcaaaaaagggaataagggcgacacggaaatgttgaatactcatactcttcctttttcaatattattgaagcatttatcagggttattgtctcatgagcggatacatatttgaatgtatttagaaaaataaacaaataggggttccgcgcacatttccccgaaaagtgccacctgacgtctaagaaaccattattatcatgacattaacctataaaaataggcgtatcacgaggcccttttgtc

SEQ ID NO: 43 - DNA, 23951 bp, Artificial Sequence
  plasmid
atgactctcttaaggtagccaaatttccataggctccgcccccctgacgagcatcacaaaaatcgacgctcaagtcagaggtggcgaaacccgacaggactataaagataccaggcgtttccccctggaagctccctcgtgcgctctcctgttccgaccctgccgcttaccggatacctgtccgcctttctcccttcgggaagcgtggcgctttctcatagctcacgctgtaggtatctcagttcggtgtaggtcgttcgctccaagctgggctgtgtgcacgaaccccccgttcagcccgaccgctgcgccttatccggtaactatcgtcttgagtccaacccggtaagacacgacttatcgccactggcagcagccactggtaacaggattagcagagcgaggtatgtaggcggtgctacagagttcttgaagtggtggcctaactacggctacactagaaggacagtatttggtatctgcgctctgctgaagccagttaccttcggaaaaagagttggtagctcttgatccggcaaacaaaccaccgctggtagcggtggtttttttgtttgcaagcagcagattacgcgcagaaaaaaaggatctcaagaagatcctttgatcttttctacggggtctgacgctcagtggaacgaaaactcacgttaagggattttggtcatgagattatcaaaaaggatcttcacctagatccttttaaattaaaaatgaagttttaaatcaatctaaagtatatatgagtaaacttggtctgacagttaccaatgcttaatcagtgaggcacctatctcagcgatctgtctatttcgttcatccatagttgcctgactccccgtcgtgtagataactacgatacgggagggcttaccatctggccccagtgctgcaatgataccgcgagacccacgctcaccggctccagatttatcagcaataaaccagccagccggaagggccgagcgcagaagtggtcctgcaactttatccgcctccatccagtctattaattgttgccgggaagctagagtaagtagttcgccagttaatagtttgcgcaacgttgttgccattgctacaggcatcgtggtgtcacgctcgtcgtttggtatggcttcattcagctccggttcccaacgatcaaggcgagttacatgatcccccatgttgtgcaaaaaagcggttagctccttcggtcctccgatcgttgtcagaagtaagttggccgcagtgttatcactcatggttatggcagcactgcataattctcttactgtcatgccatccgtaagatgcttttctgtgactggtgagtactcaaccaagtcattctgagaatagtgtatgcggcgaccgagttgctcttgcccggcgtcaatacgggataataccgcgccacatagcagaactttaaaagtgctcatcattggaaaacgttcttcggggcgaaaactctcaaggatcttaccgctgttgagatccagttcgatgtaacccactcgtgcacccaactgatcttcagcatcttttactttcaccagcgtttctgggtgagcaaaaacaggaaggcaaaatgccgcaaaaaagggaataagggcgacacggaaatgttgaatactcatactcttcctttttcaatattattgaagcatttatcagggttattgtctcatgagcggatacatatttgaatgtatttagaaaaataaacaaataggggttccgcgcacatttccccgaaaagtgccacctaaattgtaagcgttaatattttgttaaaattcgcgttaaatttttgttaaatcagctcattttttaaccaataggccgaaatcggcaaaatcccttataaatcaaaagaatagaccgagatagggttgagtgttgttccagtttggaacaagagtccactattaaagaacgtggactccaacgtcaaagggcgaaaaaccgtctatcagggcgatggcccactacgtgaaccatcaccctaatcaagttttttggggtcgaggtgccgtaaagcactaaatcggaaccctaaagggagcccccgatttagagcttgacggggaaagccggcgaacgtggcgagaaaggaagggaagaaagcgaaaggagcgggcgctagggcgctggcaagtgtagcggtcacgctgcgcgtaaccaccacacccgccgcgcttaatgcgccgctacagggcgcgtcccattcgccattcaggctgcgcaactgttgggaagggcgatcggtgcgggcctcttcgctattacgccagctggcgaaagggggatgtgctgcaaggcgattaagttgggtaacgccagggttttcccagtcacgacgttaccccacagtggggccactagggtcaatttctgagaactgtcattctcggaaattgagtaaaacgacggccagtgagcgcgcctcgttcattcacgtttttgaacccgtggaggacgggcagactcgcggtgcaaatgtgttttacagcgtgatggagcagatgaagatgctcgacacgctgcagaacacgcagctagattaaccctagaaagataatcatattgtgacgtacgttaaagataatcatgcgtaaaattgacgcatgtgttttatcggtctgtatatcgaggtttatttattaatttgaatagatattaagttttattatatttacacttacatactaataataaattcaacaaacaatttatttatgtttatttatttattaaaaaaaaacaaaaactcaaaatttcttctataaagtaacaaaacttttatcgaattcctgcagcccgggggatccactagttctagagggacagcccccccccaaagcccccagggatgtaattacgtccctcccccgctagggggcagcagcgagccgcccggggctccgctccggtccggcgctccccccgcatccccgagccggcagcgtgcggggacagcccgggcacggggaaggtggcacgggatcgctttcctctgaacgcttctcgctgctctttgagcctgcagacacctggggggatacggggaaaaggcctccaaggccagcttcccacaataagttgggtgaattttggctcattcctcctttctataggattgaggtcagagctttgtgatgggaattctgtggaatgtgtgtcagttagggtgtggaaagtcccgcgatcgctagcgtttaaacttaagcttggtaccgagctcggatccactagtccagtgtggtggaattcctgcttcgcgatgtacgggccagatatacgcgttgcccgggcgaccgcaccctgtgacgaaagccgcccgcaagctgcgcccctgagttagtcatctgaacttcggcctgggcgtctctgggaagtaccacagtggtgggagcgggactttcctggtacaccagggcagcgggccaactacggggattaaggttattacgaggtgtggtggtaatagccgcctgttcgaggagaattcggtttcggtgggcgcggattccgttgacccgggatatcatgtggggtcccgcgctcatgtagtttattcgggttgagtagtcttgggcagctccagccgcaagtcccatttgtggctggtaactccacatgtagggcgtgggaatttccttgctcataatggcgctgacgacaggtgctggcgccgggtgtggccgctggagatgacgtagttttcgcgcttaaatttgagaaagggcgcgaaactagtccttaagagtcagcgcgcagtatttgctgaagagagcctccgcgtcttccagcgtgcgccgaagctgatcttcgcttttgtgatacaggcagctgcgggtgagggagcgcagagacctgttttttattttcagctcttgttcttggcccctgctttgttgaaatatagcatacagagtgggaaaaatcctatttctaagctcgcgggtcgatacgggttcgttgggcgccagacgcagcgctcctcctcctgctgctgccgccgctgtggatttcttgggctttgtcagagtcttgctatccggtcgcctttgcttctgtgtgaccgctgctgttgctgccgctgccgctgccgccggtgcagtaggggctgtagagatgacggtagtaatgcaggatgttacgggggaaggccacgccgtgatggtagagaagaaagcggcgggcgaaggagatgttgcccccacagtcttgcaagcaagcaactatggcgttcttgtgcccgcgccacgagcggtagccttggcgctgttgttgctcttgggctaacggcggcggctgcttagacttaccggccctggttccagtggtgtcccatctacggttgggtcggcgaacaggcagtgccggcggcgcctgaggagcggaggttgtagcgatgctgggaacggttgccaatttctggggcgccggcgaggggaatgcgaccgagggtgacggtgtttcgtctgacacctcttcggcctcggaagcttcgtctaggctgtcccagtcttccatcatctcctcctcctcgtccaaaacctcctctgcctgactgtcccagtattcctcctcgtccgtgggtggcggcggcggcagctgcagcttctttttgggtgccatcctgggaagcaagggcccgcggctgctgatagggctgcggcggcggggggattgggttgagctcctcgccggactgggggtccaggtaaaccccccgtccctttcgtagcagaaactcttggcgggctttgttgatggcttgcaattggccaaggatgtggccctgggtaatgacgcaggcggtaagctccgcatttggcgggcgggattggtcttcgtagaacctaatctcgtgggcgtggtagtcctcaggtacaaatttgcgaaggtaagccgacgtccacagccccggagtgagtttcaaccccggagccgcggacttttcgtcaggcgagggaccctgcagctcaaaggtaccgataatttgactttcgctaagcagttgcgaattgcagaccagggagcggtgcggggtgcataggttgcagcgacagtgacactccagtaggccgtcaccgctcacgtcttccatgatgtcggagtggtaggcaaggtagttggctagctgcagaaggtagcagtgaccccaaagcggcggagggcattcacggtacttaatgggcacaaagtcgctaggaagcgcacagcaggtggcgggcagaattcctgaacgctctaggataaagttcctaaagttttgcaacatgctttgactggtgaagtctggcagaccctgttgcagggttttaagcaggcgttcggggaagataatgtccgccaggtgcgcggccacggagcgctcgttgaaggccgtccataggtccttcaagttttgctttagcagcttctgcagctcctttaggttgcgctcctccaggcattgctgccacacgcccatggccgtttgccaggtgtagcacagaaataagtaaacgcagtcgcggacgtagtcgcggcgcgcctcgcccttgagcgtggaatgaagcacgttttgcccgaggcggttttcgtgcaaaattccaaggtaggagaccaggttgcagagctccacgttggaaattttgcaggcctggcgcacgtagccctggcgaaaggtgtagtgcaacgtttcctctagcttgcgctgcatctccgggtcagcaaagaaccgctgcatgcactcaagctccacggtaacaagcactgcggccatcattagcttgcgtcgctcctccaagtcggcaggctcgcgcgtctcaagccagcgcgccagctgctcatcgccaactgcgggtaggccctcctcggtttgttcttgcaagtttgcatccctctccaggggtcgtgcacggcgcacgatcagctcgctcatgactgtgctcataaccttggggggtaggttaagtgccgggtaggcaaagtgggtgacctcgatgctgcgtttcagcacggctaggcgcgcgttgtcaccctcaagttccaccagcactccacagtgactttcattttcgctgttttcttgttgcagagcgtttgccgcgcgtttctcgtcgcgtccaagaccctcaaagatttttggcacttcgtcgagcgaggcgatatcaggtatgacagcgccctgccgcaaggccagctgcttgtccgctcggctgcggttggcacggcaggataggggtatcttgcagttttggaaaaagatgtgataggtggcaagcacctctggcacggcaaatacggggtagaagttgaggcgcgggttgggctcgcatgtgccgttttcttggcgtttggggggtacgcgcggtgagaacaggtggcgttcgtaggcaaggctgacatccgctatggcgaggggcacatcgctgcgctcttgcaacgcgtcgcagataatggcgcactggcgctgcagatgcttcaacagcacgtcgtctcccacatctaggtagtcgccatgcctttggtccccccgcccgacttgttcctcgtttgcctctgcgtcgtcctggtcttgctttttatcctctgttggtactgagcgatcctcgtcgtcttcgcttacaaaacctgggtcctgctcgataatcacttcctcctcctcaagcgggggtgcctcgacggggaaggtggtaggcgcgttggcggcatcggtggaggcggtggtggcgaactcaaagggggcggttaggctgtcctccttctcgactgactccatgatctttttctgcctataggagaaggaaatggccagtcgggaagaggagcagcgcgaaaccacccccgagcgcggacgcggtgcggcgcgacgtccaccaaccatggaggacgtgtcgtccccgtcgccgtcgccgccgcctccccgcgcgcccccaaaaaagcggctgaggcggcgtctcgagtccgaggacgaagaagactcgtcacaagatgcgctggtgccgcgcacacccagcccgcggccatcgacctcgacggcggatttggccattgcgtccaaaaagaaaaagaagcgcccctctcccaagcccgagcgcccgccatccccagaggtgatcgtggacagcgaggaagaaagagaagatgtggcgctacaaatggtgggtttcagcaacccaccggtgctaatcaagcacggcaagggaggtaagcgcacggtgcggcggctgaatgaagacgacccagtggcgcggggtatgcggacgcaagaggaaaaggaagagtccagtgaagcggaaagtgaaagcacggtgataaacccgctgagcctgccgatcgtgtctgcgtgggagaagggcatggaggctgcgcgcgcgttgatggacaagtaccacgtggataacgatctaaaggcaaacttcaagctactgcctgaccaagtggaagctctggcggccgtatgcaagacctggctaaacgaggagcaccgcgggttgcagctgaccttcaccagcaacaagacctttgtgacgatgatggggcgattcctgcaggcgtacctgcagtcgtttgcagaggtaacctacaagcaccacgagcccacgggctgcgcgttgtggctgcaccgctgcgctgagatcgaaggcgagcttaagtgtctacacgggagcattatgataaataaggagcacgtgattgaaatggatgtgacgagcgaaaacgggcagcgcgcgctgaaggagcagtctagcaaggccaagatcgtgaagaaccggtggggccgaaatgtggtgcagatctccaacaccgacgcaaggtgctgcgtgcatgacgcggcctgtccggccaatcagttttccggcaagtcttgcggcatgttcttctctgaaggcgcaaaggctcaggtggcttttaagcagatcaaggctttcatgcaggcgctgtatcctaacgcccagaccgggcacggtcaccttctgatgccactacggtgcgagtgcaactcaaagcctgggcatgcaccctttttgggaaggcagctaccaaagttgactccgttcgccctgagcaacgcggaggacctggacgcggatctgatctccgacaagagcgtgctggccagcgtgcaccacccggcgctgatagtgttccagtgctgcaaccctgtgtatcgcaactcgcgcgcgcagggcggaggccccaactgcgacttcaagatatcggcgcccgacctgctaaacgcgttggtgatggtgcgcagcctgtggagtgaaaacttcaccgagctgccgcggatggttgtgcctgagtttaagtggagcactaaacaccagtatcgcaacgtgtccctgccagtggcgcatagcgatgcgcggcagaacccctttgatttttaaacggcgcagacggcaagggtggggggtaaataatcacccgagagtgtacaaataaaaacatttgcctttattgaaagtgtctcctagtacattatttttacatgtttttcaagtgacaaaaagaagtggcgctcctaatctgcgcactgtggctgcggaagtagggcgagtggcgctccaggaagctgtagagctgttcctggttgcgacgcagggtgggctgtacctggggactgttaagcatggagttgggtaccccatagagcccaccgcatcgaggctgatcagcgggtttaaacgggccctctagactcgagcggccgcctacatgggggtagagtcataatcgtgcatcaggatagggcggtggtgctgcagcagcgcgcgaataaactgctgccgccgccgctccgtcctgcaggaatacaacatggcagtggtctcctcagcgatgattcgcaccgcccgcagcatgagacgccttgtcctccgggcacagcagcgcaccctgatctcacttaaatcagcacagtaactgcagcacagcaccacaatattgttcaaaatcccacagtgcaaggcgctgtatccaaagctcatggcggggaccacagaacccacgtggccatcataccacaagcgcaggtagattaagtggcgacccctcataaacacgctggacataaacattacctcttttggcatgttgtaattcaccacctcccggtaccatataaacctctgattaaacatggcgccatccaccaccatcctaaaccagctggccaaaacctgcccgccggctatgcactgcagggaaccgggactggaacaatgacagtggagagcccaggactcgtaaccatggatcatcatgctcgtcatgatatcaatgttggcacaacacaggcacacgtgcatacacttcctcaggattacaagctcctcccgcgtcagaaccatatcccagggaacaacccattcctgaatcagcgtaaatcccacactgcagggaagacctcgcacgtaactcacgttgtgcattgtcaaagtgttacattcgggcagcagcggatgatcctccagtatggtagcgcgggtctctgtctcaaaaggaggtaggcgatccctactgtacggagtgcgccgagacaaccgagatcgtgttggtcgtagtgtcatgccaaatggaacgccggacgtagtcatatttcctcgacgatctctatcactgatagggagatctctatcactgatagggagagctctgcttatatagacctcccaccgtacacgcctaccgcccatttgcgtcaatggggcggagttgttacgacattttggaaagtcccgttgattttggttccaaaacaaactcccattgacgtcaatggggtggagacttggaaatccccgtgagtcaaaccgctatccacgcccattgatgtactgccaaaaccgcatcacatggtgcactctcagtacaatcatccgtattgggatgcggccgcaatatttgcatgtcgctatgtgttctgggaaatcaccataaacgtgaaatccctatcagtgatagagacttataagttccctatcagtgatagagaaccggtgggcactcttccgtggtctggtggataaattcgcaagggtatcatggcggacgaccggggttcgaaccccggatccggccgtccgccgtgatccatgcggttaccgcccgcgtgtcgaacccaggtgtgcgacgtcagacaacgggggagcgctcctttttgaattccactttggccgcggctcgaggacattgattattgactagttattaatagtaatcaattacggggtcattagttcatagcccatatatggagttccgcgttacataacttacggtaaatggcccgcctggctgaccgcccaacgacccccgcccattgacgtcaataatgacgtatgttcccatagtaacgccaatagggactttccattgacgtcaatgggtggagtatttacggtaaactgcccacttggcagtacatcaagtgtatcatatgccaagtacgccccctattgacgtcaatgacggtaaatggcccgcctggcattatgcccagtacatgaccttatgggactttcctacttggcagtacatctacgtattagtcatcgctattaccatggtgatgcggttttggcagtacatcaatgggcgtggatagcggtttgactcacggggatttccaagtctccaccccattgacgtcaatgggagtttgttttggcaccaaaatcaacgggactttccaaaatgtcgtaacaactccgccccattgacgcaaatgggcggtaggcgtgtacggtgggaggtctatataagcagagctcgtttagtgaaccgtcagatcgcctggagacgccatccacgctgttttgacctccatagaagacaccgggaccgatccagcctccgcggccccgaattcaccatgtctagattagataaaagtaaagtgattaacagcgcattagagctgcttaatgaggtcggaatcgaaggtttaacaacccgtaaactcgcccagaagctaggtgtagagcagcctacattgtattggcacgtgcgcaacaagcagactcttatgaacatgctttcagaggcaatactggcgaagcatcacacccgttcagcaccgttaccgactgagagttggcagcagtttctccaggaaaatgctctgagtttccgtaaagcattactggtccatcgtgatggagcccgattgcatatagggacctctcctacgcccccccagtttgaacaagcagaggcgcaactacgctgtctatgcgatgcagggttttcggtcgaggaggctcttttcattctgcaatctatcagccattttacgttgggtgcagtattagaggagcaagcaacaaaccagatagaaaataatcatgtgatagacgctgcaccaccattattacaagaggcatttaatattcaggcgagaacctctgctgaaatggccttccatttcgggctgaaatcattaatatttggattttctgcacagttagatgaaaaaaagcatacacccattgaggatggtaataaaccaaaaaagaagagaaagctagcagtgtcagtgacatttgaagatgtggctgtgctctttactcgggacgagtggaagaagctggatctgtctcagagaagcctgtaccgtgaggtgatgctggagaattacagcaacctggcctccatggcaggattcctgtttaccaaaccaaaggtgatctccctgttgcagcaaggagaggatccctggtaaatcgatctgagaacttcagggtgagtttggggacccttgattgttctttctttttcgctattgtaaaattcatgttatatggagggggcaaagttttcagggtgttgtttagaatgggaagatgtcccttgtatcaccatggaccctcatgataattttgtttctttcactttctactctgttgacaaccattgtctcctcttattttcttttcattttctgtaactttttcgttaaactttagcttgcatttgtaacgaatttttaaattcacttttgtttatttgtcagattgtaagtactttctctaatcacttttttttcaaggcaatcagggtatattatattgtacttcagcacagttttagagaacaattgttataattaaatgataaggtagaatatttctgcatataaattctggctggcgtggaaatattcttattggtagaaacaactacaccctggtcatcatcctgcctttctctttatggttacaatgatatacactgtttgagatgaggataaaatactctgagtccaaaccgggcccctctgctaaccatgttcatgccttcttctctttcctacagctcctgggcaacgtgctggttgttgtgctgtctcatcattttggcaaagaattcactcctcaggtgcaggctgcctatcagaaggtggtggctggtgtggccaatgccctggctcacaaataccactgagatctttttccctctgccaaaaattatggggacatcatgaagccccttgagcatctgacttctggctaataaaggaaatttattttcattgcaatagtgtgttggaattttttgtgtctctcactctagagcggccgcggatccaattctaccgggtaggggaggcgcttttcccaaggcagtctggagcatgcgctttagcagccccgctgggcacttggcgctacacaagtggcctctggcctcgcacacattccacatccaccggtaggcgccaaccggctccgttctttggtggccccttcgcgccaccttctactcctcccctagtcaggaagttcccccccgccccgcagctcgcgtcgtgcaggacgtgacaaatggaagtagcacgtctcactagtctcgtgcagatggacagcaccgctgagcaatggaagcgggtaggcctttggggcagcggccaatagcagctttgctccttcgctttctgggctcagaggctgggaaggggtgggtccgggggcgggctcaggggcgggctcaggggcggggcgggcgcccgaaggtcctccggaggcccggcattctgcacgcttcaaaagcgcacgtctgccgcgctgttctcctcttcctcatctccgggcctttcgacctgcagttaacgccgccatgaccgagtacaagcccacggtgcgcctcgccacccgcgacgacgtccccagggccgtacgcaccctcgccgccgcgttcgccgactaccccgccacgcgccacaccgtcgatccggaccgccacatcgagcgggtcaccgagctgcaagaactcttcctcacgcgcgtcgggctcgacatcggcaaggtgtgggtcgcggacgacggcgccgcggtggcggtctggaccacgccggagagcgtcgaagcgggggcggtgttcgccgagatcggcccgcgcatggccgagttgagcggttcccggctggccgcgcagcaacagatggaaggcctcctggcgccgcaccggcccaaggagcccgcgtggttcctggccaccgtcggcgtctcgcccgaccaccagggcaagggtctgggcagcgccgtcgtgctccccggagtggaggcggccgagcgcgccggggtgcccgccttcctggagacctccgcgccccgcaacctccccttctacgagcggctcggcttcaccgtcaccgccgacgtcgaggtgcccgaaggaccgcgcacctggtgcatgacccgcaagcccggtgcctgaccgcgtctggaacaatcaacctctggattacaaaatttgtgaaagattgactggtattcttaactatgttgctccttttacgctatgtggatacgctgctttaatgcctttgtatcatgctattgcttcccgtatggctttcattttctcctccttgtataaatcctggttgctgtctctttatgaggagttgtggcccgttgtcaggcaacgtggcgtggtgtgcactgtgtttgctgacgcaacccccactggttggggcattgccaccacctgtcagctcctttccgggactttcgctttccccctccctattgccacggcggaactcatcgccgcctgccttgcccgctgctggacaggggctcggctgttgggcactgacaattccgtggtgttgtcggggaagctgacgtcctttccatggctgctcgcctgtgttgccacctggattctgcgcgggacgtccttctgctacgtcccttcggccctcaatccagcggaccttccttcccgcggcctgctgccggctctgcggcctcttccgcgtcttcgccttcgccctcagacgagtcggatctccctttgggccgcctccccgcaaaatgaccgaccaagcgacgcccaacctgccatcacgagatttcgattccaccgccgccttctatgaaaggttgggcttcggaatcgttttccgggacgccggctggatgatcctccagcgcggggatctcatgctggagttcttcgcccaccccaacttgtttattgcagcttataatggttacaaataaagcaatagcatcacaaatttcacaaataaagcatttttttcactgcattctagttgtggtttgtccaaactcatcaatgtatcttatcatgtctgtagctgatcaattggcgcgccgaattcgttatctgcagaattcggcttgagcgcgccagcgctcgttcaaacctcccgcttcaaaatggagaccctgcgtgctcactcgggcccccccccccagcgagaccacatggtgtcgcaaaatgtcgcaaaacactcacgtgacctctaatacaggacctccctaaccctatgacgtaattcacgtcacgactccacccctccgcccgctgtttaaacgcccgggctgtagttaatgattaacccgccatgctacttatctacgtagccatggaaactagataagaaagaaatacgcagagaccaaagttcaactgaaacgaattaaacggtttattgattaacaagcaattaaaggggtcgggtaaggtatcgggttccgataggtctggtggttctgtattccccggtgctgtccggggcaaagtccacaaactgggggtcgttgtagttgtttgtgtactggatctctgggttccacctcttggagttttccttcttgagctcccactccatctccacggtgacctgcccggtgctgtactgggtgatgaagctgctgacgggcacgtccgagaagctggtgatatttccgggcacaggcgtgttcttgatgagcatcatgggcggtgggtgtttgagtccgaatccgcccatggccggagaggggtgaaagtgcgcccccgtctctgggatcttggcccagatgggtccttggaggtacacgtccctctccatccacacgctgccgggcacgatttcctggaggttgtacgtgccggtcgcgggggcagtggtggagctctggttgttggtggccatctgcccgccgacgttgtacgccacgcggttcaccggctgcgtctcgctctcgctggtgatgagcatgttgccctcgaggtacgtggcggtggtgcccgggttcgccggctggctgttgaagatcatagtgttctccagggcataggtgttgctgccctggaggttgttggtcatgccgttcggctgcgggggcacctggtaactcgcgccctcgagctccatcctattggtcgtggcgaaggcgctgacactggcgcggttgaccccggagcccaggttccagccctgggttcggcccatgggccccgggaaccagtttttgtaggtgttggcgtatctcccggccaggttcttgttgaactggactccgccagtgttatttgtgctcacgaagcggtacaagtactggtccaccagcgggttggccagcttgaacaggttctgactgggagcgaagctggagtggaagggcacctcctcaaagttgtaggtaaactcaaagttgttgcccgttctcagcatcttgctgggaaagtactctaggcagaagaagctgctcctctcggtgggattttctgtgttgtcgcggttcagcgtcgcgtaaccgtactgcggcagcgtaaagacctgcggagggaaggccggcaggcatccctcggtcccgttgccgacgacgtagggcagctggtagtcgtcgtccgtaaacacttggacggtggaggtgaggttgttggcgatggtggtggtggagtcctgcaccgtgacctctttgacttgaatgttgaagattttgactctgagggaccggggtctgaagccccagtagttgttgatgagtctttgccagtctcgggggctccagtggctgtggaagcggttaaagtcaaagtacccccagggggtgctgtatccaaagtaggcgttggcgttgcttccgtcgacggagccgcttttgatctctcggtactggtggttgttgtagctgggcagcacccaggttcgggtggacttggtgacgactctgtcccccatccacgtggaatcgcaatgccaatctcccgaggcattgcccactccatcggcaccttggttattgtcgcccaatgggccgccacctcccgcagacattgtatcagctcccaaacttgaggctggttgggctgggatttgcagctgctgggatccgctgggtccagcttcggcgtctgacgaggtggaaggcttggagtcctcttcggtccgagccttctttctttttggaaagtggtcgtctatccgctttccggtaggggccgtcttagcaccctcttcaaccaggccaaaaggttcgagaacccttttcttggcctgaaagactgcctttccgaggtttcccccgaaggatgtgtcgtcggcgagcttctcctgaaactcggcgtccgcgtggttgtacttgaggtaggggttgtctcccgcctcaagctgctcgttgtacgagatgtcgtgctctcgcgcgacctcgtctgccctgttgacaggctctcctcgatcgagaccgtttccgggtccgagatagttataaccaggcagcacaagaccacgggcttgatcttgatgctgctgattgggttttggtttcggtgggcccgcttcaaggcccaaaaactcgcgaagaccttcaccaacttcttccaaccaatctggagggtgatcaacaaaagacatacctgatttaaatcatttattgttcaaagatgcagtcatccaaatccacattgaccagatcgcaggcagtgcaagcgtctggcacctttcccatgatatgatgaatgtagcacagtttctgatacgcctttttgacgacagaaacgggttgagattctgacacgggaaagcactctaaacagtctttctgtccgtgagtgaagcagatatttgaattctgattcattctctcgcattgtctgcagggaaacagcatcagattcatgcccacgtgacgagaacatttgttttggtacctgtctgcgtagttgatcgaagcttccgcgtctgacgtcgatggctgcgcaactgactcgcgcacccgtttgggctcacttatatctgcgtcactgggggcgggtcttttcttggctccaccctttttgacgtagaattcatgctccacctcaaccacgtgatcctttgcccaccggaaaaagtctttgacttcctgcttggtgaccttcccaaagtcatgatccagacggcgggtgagttcaaatttgaacatccggtcttgcaacggctgctggtgttcgaaggtcgttgagttcccgtcaatcacggcgcacatgttggtgttggaggtgacgatcacgggagtcgggtctatctgggccgaggacttgcatttctggtccacgcgcaccttgcttcctccgagaatggctttggccgactccacgaccttggcggtcatcttcccctcctcccaccagatcaccatcttgtcgacacagtcgttgaagggaaagttctcattggtccagtttacgcacccgtagaagggcacagtgtgggctatggcctccgcgatgttggtcttcccggtagttgcaggcccaaacagccagatggtgttcctcttgccgaactttttcgtggcccatcccagaaagacggaagccgcatattggggatcgtacccgtttagttccaaaattttataaatccgattgctggaaatgtcctccacgggctgctggcccaccaggtagtcgggggcggttttagtcaggctcataatctttcccgcattgtccaaggcagccttgatttgggaccgcgagttggaggccgcattgaaggagatgtatgaggcctggtcctcctggatccactgcttctccgaggtaatccccttgtccacgagccacccgaccagctccatgtacctggctgaagtttttgatctgatcaccggcgcatcagaattgggattctgattctctttgttctgctcctgcgtctgcgacacgtgcgtcagatgctgcgccaccaaccgtttacgctccgtgagattcaaacaggcgcttaaatactgttccatattagtccacgcccactggagctcaggctgggttttggggagcaagtaattggggatgtagcactcatccaccaccttgttcccgcctccggcgccatttctggtctttgtgaccgcgaaccagtttggcaaagtcggctcgatcccgcggtaaattctctgaatcagtttttcgcgaatctgactcaggaaacgtcccaaaaccatggatttcaccccggtggtttccacgagcacgtgcatgtggaagtagctctctcccttctcaaattgcacaaagaaaagagcctccggggccttactcacacggcgccattccgtcagaaagtcgcgctgcagcttctcggccacggtcaggggtgcctgctcaatcagattcagatccatgtcagaatctggcggcaactcccattccttctcggccacccagttcacaaagctgtcagaaatgccgggcagatgctcgtcaaggtcgctggggaccttaatcacaatctcgtaaaaccccggcatggcggctgcgcgttcaaacctcccgcttcaaaatggagaccctgcgtgctcactcgggcttaaatagaatggctaggatccggccggcctgcaggtgtcctcacaggaacgaagtccctaaagaaacagtggcagccaggtttagccccggaattgactggattccttttttagggcccattggtatggctttttccccgtatccccccaggtgtctgcaggctcaaagagcagcgagaagcgttcagaggaaagcgatcccgtgccaccttccccgtgcccgggctgtccccgcacgctgccggctcggggatgcggggggagcgccggaccggagcggagccccgggcggctcgctgctgccccctagcgggggagggacgtaattacatccctgggggctttgggggggggctgtccctctagagcggccgccaccgcggtggagctccagcttttgttccctttagtgagggttaattagatcttaatacgactcactatagggcgaattgggtaccgggccccccctcgaggtcgacggtatcgcctccaaggccagcttcccacaataagttgggtgaattttggctcattcctcctttctataggattgaggtcagagctttgtgatgggaattctgtggaatgtgtgtcagttagggtgtggaaagtcccgcgatcgctagcaaacgccagcaacgcggcctttttacggttcctggccttttgctggccttttgctcacatgtcctgcaggcagctgcgcgctcgctcgctcactgaggccgcccgggcaaagcccgggcgtcgggcgacctttggtcgcccggcctcagtgagcgagcgagcgcgcagagagggagtggccaactccatcactaggggttcctgcggccgcacgcgtggagctagttattaatagtaatcaattacggggtcattagttcatagcccatatatggagttccgcgttacataacttacggtaaatggcccgcctggctgaccgcccaacgacccccgcccattgacgtcaataatgacgtatgttcccatagtaacgtcaatagggactttccattgacgtcaatgggtggagtatttacggtaaactgcccacttggcagtacatcaagtgtatcatatgccaagtacgccccctattgacgtcaatgacggtaaatggcccgcctggcattatgcccagtacatgaccttatgggactttcctacttggcagtacatctacgtattagtcatcgctattaccatggtgatgcggttttggcagtacatcaatgggcgtggatagcggtttgactcacggggatttccaagtctccaccccattgacgtcaatgggagtttgttttgcaccaaaatcaacgggactttccaaaatgtcgtaacaactccgccccattgacgcaaatgggcggtaggcgtgtacggtgggaggtctatataagcagagctcgtttagtgaaccgtcagatcgcctggagacgccatccacgctgttttgacctccatagaagacaccgggaccgatccagcctccgcggattcgaatcccggccgggaacggtgcattggaacgcggattccccgtgccaagagtgacgtaagtaccgcctatagagtctataggcccacaaaaaatgctttcttcttttaatatacttttttgtttatcttatttctaatactttccctaatctctttctttcagggcaataatgatacaatgtatcatgcctctttgcaccattctaaagaataacagtgataatttctgggttaaggcaatagcaatatttctgcatataaatatttctgcatataaattgtaactgatgtaagaggtttcatattgctaatagcagctacaatccagctaccattctgcttttattttatggttgggataaggctggattattctgagtccaagctaggcccttttgctaatcatgttcatacctcttatcttcctcccacagctcctgggcaacgtgctggtctgtgtgctggcccatcactttggcaaagaattgggattcgaacatcgattgaattctgaatggtgagcaagggcgaggagctgttcaccggggtggtgcccatcctggtcgagctggacggcgacgtaaacggccacaagttcagcgtgtccggcgagggcgagggcgatgccacctacggcaagctgaccctgaagttcatctgcaccaccggcaagctgcccgtgccctggcccaccctcgtgaccaccctgacctacggcgtgcagtgcttcagccgctaccccgaccacatgaagcagcacgacttcttcaagtccgccatgcccgaaggctacgtccaggagcgcaccatcttcttcaaggacgacggcaactacaagacccgcgccgaggtgaagttcgagggcgacaccctggtgaaccgcatcgagctgaagggcatcgacttcaaggaggacggcaacatcctggggcacaagctggagtacaactacaacagccacaacgtctatatcatggccgacaagcagaagaacggcatcaaggtgaacttcaagatccgccacaacatcgaggacggcagcgtgcagctcgccgaccactaccagcagaacacccccatcggcgacggccccgtgctgctgcccgacaaccactacctgagcacccagtccgccctgagcaaagaccccaacgagaagcgcgatcacatggtcctgctggagttcgtgaccgccgccgggatcactctcggcatggacgagctgtacaagtactcagatctcgagctcaagtagggatcctctagagtcgacctgcagaagcttgcctcgagcagcgctgctcgagagatctacgggtggcatccctgtgacccctccccagtgcctctcctggccctggaagttgccactccagtgcccaccagccttgtcctaataaaattaagttgcatcattttgtctgactaggtgtccttctataatattatggggtggaggggggtggtatggagcaaggggcaagttgggaagacaacctgtagggcctgcggggtctattgggaaccaagctggagtgcagtggcacaatcttggctcactgcaatctccgcctcctgggttcaagcgattctcctgcctcagcctcccgagttgttgggattccaggcatgcatgaccaggctcagctaatttttgtttttttggtagagacggggtttcaccatattggccaggctggtctccaactcctaatctcaggtgatctacccaccttggcctcccaaattgctgggattacaggcgtgaaccactgctcccttccctgtccttctgattttgtaggtaaccacgtgcggaccgagcggccgcaggaacccctagtgatggagttggccactccctctctgcgcgctcgctcgctcactgaggccgggcgaccaaaggtcgcccgacgcccgggctttgcccgggcggcctcagtgagcgagcgagcgcgcagctgcctgcaggggcgcctgatgcggtattttctccttacgcatctgtgcggtatttcacaccgcatacgtcgtagctgatcaattggcgcgccgaattcgttaacaagctttaattaacgcgtacgataagcttgatatctataacaagaaaatatatatataataagttatcacgtaagtagaacatgaaataacaatataattatcgtatgagttaaatcttaaaagtcacgtaaaagataatcatgcgtcattttgactcacgcggtcgttatagttcaaaatcagtgacacttaccgcattgacaagcacgcctcacgggagctccaagcggcgactgagatgtcctaaatgcacagcgacggattcgcgctatttagaaagagagagcaatatttcaagaatgcatgcgtcaattttacgcagactatctttctagggttaatctagctgcatcaggatcatatcgtcgggtcttttttccggctcagtcatcgcccaagctggcgctatctgggcatcggggaggaagaagcccgtgccttttcccgcgaggttgaagcggcatggaaagagtttgccgaggatgactgctgctgcattgacgttgagcgaaaacgcacgtttaccatgatgattcgggaaggtgtggccatgcacgcctttaacggtgaactgttcgttcaggccacctgggataccagttcgtcgcggcttttccggacacagttccggatggtcagcccgaagcgcatcagcaacccgaacaataccggcgacagccggaactgccgtgccggtgtgcagattaatgacagcggtgcggcgctgggatattacgtcagcgaggacgggtatcctggctggatgccgcagaaatggacatggataccccgtgagttacccggcgggcgcgcttggcgtaatcatggtcatagctgtttcctgctcgtgtccgataactgtaattatcggacatgattgtgaaattgttatccgctcacaattccacacaacatacgagccggaagcataaagtgtaaagcctggggtgcctaatgagtgagctaactcacattaattgcgttgcgctcactgcccgctttccagtcgggaaacctgtcgtgccagctgcattaatgaatcggccaacgcgcggggagaggcggtttgcgtattgggcgctcttccgcttcctcgctcactgactcgctgcgctcggtcgttcggctgcggcgagcggtatcagctcactcaaaggcggtaatacggttatccacagaatcaggggataacgcaggaaagaacatgtgagcaaaaggccagcaaaaggccaggaaccgtaaaaaggccgcgttgctggcgtt